European Patent Application EP 4 389 903 A2, published June 26, 2024. Title: RNA-GUIDED GENE EDITING AND GENE REGULATION. Applicant: DUKE UNIVERSITY. Application EP 19168481.0, filed April 10, 2019. The sequence listing filed with the application follows.

SEQUENCE LISTING (676 sequences)

SEQ ID NO: 1 - protein, 1483 aa, synthetic construct
  REGION 1..1483: note = source = /note="Description of Artificial Sequence: Synthetic polypeptide"
MDYKDHDGDYKDHDIDYKDDDDKMAPKKKRKVGRGMDKKYSIGLAIGTNSVGWAVITDEYKVPSKKFKVLGNTDRHSIKKNLIGALLFDSGETAEATRLKRTARRRYTRRKNRICYLQEIFSNEMAKVDDSFFHRLEESFLVEEDKKHERHPIFGNIVDEVAYHEKYPTIYHLRKKLVDSTDKADLRLIYLALAHMIKFRGHFLIEGDLNPDNSDVDKLFIQLVQTYNQLFEENPINASGVDAKAILSARLSKSRRLENLIAQLPGEKKNGLFGNLIALSLGLTPNFKSNFDLAEDAKLQLSKDTYDDDLDNLLAQIGDQYADLFLAAKNLSDAILLSDILRVNTEITKAPLSASMIKRYDEHHQDLTLLKALVRQQLPEKYKEIFFDQSKNGYAGYIDGGASQEEFYKFIKPILEKMDGTEELLVKLNREDLLRKQRTFDNGSIPHQIHLGELHAILRRQEDFYPFLKDNREKIEKILTFRIPYYVGPLARGNSRFAWMTRKSEETITPWNFEEVVDKGASAQSFIERMTNFDKNLPNEKVLPKHSLLYEYFTVYNELTKVKYVTEGMRKPAFLSGEQKKAIVDLLFKTNRKVTVKQLKEDYFKKIECFDSVEISGVEDRFNASLGTYHDLLKIIKDKDFLDNEENEDILEDIVLTLTLFEDREMIEERLKTYAHLFDDKVMKQLKRRRYTGWGRLSRKLINGIRDKQSGKTILDFLKSDGFANRNFMQLIHDDSLTFKEDIQKAQVSGQGDSLHEHIANLAGSPAIKKGILQTVKVVDELVKVMGRHKPENIVIEMARENQTTQKGQKNSRERMKRIEEGIKELGSQILKEHPVENTQLQNEKLYLYYLQNGRDMYVDQELDINRLSDYDVDAIVPQSFLKDDSIDNKVLTRSDKNRGKSDNVPSEEVVKKMKNYWRQLLNAKLITQRKFDNLTKAERGGLSELDKAGFIKRQLVETRQITKHVAQILDSRMNTKYDENDKLIREVKVITLKSKLVSDFRKDFQFYKVREINNYHHAHDAYLNAVVGTALIKKYPKLESEFVYGDYKVYDVRKMIAKSEQEIGKATAKYFFYSNIMNFFKTEITLANGEIRKRPLIETNGETGEIVWDKGRDFATVRKVLSMPQVNIVKKTEVQTGGFSKESILPKRNSDKLIARKKDWDPKKYGGFDSPTVAYSVLVVAKVEKGKSKKLKSVKELLGITIMERSSFEKNPIDFLEAKGYKEVKKDLIIKLPKYSLFELENGRKRMLASAGELQKGNELALPSKYVNFLYLASHYEKLKGSPEDNEQKQLFVEQHKHYLDEIIEQISEFSKRVILADANLDKVLSAYNKHRDKPIREQAENIIHLFTLTNLGAPAAFKYFDTTIDRKRYTSTKEVLDATLIHQSITGLYETRIDLSQLGGDPIAGSKASPKKKRKVGRADALDDFDLDMLGSDALDDFDLDMLGSDALDDFDLDMLGSDALDDFDLDMLINYPYDVPDYAS

SEQ ID NO: 2 - DNA, 350 bp, synthetic construct
  misc_feature 1..350: note = source = /note="Description of Artificial Sequence: Synthetic polynucleotide"
  source 1..350: mol_type = other DNA
gagggcctatttcccatgattccttcatatttgcatatacgatacaaggctgttagagagataattggaattaatttgactgtaaacacaaagatattagtacaaaatacgtgacgtagaaagtaataatttcttgggtagtttgcagttttaaaattatgttttaaaatggactatcatatgcttatcgtaacttgaaagtatttcgatttcttggctttatatatcttgtggaaaggacgaaacaccgggtcttcgagaagacctgttttagagctagaaatagcaagttaaaataaggctagtccgttatcaacttgaaaaagtggcaccgagtcggtgcttttttt

SEQ ID NO: 3 - DNA, 338 bp, Homo sapiens
  source 1..338: mol_type = genomic DNA
acccccggcagcagcccgccccgagcgcgccgcctgtttattcagccgggagtccggcacgcgccaggcgcacgcactgcaacaacaaacccagctgaatggagagtttgcaaggagcgggagaaaggaacgggagggggggagaggagaggaggagggggagtttagggagtgggtgggaggaagaggtaagaggaggggggggagtgggggctgcagccgctcgctgcagcagcggggagtggggggcgaggcggggccagggctgcgcgtggggctgggtgtcccattgaaaaggcggacgcactccggcagcccagcactctctcacttctggc

SEQ ID NO: 4 - DNA, 305 bp, Mus musculus
  source 1..305: mol_type = genomic DNA
ccgccccgagcgcgcggcctgtttattcagccgggagtccggcacgcgccgggcgcacgcactgcaacaacaaaccaggctgaatggagagtttgcaaggagcgggcgcgggcaactggagggggggggggcgagagggagggagctgaggaggtgggggaagaggaggggtagtgggggctgcagccgctcgctgcagcagcggggagtggggggcgaggcggggccagggctgcgcgtggggctgggtgtcccattgaaaaggcggccgcaccgcagccgcccagcagtctctcacttctggc

SEQ ID NO: 5 - DNA, 19 bp, synthetic construct
  misc_feature 1..19: note = source = /note="Description of Artificial Sequence: Synthetic oligonucleotide"
  source 1..19: mol_type = other DNA
gctgggtgtcccattgaaa

SEQ ID NO: 6 - DNA, 19 bp, synthetic construct
  misc_feature 1..19: note = source = /note="Description of Artificial Sequence: Synthetic oligonucleotide"
  source 1..19: mol_type = other DNA
cagccgctcgctgcagcag

SEQ ID NO: 7 - DNA, 19 bp, synthetic construct
  misc_feature 1..19: note = source = /note="Description of Artificial Sequence: Synthetic oligonucleotide"
  source 1..19: mol_type = other DNA
tggagagtttgcaaggagc

SEQ ID NO: 8 - DNA, 19 bp, synthetic construct
  misc_feature 1..19: note = source = /note="Description of Artificial Sequence: Synthetic oligonucleotide"
  source 1..19: mol_type = other DNA
gtttattcagccgggagtc

SEQ ID NO: 9 - DNA, 20 bp, synthetic construct
  misc_feature 1..20: note = source = /note="Description of Artificial Sequence: Synthetic oligonucleotide"
  source 1..20: mol_type = other DNA
cgccaggaggggtgggtcta

SEQ ID NO: 10 - DNA, 19 bp, synthetic construct
  misc_feature 1..19: note = source = /note="Description of Artificial Sequence: Synthetic oligonucleotide"
  source 1..19: mol_type = other DNA
ccttggtgagactggtaga

SEQ ID NO: 11 - DNA, 19 bp, synthetic construct
  misc_feature 1..19: note = source = /note="Description of Artificial Sequence: Synthetic oligonucleotide"
  source 1..19: mol_type = other DNA
gtcttcaggttctgttgct

SEQ ID NO: 12 - DNA, 19 bp, synthetic construct
  misc_feature 1..19: note = source = /note="Description of Artificial Sequence: Synthetic oligonucleotide"
  source 1..19: mol_type = other DNA
atattcctgatttaaaagt

SEQ ID NO: 13 - DNA, 19 bp, synthetic construct
  misc_feature 1..19: note = source = /note="Description of Artificial Sequence: Synthetic oligonucleotide"
  source 1..19: mol_type = other DNA
ttaaaagtcggctggtagc

SEQ ID NO: 14 - DNA, 19 bp, synthetic construct
  misc_feature 1..19: note = source = /note="Description of Artificial Sequence: Synthetic oligonucleotide"
  source 1..19: mol_type = other DNA
cgggccgggggcggggtcc

SEQ ID NO: 15 - DNA, 19 bp, synthetic construct
  misc_feature 1..19: note = source = /note="Description of Artificial Sequence: Synthetic oligonucleotide"
  source 1..19: mol_type = other DNA
gcccgagccgcgtgtggaa

SEQ ID NO: 16 - DNA, 19 bp, synthetic construct
  misc_feature 1..19: note = source = /note="Description of Artificial Sequence: Synthetic oligonucleotide"
  source 1..19: mol_type = other DNA
ccttcattgcggcgggctg

SEQ ID NO: 17 - DNA, 19 bp, synthetic construct
  misc_feature 1..19: note = source = /note="Description of Artificial Sequence: Synthetic oligonucleotide"
  source 1..19: mol_type = other DNA
ccgacccctcccgggtccc

SEQ ID NO: 18 - DNA, 19 bp, synthetic construct
  misc_feature 1..19: note = source = /note="Description of Artificial Sequence: Synthetic oligonucleotide"
  source 1..19: mol_type = other DNA
caggaccgcgcttcccacg

SEQ ID NO: 19 - DNA, 19 bp, synthetic construct
  misc_feature 1..19: note = source = /note="Description of Artificial Sequence: Synthetic oligonucleotide"
  source 1..19: mol_type = other DNA
tgcaccctgggagcgcgag

SEQ ID NO: 20 - DNA, 19 bp, synthetic construct
  misc_feature 1..19: note = source = /note="Description of Artificial Sequence: Synthetic oligonucleotide"
  source 1..19: mol_type = other DNA
ccgcacgcacctgttccca

SEQ ID NO: 21 - DNA, 19 bp, synthetic construct
  misc_feature 1..19: note = source = /note="Description of Artificial Sequence: Synthetic oligonucleotide"
  source 1..19: mol_type = other DNA
aaaacagcgagggagaaac

SEQ ID NO: 22 - DNA, 19 bp, synthetic construct
  misc_feature 1..19: note = source = /note="Description of Artificial Sequence: Synthetic oligonucleotide"
  source 1..19: mol_type = other DNA
ttaacttgattgtgaaatc

SEQ ID NO: 23 - DNA, 19 bp, synthetic construct
  misc_feature 1..19: note = source = /note="Description of Artificial Sequence: Synthetic oligonucleotide"
  source 1..19: mol_type = other DNA
aaaacaatgcatatttgca

SEQ ID NO: 24 - DNA, 19 bp, synthetic construct
  misc_feature 1..19: note = source = /note="Description of Artificial Sequence: Synthetic oligonucleotide"
  source 1..19: mol_type = other DNA
aaaatccagtattttaatg

SEQ ID NO: 25 - DNA, 19 bp, synthetic construct
  misc_feature 1..19: note = source = /note="Description of Artificial Sequence: Synthetic oligonucleotide"
  source 1..19: mol_type = other DNA
acccagcactgcagcctgg

SEQ ID NO: 26 - DNA, 19 bp, synthetic construct
  misc_feature 1..19: note = source = /note="Description of Artificial Sequence: Synthetic oligonucleotide"
  source 1..19: mol_type = other DNA
aacttatgcggcgtttcct

SEQ ID NO: 27 - DNA, 19 bp, synthetic construct
  misc_feature 1..19: note = source = /note="Description of Artificial Sequence: Synthetic oligonucleotide"
  source 1..19: mol_type = other DNA
tcactttaaaaccacctct

SEQ ID NO: 28 - DNA, 19 bp, synthetic construct
  misc_feature 1..19: note = source = /note="Description of Artificial Sequence: Synthetic oligonucleotide"
  source 1..19: mol_type = other DNA
gcatctttttctctttaat

SEQ ID NO: 29 - DNA, 19 bp, synthetic construct
  misc_feature 1..19: note = source = /note="Description of Artificial Sequence: Synthetic oligonucleotide"
  source 1..19: mol_type = other DNA
tgtactctctgaggtgctc

SEQ ID NO: 30 - DNA, 19 bp, synthetic construct
  misc_feature 1..19: note = source = /note="Description of Artificial Sequence: Synthetic oligonucleotide"
  source 1..19: mol_type = other DNA
acgcagataagaaccagtt

SEQ ID NO: 31 - DNA, 19 bp, synthetic construct
  misc_feature 1..19: note = source = /note="Description of Artificial Sequence: Synthetic oligonucleotide"
  source 1..19: mol_type = other DNA
catcaagtcagccatcagc

SEQ ID NO: 32 - DNA, 19 bp, synthetic construct
  misc_feature 1..19: note = source = /note="Description of Artificial Sequence: Synthetic oligonucleotide"
  source 1..19: mol_type = other DNA
gagtcaccctcctggaaac

SEQ ID NO: 33 - DNA, 19 bp, synthetic construct
  misc_feature 1..19: note = source = /note="Description of Artificial Sequence: Synthetic oligonucleotide"
  source 1..19: mol_type = other DNA
gctagggatgaagaataaa

SEQ ID NO: 34 - DNA, 19 bp, synthetic construct
  misc_feature 1..19: note = source = /note="Description of Artificial Sequence: Synthetic oligonucleotide"
  source 1..19: mol_type = other DNA
ttgaccaatagccttgaca

SEQ ID NO: 35 - DNA, 19 bp, synthetic construct
  misc_feature 1..19: note = source = /note="Description of Artificial Sequence: Synthetic oligonucleotide"
  source 1..19: mol_type = other DNA
tgcaaatatctgtctgaaa

SEQ ID NO: 36 - DNA, 19 bp, synthetic construct
  misc_feature 1..19: note = source = /note="Description of Artificial Sequence: Synthetic oligonucleotide"
  source 1..19: mol_type = other DNA
aaattagcagtatcctctt

SEQ ID NO: 37 - DNA, 19 bp, synthetic construct
  misc_feature 1..19: note = source = /note="Description of Artificial Sequence: Synthetic oligonucleotide"
  source 1..19: mol_type = other DNA
cctgggctccggggcgttt

SEQ ID NO: 38 - DNA, 19 bp, synthetic construct
  misc_feature 1..19: note = source = /note="Description of Artificial Sequence: Synthetic oligonucleotide"
  source 1..19: mol_type = other DNA
ggcccctgcggccaccccg

SEQ ID NO: 39 - DNA, 19 bp, synthetic construct
  misc_feature 1..19: note = source = /note="Description of Artificial Sequence: Synthetic oligonucleotide"
  source 1..19: mol_type = other DNA
ctccctccctgcccggtag

SEQ ID NO: 40 - DNA, 19 bp, synthetic construct
  misc_feature 1..19: note = source = /note="Description of Artificial Sequence: Synthetic oligonucleotide"
  source 1..19: mol_type = other DNA
aggtttggaaagggcgtgc

SEQ ID NO: 41 - DNA, 20 bp, synthetic construct
  misc_feature 1..20: note = source = /note="Description of Artificial Sequence: Synthetic primer"
  source 1..20: mol_type = other DNA
ggagcttctcgacttcacca

SEQ ID NO: 42 - DNA, 20 bp, synthetic construct
  misc_feature 1..20: note = source = /note="Description of Artificial Sequence: Synthetic primer"
  source 1..20: mol_type = other DNA
gatttgtgggcctgaagaaa

SEQ ID NO: 43 - DNA, 20 bp, synthetic construct
  misc_feature 1..20: note = source = /note="Description of Artificial Sequence: Synthetic primer"
  source 1..20: mol_type = other DNA
aaggaggagggcagaatcat

SEQ ID NO: 44 - DNA, 21 bp, synthetic construct
  misc_feature 1..21: note = source = /note="Description of Artificial Sequence: Synthetic primer"
  source 1..21: mol_type = other DNA
aaaccttcctcagctatgccc

SEQ ID NO: 45 - DNA, 20 bp, synthetic construct
  misc_feature 1..20: note = source = /note="Description of Artificial Sequence: Synthetic primer"
  source 1..20: mol_type = other DNA
agctgatggccctaaacaga

SEQ ID NO: 46 - DNA, 20 bp, synthetic construct
  misc_feature 1..20: note = source = /note="Description of Artificial Sequence: Synthetic primer"
  source 1..20: mol_type = other DNA
caggaggactctggcaccta

SEQ ID NO: 47 - DNA, 20 bp, synthetic construct
  misc_feature 1..20: note = source = /note="Description of Artificial Sequence: Synthetic primer"
  source 1..20: mol_type = other DNA
ggaatccatggagggaagat

SEQ ID NO: 48 - DNA, 21 bp, synthetic construct
  misc_feature 1..21: note = source = /note="Description of Artificial Sequence: Synthetic primer"
  source 1..21: mol_type = other DNA
gctgagtgaactgcactgtga

SEQ ID NO: 49 - DNA, 20 bp, synthetic construct
  misc_feature 1..20: note = source = /note="Description of Artificial Sequence: Synthetic primer"
  source 1..20: mol_type = other DNA
ctctctgctcctttgccaca

SEQ ID NO: 50 - DNA, 20 bp, synthetic construct
  misc_feature 1..20: note = source = /note="Description of Artificial Sequence: Synthetic primer"
  source 1..20: mol_type = other DNA
caatgaccccttcattgacc

SEQ ID NO: 51 - DNA, 20 bp, synthetic construct
  misc_feature 1..20: note = source = /note="Description of Artificial Sequence: Synthetic primer"
  source 1..20: mol_type = other DNA
ggaacaagagctgctggact

SEQ ID NO: 52 - DNA, 20 bp, synthetic construct
  misc_feature 1..20: note = source = /note="Description of Artificial Sequence: Synthetic primer"
  source 1..20: mol_type = other DNA
aactttggcattgtggaagg

SEQ ID NO: 53 - DNA, 20 bp, synthetic construct
  misc_feature 1..20: note = source = /note="Description of Artificial Sequence: Synthetic primer"
  source 1..20: mol_type = other DNA
aacgccactgacaagaaagc

SEQ ID NO: 54 - DNA, 20 bp, synthetic construct
  misc_feature 1..20: note = source = /note="Description of Artificial Sequence: Synthetic primer"
  source 1..20: mol_type = other DNA
cagatccatggaggaaggaa

SEQ ID NO: 55 - DNA, 21 bp, synthetic construct
  misc_feature 1..21: note = source = /note="Description of Artificial Sequence: Synthetic primer"
  source 1..21: mol_type = other DNA
gggtactcctggaagatgtcc

SEQ ID NO: 56 - DNA, 20 bp, synthetic construct
  misc_feature 1..20: note = source = /note="Description of Artificial Sequence: Synthetic primer"
  source 1..20: mol_type = other DNA
gtttgcgacgcatgttcctc

SEQ ID NO: 57 - DNA, 20 bp, synthetic construct
  misc_feature 1..20: note = source = /note="Description of Artificial Sequence: Synthetic primer"
  source 1..20: mol_type = other DNA
aagcccttgctgtagtggtg

SEQ ID NO: 58 - DNA, 20 bp, synthetic construct
  misc_feature 1..20: note = source = /note="Description of Artificial Sequence: Synthetic primer"
  source 1..20: mol_type = other DNA
cggcaggaaagcatctgtat

SEQ ID NO: 59 - DNA, 20 bp, synthetic construct
  misc_feature 1..20: note = source = /note="Description of Artificial Sequence: Synthetic primer"
  source 1..20: mol_type = other DNA
tgttctcgctcaggtcagtg

SEQ ID NO: 60 - DNA, 20 bp, synthetic construct
  misc_feature 1..20: note = source = /note="Description of Artificial Sequence: Synthetic primer"
  source 1..20: mol_type = other DNA
gaattctttgccgaaatgga

SEQ ID NO: 61 - DNA, 20 bp, synthetic construct
  misc_feature 1..20: note = source = /note="Description of Artificial Sequence: Synthetic primer"
  source 1..20: mol_type = other DNA
gtgctcttcgggtttcagga

SEQ ID NO: 62 - DNA, 20 bp, synthetic construct
  misc_feature 1..20: note = source = /note="Description of Artificial Sequence: Synthetic primer"
  source 1..20: mol_type = other DNA
ttgattttggagggatctcg

SEQ ID NO: 63 - DNA, 20 bp, synthetic construct
  misc_feature 1..20: note = source = /note="Description of Artificial Sequence: Synthetic primer"
  source 1..20: mol_type = other DNA
gtttttctgcctccccattt

SEQ ID NO: 64 - DNA, 20 bp, synthetic construct
  misc_feature 1..20: note = source = /note="Description of Artificial Sequence: Synthetic primer"
  source 1..20: mol_type = other DNA
ggatgcagggatgatgttct

SEQ ID NO: 65 - DNA, 20 bp, synthetic construct
  misc_feature 1..20: note = source = /note="Description of Artificial Sequence: Synthetic oligonucleotide"
  source 1..20: mol_type = other DNA
gattggctttgatttcccta

SEQ ID NO: 66 - DNA, 23 bp, synthetic construct
  misc_feature 1..23: note = source = /note="Description of Artificial Sequence: Synthetic oligonucleotide"
  source 1..23: mol_type = other DNA
gtgtagagtaagtcagcctatgg

SEQ ID NO: 67 - DNA, 20 bp, synthetic construct
  misc_feature 1..20: note = source = /note="Description of Artificial Sequence: Synthetic oligonucleotide"
  source 1..20: mol_type = other DNA
gcctactcagactgttactc

SEQ ID NO: 68 - DNA, 23 bp, synthetic construct
  misc_feature 1..23: note = source = /note="Description of Artificial Sequence: Synthetic oligonucleotide"
  source 1..23: mol_type = other DNA
gttggacagaacttaccgactgg

SEQ ID NO: 69 - DNA, 20 bp, synthetic construct
  misc_feature 1..20: note = source = /note="Description of Artificial Sequence: Synthetic oligonucleotide"
  source 1..20: mol_type = other DNA
gcagttgcctaagaactggt

SEQ ID NO: 70 - DNA, 20 bp, synthetic construct
  misc_feature 1..20: note = source = /note="Description of Artificial Sequence: Synthetic oligonucleotide"
  source 1..20: mol_type = other DNA
ggggctccaccctcacgagt

SEQ ID NO: 71 - DNA, 23 bp, synthetic construct
  misc_feature 1..23: note = source = /note="Description of Artificial Sequence: Synthetic oligonucleotide"
  source 1..23: mol_type = other DNA
gtttgcttcgctataaaacgagg

SEQ ID NO: 72 - DNA, 23 bp, synthetic construct
  misc_feature 1..23: note = source = /note="Description of Artificial Sequence: Synthetic oligonucleotide"
  source 1..23: mol_type = other DNA
gtctgaggatggggccgcaatgg

SEQ ID NO: 73 - DNA, 23 bp, synthetic construct
  misc_feature 1..23: note = source = /note="Description of Artificial Sequence: Synthetic oligonucleotide"
  source 1..23: mol_type = other DNA
ggatctgtcaaatcgcctgcagg

SEQ ID NO: 74 - DNA, 23 bp, synthetic construct
  misc_feature 1..23: note = source = /note="Description of Artificial Sequence: Synthetic oligonucleotide"
  source 1..23: mol_type = other DNA
gccaggatggcattgggcagcgg

SEQ ID NO: 75 - DNA, 23 bp, synthetic construct
  misc_feature 1..23: note = source = /note="Description of Artificial Sequence: Synthetic oligonucleotide"
  source 1..23: mol_type = other DNA
gctgaatctgcggtggcaggagg

SEQ ID NO: 76 - DNA, 23 bp, synthetic construct
  misc_feature 1..23: note = source = /note="Description of Artificial Sequence: Synthetic oligonucleotide"
  source 1..23: mol_type = other DNA
gttcttttgttcttctagcctgg

SEQ ID NO: 77 - DNA, 23 bp, synthetic construct
  misc_feature 1..23: note = source = /note="Description of Artificial Sequence: Synthetic oligonucleotide"
  source 1..23: mol_type = other DNA
ggaaaagcttgagcaagtcaagg

SEQ ID NO: 78 - DNA, 23 bp, synthetic construct
  misc_feature 1..23: note = source = /note="Description of Artificial Sequence: Synthetic oligonucleotide"
  source 1..23: mol_type = other DNA
ggaagagttgcccctgcgccagg

SEQ ID NO: 79 - DNA, 23 bp, synthetic construct
  misc_feature 1..23: note = source = /note="Description of Artificial Sequence: Synthetic oligonucleotide"
  source 1..23: mol_type = other DNA
gacaaatctccagtggataaagg

SEQ ID NO: 80 - DNA, 23 bp, synthetic construct
  misc_feature 1..23: note = source = /note="Description of Artificial Sequence: Synthetic oligonucleotide"
  source 1..23: mol_type = other DNA
gtgtttctcaggtaaagctctgg

SEQ ID NO: 81 - DNA, 23 bp, synthetic construct
  misc_feature 1..23: note = source = /note="Description of Artificial Sequence: Synthetic oligonucleotide"
  source 1..23: mol_type = other DNA
ggaaggaccatttgacgttaagg

SEQ ID NO: 82 - DNA, 23 bp, synthetic construct
  misc_feature 1..23: note = source = /note="Description of Artificial Sequence: Synthetic oligonucleotide"
  source 1..23: mol_type = other DNA
gaactgctatttcagtttcctgg

SEQ ID NO: 83 - DNA, 23 bp, synthetic construct
  misc_feature 1..23: note = source = /note="Description of Artificial Sequence: Synthetic oligonucleotide"
  source 1..23: mol_type = other DNA
gccagccactcagccagtgaagg

SEQ ID NO: 84 - DNA, 23 bp, synthetic construct
  misc_feature 1..23: note = source = /note="Description of Artificial Sequence: Synthetic oligonucleotide"
  source 1..23: mol_type = other DNA
ggtatgcttttctgttaaagagg

SEQ ID NO: 85 - DNA, 23 bp, synthetic construct
  misc_feature 1..23: note = source = /note="Description of Artificial Sequence: Synthetic oligonucleotide"
  source 1..23: mol_type = other DNA
gctcctggactgaccactattgg

SEQ ID NO: 86 - DNA, 23 bp, synthetic construct
  misc_feature 1..23: note = source = /note="Description of Artificial Sequence: Synthetic oligonucleotide"
  source 1..23: mol_type = other DNA
ggaacagaggcgtccccagttgg

SEQ ID NO: 87 - DNA, 23 bp, synthetic construct
  misc_feature 1..23: note = source = /note="Description of Artificial Sequence: Synthetic oligonucleotide"
  source 1..23: mol_type = other DNA
ggaggctagaacaatcattacgg

SEQ ID NO: 88 - DNA, 23 bp, synthetic construct
  misc_feature 1..23: note = source = /note="Description of Artificial Sequence: Synthetic oligonucleotide"
  source 1..23: mol_type = other DNA
gacaagaacaccttcagaaccgg

SEQ ID NO: 89 - DNA, 23 bp, synthetic construct
  misc_feature 1..23: note = source = /note="Description of Artificial Sequence: Synthetic oligonucleotide"
  source 1..23: mol_type = other DNA
gggtttctgtgattttcttttgg

SEQ ID NO: 90 - DNA, 23 bp, synthetic construct
  misc_feature 1..23: note = source = /note="Description of Artificial Sequence: Synthetic oligonucleotide"
  source 1..23: mol_type = other DNA
gggccaaagacctccgccagtgg

SEQ ID NO: 91 - DNA, 23 bp, synthetic construct
  misc_feature 1..23: note = source = /note="Description of Artificial Sequence: Synthetic oligonucleotide"
  source 1..23: mol_type = other DNA
gttggagaagcattcataaaagg

SEQ ID NO: 92 - DNA, 23 bp, synthetic construct
  misc_feature 1..23: note = source = /note="Description of Artificial Sequence: Synthetic oligonucleotide"
  source 1..23: mol_type = other DNA
gtcgctcactcaccctgcaaagg

SEQ ID NO: 93 - DNA, 23 bp, synthetic construct
  misc_feature 1..23: note = source = /note="Description of Artificial Sequence: Synthetic oligonucleotide"
  source 1..23: mol_type = other DNA
gaaaagagctgatgaaacaatgg

SEQ ID NO: 94 - DNA, 23 bp, synthetic construct
  misc_feature 1..23: note = source = /note="Description of Artificial Sequence: Synthetic oligonucleotide"
  source 1..23: mol_type = other DNA
gtacacttttcaaaatgctttgg

SEQ ID NO: 95 - DNA, 23 bp, synthetic construct
  misc_feature 1..23: note = source = /note="Description of Artificial Sequence: Synthetic oligonucleotide"
  source 1..23: mol_type = other DNA
ggagatgatcatcaagcagaagg

SEQ ID NO: 96 - DNA, 23 bp, synthetic construct
  misc_feature 1..23: note = source = /note="Description of Artificial Sequence: Synthetic oligonucleotide"
  source 1..23: mol_type = other DNA
gctttgaaagagcaataaaatgg

SEQ ID NO: 97 - DNA, 23 bp, synthetic construct
  misc_feature 1..23: note = source = /note="Description of Artificial Sequence: Synthetic oligonucleotide"
  source 1..23: mol_type = other DNA
gcacaaaagtcaaatcggaatgg

SEQ ID NO: 98 - DNA, 23 bp, synthetic construct
  misc_feature 1..23: note = source = /note="Description of Artificial Sequence: Synthetic oligonucleotide"
  source 1..23: mol_type = other DNA
gatttcaatataagattcggagg

SEQ ID NO: 99 - DNA, 23 bp, synthetic construct
  misc_feature 1..23: note = source = /note="Description of Artificial Sequence: Synthetic oligonucleotide"
  source 1..23: mol_type = other DNA
gcttaagcaatcccgaactctgg

SEQ ID NO: 100 - DNA, 20 bp, synthetic construct
  misc_feature 1..20: note = source = /note="Description of Artificial Sequence: Synthetic oligonucleotide"
  source 1..20: mol_type = other DNA
gccttctttatcccctatcg

SEQ ID NO: 101-103 - skipped (3 entries)

SEQ ID NO: 104 - DNA, 25 bp, synthetic construct
  variation 21..22: note = a, c, t, g, unknown or other
  misc_feature 1..25: note = source = /note="Description of Artificial Sequence: Synthetic oligonucleotide"
  source 1..25: mol_type = other DNA
gaggccaaacctcggcttacnngrr

SEQ ID NO: 105 - DNA, 25 bp, synthetic construct
  variation 21..22: note = a, c, t, g, unknown or other
  misc_feature 1..25: note = source = /note="Description of Artificial Sequence: Synthetic oligonucleotide"
  source 1..25: mol_type = other DNA
gttcgaaaatttcaggtaagnngrr

SEQ ID NO: 106 - DNA, 26 bp, synthetic construct
  variation 21..22: note = a, c, t, g, unknown or other
  misc_feature 1..26: note = source = /note="Description of Artificial Sequence: Synthetic oligonucleotide"
  source 1..26: mol_type = other DNA
ggcagaacaggagataacagnngrrt

SEQ ID NO: 107 - DNA, 26 bp, synthetic construct
  misc_feature 1..26: note = source = /note="Description of Artificial Sequence: Synthetic oligonucleotide"
  source 1..26: mol_type = other DNA
ggcggccctcgcccttctctggggat

SEQ ID NO: 108 - DNA, 23 bp, synthetic construct
  misc_feature 1..23: note = source = /note="Description of Artificial Sequence: Synthetic oligonucleotide"
  source 1..23: mol_type = other DNA
gtagtgatcgtggatacgagagg

SEQ ID NO: 109 - DNA, 23 bp, synthetic construct
  misc_feature 1..23: note = source = /note="Description of Artificial Sequence: Synthetic oligonucleotide"
  source 1..23: mol_type = other DNA
gtacagccctcggtgtatattgg

SEQ ID NO: 110 - DNA, 23 bp, synthetic construct
  misc_feature 1..23: note = source = /note="Description of Artificial Sequence: Synthetic oligonucleotide"
  source 1..23: mol_type = other DNA
gggaaggaattaagcccgaatgg

SEQ ID NO: 111 - DNA, 23 bp, synthetic construct
  misc_feature 1..23: note = source = /note="Description of Artificial Sequence: Synthetic oligonucleotide"
  source 1..23: mol_type = other DNA
gggaacagctttcgtagttgagg

SEQ ID NO: 112 - DNA, 23 bp, synthetic construct
  misc_feature 1..23: note = source = /note="Description of Artificial Sequence: Synthetic oligonucleotide"
  source 1..23: mol_type = other DNA
gataaagtccagtgtcgatcagg

SEQ ID NO: 113 - DNA, 23 bp, synthetic construct
  misc_feature 1..23: note = source = /note="Description of Artificial Sequence: Synthetic oligonucleotide"
  source 1..23: mol_type = other DNA
gaaaaccagagcttcggtcaagg

SEQ ID NO: 114 - DNA, 34 bp, synthetic construct
  misc_feature 1..34: note = source = /note="Description of Artificial Sequence: Synthetic oligonucleotide"
  source 1..34: mol_type = other DNA
ggagtcttctgggcaggcttaaaggctaacctgg

SEQ ID NO: 115 - DNA, 34 bp, synthetic construct
  misc_feature 1..34: note = source = /note="Description of Artificial Sequence: Synthetic oligonucleotide"
  source 1..34: mol_type = other DNA
gtcgggtgagcatgtctttaatctacctcgatgg

SEQ ID NO: 116 - DNA, 26 bp, synthetic construct
  misc_feature 1..26: note = source = /note="Description of Artificial Sequence: Synthetic oligonucleotide"
  source 1..26: mol_type = other DNA
ggtgtcaccagagtaacagtctgagt

SEQ ID NO: 117 - DNA, 25 bp, synthetic construct
  misc_feature 1..25: note = source = /note="Description of Artificial Sequence: Synthetic oligonucleotide"
  source 1..25: mol_type = other DNA
gtgatcatcaagcagaaggtatgag

SEQ ID NO: 118 - DNA, 29 bp, synthetic construct
  misc_feature 1..29: note = source = /note="Description of Artificial Sequence: Synthetic oligonucleotide"
  source 1..29: mol_type = other DNA
gaacttcgaaaatttcaggtaagccgagg

SEQ ID NO: 119 - DNA, 29 bp, synthetic construct
  misc_feature 1..29: note = source = /note="Description of Artificial Sequence: Synthetic oligonucleotide"
  source 1..29: mol_type = other DNA
ggaaactcatcaaatatgcgtgttagtgt

SEQ ID NO: 120 - DNA, 29 bp, synthetic construct
  misc_feature 1..29: note = source = /note="Description of Artificial Sequence: Synthetic oligonucleotide"
  source 1..29: mol_type = other DNA
gtcatttacactaacacgcatatttgatg

SEQ ID NO: 121 - DNA, 29 bp, synthetic construct
  misc_feature 1..29: note = source = /note="Description of Artificial Sequence: Synthetic oligonucleotide"
  source 1..29: mol_type = other DNA
ggaatgaaactcatcaaatatgcgtgtta

SEQ ID NO: 122 - DNA, 29 bp, synthetic construct
  misc_feature 1..29: note = source = /note="Description of Artificial Sequence: Synthetic oligonucleotide"
  source 1..29: mol_type = other DNA
gtcatcaatatctttgaaggactctgggt

SEQ ID NO: 123 - DNA, 29 bp, synthetic construct
  misc_feature 1..29: note = source = /note="Description of Artificial Sequence: Synthetic oligonucleotide"
  source 1..29: mol_type = other DNA
gtgttttcataggaaaaataggcaagttg

SEQ ID NO: 124 - DNA, 29 bp, synthetic construct
  misc_feature 1..29: note = source = /note="Description of Artificial Sequence: Synthetic oligonucleotide"
  source 1..29: mol_type = other DNA
gaattggaaaatgtgatgggaaacagata

SEQ ID NO: 125 - DNA, 29 bp, synthetic construct
  misc_feature 1..29: note = source = /note="Description of Artificial Sequence: Synthetic oligonucleotide"
  source 1..29: mol_type = other DNA
gatgatcatcaagcagaaggtatgagaaa

SEQ ID NO: 126 - DNA, 29 bp, synthetic construct
  misc_feature 1..29: note = source = /note="Description of Artificial Sequence: Synthetic oligonucleotide"
  source 1..29: mol_type = other DNA
gagatgatcatcaagcagaaggtatgaga

SEQ ID NO: 127 - DNA, 29 bp, synthetic construct
  misc_feature 1..29: note = source = /note="Description of Artificial Sequence: Synthetic oligonucleotide"
  source 1..29: mol_type = other DNA
gcattttttctcataccttctgcttgatg

SEQ ID NO: 128 - DNA, 29 bp, synthetic construct
  misc_feature 1..29: note = source = /note="Description of Artificial Sequence: Synthetic oligonucleotide"
  source 1..29: mol_type = other DNA
gtcctactcagactgttactctggtgaca

SEQ ID NO: 129 - DNA, 29 bp, synthetic construct
  misc_feature 1..29: note = source = /note="Description of Artificial Sequence: Synthetic oligonucleotide"
  source 1..29: mol_type = other DNA
gacaggttgtgtcaccagagtaacagtct

SEQ ID NO: 130 - DNA, 29 bp, synthetic construct
  misc_feature 1..29: note = source = /note="Description of Artificial Sequence: Synthetic oligonucleotide"
  source 1..29: mol_type = other DNA
gttatcattttttctcataccttctgctt

SEQ ID NO: 131 - DNA, 29 bp, synthetic construct
  misc_feature 1..29: note = source = /note="Description of Artificial Sequence: Synthetic oligonucleotide"
  source 1..29: mol_type = other DNA
gttgcctaagaactggtgggaaatggtct

SEQ ID NO: 132 - DNA, 29 bp, synthetic construct
  misc_feature 1..29: note = source = /note="Description of Artificial Sequence: Synthetic oligonucleotide"
  source 1..29: mol_type = other DNA
gaaacagttgcctaagaactggtgggaaa

SEQ ID NO: 133 - DNA, 29 bp, synthetic construct
  misc_feature 1..29: note = source = /note="Description of Artificial Sequence: Synthetic oligonucleotide"
  source 1..29: mol_type = other DNA
gtttcccaccagttcttaggcaactgttt

SEQ ID NO: 134 - DNA, 29 bp, synthetic construct
  misc_feature 1..29: note = source = /note="Description of Artificial Sequence: Synthetic oligonucleotide"
  source 1..29: mol_type = other DNA
gtggctttgatttccctagggtccagctt

SEQ ID NO: 135 - DNA, 29 bp, synthetic construct
  misc_feature 1..29: note = source = /note="Description of Artificial Sequence: Synthetic oligonucleotide"
  source 1..29: mol_type = other DNA
gtagggaaatcaaagccaatgaaacgttc

SEQ ID NO: 136 - DNA, 29 bp, synthetic construct
  misc_feature 1..29: note = source = /note="Description of Artificial Sequence: Synthetic oligonucleotide"
  source 1..29: mol_type = other DNA
ggaccctagggaaatcaaagccaatgaaa

SEQ ID NO: 137 - DNA, 29 bp, synthetic construct
  misc_feature 1..29: note = source = /note="Description of Artificial Sequence: Synthetic oligonucleotide"
  source 1..29: mol_type = other DNA
gtgagggctccaccctcacgagtgggttt

SEQ ID NO: 138 - DNA, 29 bp, synthetic construct
  misc_feature 1..29: note = source = /note="Description of Artificial Sequence: Synthetic oligonucleotide"
  source 1..29: mol_type = other DNA
gaaggattgagggctccaccctcacgagt

SEQ ID NO: 139 - DNA, 29 bp, synthetic construct
  misc_feature 1..29: note = source = /note="Description of Artificial Sequence: Synthetic oligonucleotide"
  source 1..29: mol_type = other DNA
ggctccaccctcacgagtgggtttggttc

SEQ ID NO: 140 - DNA, 29 bp, synthetic construct
  misc_feature 1..29: note = source = /note="Description of Artificial Sequence: Synthetic oligonucleotide"
  source 1..29: mol_type = other DNA
gtatcccctatcgaggaaaccacgagttt

SEQ ID NO: 141 - DNA, 29 bp, synthetic construct
  misc_feature 1..29: note = source = /note="Description of Artificial Sequence: Synthetic oligonucleotide"
  source 1..29: mol_type = other DNA
ggataaagaaggcctatttcatagagttg

SEQ ID NO: 142 - DNA, 29 bp, synthetic construct
  misc_feature 1..29: note = source = /note="Description of Artificial Sequence: Synthetic oligonucleotide"
  source 1..29: mol_type = other DNA
gaggccttctttatcccctatcgaggaaa

SEQ ID NO: 143 - DNA, 27 bp, synthetic construct
  misc_feature 1..27: note = source = /note="Description of Artificial Sequence: Synthetic oligonucleotide"
  source 1..27: mol_type = other DNA
gtgagggctccaccctcacgagtgggt

SEQ ID NO: 144 - DNA, 27 bp, synthetic construct
  misc_feature 1..27: note = source = /note="Description of Artificial Sequence: Synthetic oligonucleotide"
  source 1..27: mol_type = other DNA
ggataaagaaggcctatttcatagagt

SEQ ID NO: 145 - DNA, 4932 bp, synthetic construct
  misc_feature 1..4932: note = source = /note="Description of Artificial Sequence: Synthetic polynucleotide"
  source 1..4932: mol_type = other DNA
gccaccatggacaagaagtactccattgggctcgatatcggcacaaacagcgtcggctgggccgtcattacggacgagtacaaggtgccgagcaaaaaattcaaagttctgggcaataccgatcgccacagcataaagaagaacctcattggcgccctcctgttcgactccggggagacggccgaagccacgcggctcaaaagaacagcacggcgcagatatacccgcagaaagaatcggatctgctacctgcaggagatctttagtaatgagatggctaaggtggatgactctttcttccataggctggaggagtcctttttggtggaggaggataaaaagcacgagcgccacccaatctttggcaatatcgtggacgaggtggcgtaccatgaaaagtacccaaccatatatcatctgaggaagaagcttgtagacagtactgataaggctgacttgcggttgatctatctcgcgctggcgcatatgatcaaatttcggggacacttcctcatcgagggggacctgaacccagacaacagcgatgtcgacaaactctttatccaactggttcagacttacaatcagcttttcgaagagaacccgatcaacgcatccggagttgacgccaaagcaatcctgagcgctaggctgtccaaatcccggcggctcgaaaacctcatcgcacagctccctggggagaagaagaacggcctgtttggtaatcttatcgccctgtcactcgggctgacccccaactttaaatctaacttcgacctggccgaagatgccaagcttcaactgagcaaagacacctacgatgatgatctcgacaatctgctggcccagatcggcgaccagtacgcagacctttttttggcggcaaagaacctgtcagacgccattctgctgagtgatattctgcgagtgaacacggagatcaccaaagctccgctgagcgctagtatgatcaagcgctatgatgagcaccaccaagacttgactttgctgaaggcccttgtcagacagcaactgcctgagaagtacaaggaaattttcttcgatcagtctaaaaatggctacgccggatacattgacggcggagcaagccaggaggaattttacaaatttattaagcccatcttggaaaaaatggacggcaccgaggagctgctggtaaagcttaacagagaagatctgttgcgcaaacagcgcactttcgacaatggaagcatcccccaccagattcacctgggcgaactgcacgctatcctcaggcggcaagaggatttctacccctttttgaaagataacagggaaaagattgagaaaatcctcacatttcggataccctactatgtaggccccctcgcccggggaaattccagattcgcgtggatgactcgcaaatcagaagagaccatcactccctggaacttcgaggaagtcgtggataagggggcctctgcccagtccttcatcgaaaggatgactaactttgataaaaatctgcctaacgaaaaggtgcttcctaaacactctctgctgtacgagtacttcacagtttataacgagctcaccaaggtcaaatacgtcacagaagggatgagaaagccagcattcctgtctggagagcagaagaaagctatcgtggacctcctcttcaagacgaaccggaaagttaccgtgaaacagctcaaagaagactatttcaaaaagattgaatgtttcgactctgttgaaatcagcggagtggaggatcgcttcaacgcatccctgggaacgtatcacgatctcctgaaaatcattaaagacaaggacttcctggacaatgaggagaacgaggacattcttgaggacattgtcctcacccttacgttgtttgaagatagggagatgattgaagaacgcttgaaaacttacgctcatctcttcgacgacaaagtcatgaaacagctcaagaggcgccgatatacaggatgggggcggctgtcaagaaaactgatcaatgggatccgagacaagcagagtggaaagacaatcctggattttcttaagtccgatggatttgccaaccggaacttcatgcagttgatccatgatgactctctcacctttaaggaggacatccagaaagcacaagtttctggccagggggacagtcttcacgagcacatcgctaatcttgcaggtagcccagctatcaaaaagggaatactgcagaccgttaaggtcgtggatgaactcgtcaaagtaatgggaaggcataagcccgagaatatcgttatcgagatggcccgagagaaccaaactacccagaagggacagaagaacagtagggaaaggatgaagaggattgaagagggtataaaagaactggggtcccaaatccttaaggaacacccagttgaaaacacccagcttcagaatgagaagctctacctgtactacctgcagaacggcagggacatgtacgtggatcaggaactggacatcaatcggctctccgactacgacgtggatcatatcgtgccccagtcttttctcaaagatgattctattgataataaagtgttgacaagatccgataaaaatagagggaagagtgataacgtcccctcagaagaagttgtcaagaaaatgaaaaattattggcggcagctgctgaacgccaaactgatcacacaacggaagttcgataatctgactaaggctgaacgaggtggcctgtctgagttggataaagccggcttcatcaaaaggcagcttgttgagacacgccagatcaccaagcacgtggcccaaattctcgattcacgcatgaacaccaagtacgatgaaaatgacaaactgattcgagaggtgaaagttattactctgaagtctaagctggtctcagatttcagaaaggactttcagttttataaggtgagagagatcaacaattaccaccatgcgcatgatgcctacctgaatgcagtggtaggcactgcacttatcaaaaaatatcccaagcttgaatctgaatttgtttacggagactataaagtgtacgatgttaggaaaatgatcgcaaagtctgagcaggaaataggcaaggccaccgctaagtacttcttttacagcaatattatgaattttttcaagaccgagattacactggccaatggagagattcggaagcgaccacttatcgaaacaaacggagaaacaggagaaatcgtgtgggacaagggtagggatttcgcgacagtccggaaggtcctgtccatgccgcaggtgaacatcgttaaaaagaccgaagtacagaccggaggcttctccaaggaaagtatcctcccgaaaaggaacagcgacaagctgatcgcacgcaaaaaagattgggaccccaagaaatacggcggattcgattctcctacagtcgcttacagtgtactggttgtggccaaagtggagaaagggaagtctaaaaaactcaaaagcgtcaaggaactgctgggcatcacaatcatggagcgatcaagcttcgaaaaaaaccccatcgactttctcgaggcgaaaggatataaagaggtcaaaaaagacctcatcattaagcttcccaagtactctctctttgagcttgaaaacggccggaaacgaatgctcgctagtgcgggcgagctgcagaaaggtaacgagctggcactgccctctaaatacgttaatttcttgtatctggccagccactatgaaaagctcaaagggtctcccgaagataatgagcagaagcagctgttcgtggaacaacacaaacactaccttgatgagatcatcgagcaaataagcgaattctccaaaagagtgatcctcgccgacgctaacctcgataaggtgctttctgcttacaataagcacagggataagcccatcagggagcaggcagaaaacattatccacttgtttactctgaccaacttgggcgcgcctgcagccttcaagtacttcgacaccaccatagacagaaagcggtacacctctacaaaggaggtcctggacgccacactgattcatcagtcaattacggggctctatgaaacaagaatcgacctctctcagctcggtggagacagcagggctgaccccaagaagaagaggaaggtggctagcgagggcagaggaagtcttctaacatgcggtgacgtggaggagaatcccggccctggtaccgtgagcaagggcgaggagctgttcaccggggtggtgcccatcctggtcgagctggacggcgacgtaaacggccacaagttcagcgtgtccggcgagggcgagggcgatgccacctacggcaagctgaccctgaagttcatctgcaccaccggcaagctgcccgtgccctggcccaccctcgtgaccaccctgacctacggcgtgcagtgcttcagccgctaccccgaccacatgaagcagcacgacttcttcaagtccgccatgcccgaaggctacgtccaggagcgcaccatcttcttcaaggacgacggcaactacaagacccgcgccgaggtgaagttcgagggcgacaccctggtgaaccgcatcgagctgaagggcatcgacttcaaggaggacggcaacatcctggggcacaagctggagtacaactacaacagccacaacgtctatatcatggccgacaagcagaagaacggcatcaaggtgaacttcaagatccgccacaacatcgaggacggcagcgtgcagctcgccgaccactaccagcagaacacccccatcggcgacggccccgtgctgctgcccgacaaccactacctgagcacccagtccgccctgagcaaagaccccaacgagaagcgcgatcacatggtcctgctggagttcgtgaccgccgccgggatcactctcggcatggacgagctgtacaagaccggttag

SEQ ID NO: 146-149 - skipped (4 entries)

SEQ ID NO: 150 - DNA, 23 bp, synthetic construct
  misc_feature 1..23: note = source = /note="Description of Artificial Sequence: Synthetic oligonucleotide"
  source 1..23: mol_type = other DNA
tcctactcagactgttactctgg

SEQ ID NO: 151 - DNA, 23 bp, synthetic construct
  misc_feature 1..23: note = source = /note="Description of Artificial Sequence: Synthetic oligonucleotide"
  source 1..23: mol_type = other DNA
tcctactcacactgttactcagg

SEQ ID NO: 152 - DNA, 23 bp, synthetic construct
  misc_feature 1..23: note = source = /note="Description of Artificial Sequence: Synthetic oligonucleotide"
  source 1..23: mol_type = other DNA
acctgctcacactgttactccag

SEQ ID NO: 153 - DNA, 23 bp, synthetic construct
  misc_feature 1..23: note = source = /note="Description of Artificial Sequence: Synthetic oligonucleotide"
  source 1..23: mol_type = other DNA
gcattctcaaactgttactcagg

SEQ ID NO: 154 - DNA, 23 bp, synthetic construct
  misc_feature 1..23: note = source = /note="Description of Artificial Sequence: Synthetic oligonucleotide"
  source 1..23: mol_type = other DNA
ggattctcacactgttactcggg

SEQ ID NO: 155 - DNA, 23 bp, synthetic construct
  misc_feature 1..23: note = source = /note="Description of Artificial Sequence: Synthetic oligonucleotide"
  source 1..23: mol_type = other DNA
acatacttatactgttactctag

SEQ ID NO: 156 - DNA, 23 bp, synthetic construct
  misc_feature 1..23: note = source = /note="Description of Artificial Sequence: Synthetic oligonucleotide"
  source 1..23: mol_type = other DNA
tattcctaagactgttactcaag

SEQ ID NO: 157 - DNA, 23 bp, synthetic construct
  misc_feature 1..23: note = source = /note="Description of Artificial Sequence: Synthetic oligonucleotide"
  source 1..23: mol_type = other DNA
aaggactaagactgttactcggg

SEQ ID NO: 158 - DNA, 23 bp, synthetic construct
  misc_feature 1..23: note = source = /note="Description of Artificial Sequence: Synthetic oligonucleotide"
  source 1..23: mol_type = other DNA
gagctctcatactgttactctag

SEQ ID NO: 159 - DNA, 23 bp, synthetic construct
  misc_feature 1..23: note = source = /note="Description of Artificial Sequence: Synthetic oligonucleotide"
  source 1..23: mol_type = other DNA
gcaaaatgagactgttactccag

SEQ ID NO: 160 - DNA, 23 bp, synthetic construct
  misc_feature 1..23: note = source = /note="Description of Artificial Sequence: Synthetic oligonucleotide"
  source 1..23: mol_type = other DNA
cctcattcagactgttactcaag

SEQ ID NO: 161 - DNA, 23 bp, synthetic construct
  misc_feature 1..23: note = source = /note="Description of Artificial Sequence: Synthetic oligonucleotide"
  source 1..23: mol_type = other DNA
cattggctttgatttccctaggg

SEQ ID NO: 162 - DNA, 23 bp, synthetic construct
  misc_feature 1..23: note = source = /note="Description of Artificial Sequence: Synthetic oligonucleotide"
  source 1..23: mol_type = other DNA
aattggcattgatttccctagag

SEQ ID NO: 163 - DNA, 23 bp, synthetic construct
  misc_feature 1..23: note = source = /note="Description of Artificial Sequence: Synthetic oligonucleotide"
  source 1..23: mol_type = other DNA
cattggctttaatttccctatag

SEQ ID NO: 164 - DNA, 23 bp, synthetic construct
  misc_feature 1..23: note = source = /note="Description of Artificial Sequence: Synthetic oligonucleotide"
  source 1..23: mol_type = other DNA
gataggctgtgatttccctagag

SEQ ID NO: 165 - DNA, 23 bp, synthetic construct
  misc_feature 1..23: note = source = /note="Description of Artificial Sequence: Synthetic oligonucleotide"
  source 1..23: mol_type = other DNA
gaatagccttgatttccctaaag

SEQ ID NO: 166 - DNA, 23 bp, synthetic construct
  misc_feature 1..23: note = source = /note="Description of Artificial Sequence: Synthetic oligonucleotide"
  source 1..23: mol_type = other DNA
aatttgctttgatttccctgagg

SEQ ID NO: 167 - DNA, 23 bp, synthetic construct
  misc_feature 1..23: note = source = /note="Description of Artificial Sequence: Synthetic oligonucleotide"
  source 1..23: mol_type = other DNA
gatgtgctttgatttcccttggg

SEQ ID NO: 168 - DNA, 23 bp, synthetic construct
  misc_feature 1..23: note = source = /note="Description of Artificial Sequence: Synthetic oligonucleotide"
  source 1..23: mol_type = other DNA
aattggttttaatttccctaaag

SEQ ID NO: 169 - DNA, 23 bp, synthetic construct
  misc_feature 1..23: note = source = /note="Description of Artificial Sequence: Synthetic oligonucleotide"
  source 1..23: mol_type = other DNA
aattgggtttgatttccctttgg

SEQ ID NO: 170 - DNA, 23 bp, synthetic construct
  misc_feature 1..23: note = source = /note="Description of Artificial Sequence: Synthetic oligonucleotide"
  source 1..23: mol_type = other DNA
gatgggtttttatttccctagag

SEQ ID NO: 171 - DNA, 23 bp, synthetic construct
  misc_feature 1..23: note = source = /note="Description of Artificial Sequence: Synthetic oligonucleotide"
  source 1..23: mol_type = other DNA
gaatggttttgatttccctggag

SEQ ID NO: 172 - DNA, 23 bp, synthetic construct
  misc_feature 1..23: note = source = /note="Description of Artificial Sequence: Synthetic oligonucleotide"
  source 1..23: mol_type = other DNA
acagttgcctaagaactggtggg

SEQ ID NO: 173 - DNA, 23 bp, synthetic construct
  misc_feature 1..23: note = source = /note="Description of Artificial Sequence: Synthetic oligonucleotide"
  source 1..23: mol_type = other DNA
ccagttgtctaagaactggggag

SEQ ID NO: 174 - DNA, 23 bp, synthetic construct
  misc_feature 1..23: note = source = /note="Description of Artificial Sequence: Synthetic oligonucleotide"
  source 1..23: mol_type = other DNA
gcagttgcctgtgaactggtagg

SEQ ID NO: 175 - DNA, 23 bp, synthetic construct
  misc_feature 1..23: note = source = /note="Description of Artificial Sequence: Synthetic oligonucleotide"
  source 1..23: mol_type = other DNA
gcagatgcagaagaactggtgag

SEQ ID NO: 176 - DNA, 23 bp, synthetic construct
  misc_feature 1..23: note = source = /note="Description of Artificial Sequence: Synthetic oligonucleotide"
  source 1..23: mol_type = other DNA
gcagttccagaagaactggtgag

SEQ ID NO: 177 - DNA, 23 bp, synthetic construct
  misc_feature 1..23: note = source = /note="Description of Artificial Sequence: Synthetic oligonucleotide"
  source 1..23: mol_type = other DNA
caacttgcctatgaactggtagg

SEQ ID NO: 178 - DNA, 23 bp, synthetic construct
  misc_feature 1..23: note = source = /note="Description of Artificial Sequence: Synthetic oligonucleotide"
  source 1..23: mol_type = other DNA
acacctgcctaagaactggaggg

SEQ ID NO: 179 - DNA, 23 bp, synthetic construct
  misc_feature 1..23: note = source = /note="Description of Artificial Sequence: Synthetic oligonucleotide"
  source 1..23: mol_type = other DNA
tcaggtggctaagaactgggtgg

SEQ ID NO: 180 - DNA, 23 bp, synthetic construct
  misc_feature 1..23: note = source = /note="Description of Artificial Sequence: Synthetic oligonucleotide"
  source 1..23: mol_type = other DNA
gaagttggccaagaactggagag

SEQ ID NO: 181 - DNA, 23 bp, synthetic construct
  misc_feature 1..23: note = source = /note="Description of Artificial Sequence: Synthetic oligonucleotide"
  source 1..23: mol_type = other DNA
gctgctgcccaagaactggcagg

SEQ ID NO: 182 - DNA, 23 bp, synthetic construct
  misc_feature 1..23: note = source = /note="Description of Artificial Sequence: Synthetic oligonucleotide"
  source 1..23: mol_type = other DNA
tcagctggctaagaacgggtaag

SEQ ID NO: 183 - DNA, 23 bp, synthetic construct
  misc_feature 1..23: note = source = /note="Description of Artificial Sequence: Synthetic oligonucleotide"
  source 1..23: mol_type = other DNA
agggctccaccctcacgagtggg

SEQ ID NO: 184 - DNA, 23 bp, synthetic construct
  misc_feature 1..23: note = source = /note="Description of Artificial Sequence: Synthetic oligonucleotide"
  source 1..23: mol_type = other DNA
gcagctcagccctcacgagtcag

SEQ ID NO: 185 - DNA, 23 bp, synthetic construct
  misc_feature 1..23: note = source = /note="Description of Artificial Sequence: Synthetic oligonucleotide"
  source 1..23: mol_type = other DNA
ggggcttcagcatcacgagtgag

SEQ ID NO: 186 - DNA, 23 bp, synthetic construct
  misc_feature 1..23: note = source = /note="Description of Artificial Sequence: Synthetic oligonucleotide"
  source 1..23: mol_type = other DNA
ggggctctcccctcactagtgag

SEQ ID NO: 187 - DNA, 23 bp, synthetic construct
  misc_feature 1..23: note = source = /note="Description of Artificial Sequence: Synthetic oligonucleotide"
  source 1..23: mol_type = other DNA
ggggatccaccttcaccagtcag

SEQ ID NO: 188 - DNA, 23 bp, synthetic construct
  misc_feature 1..23: note = source = /note="Description of Artificial Sequence: Synthetic oligonucleotide"
  source 1..23: mol_type = other DNA
agggctggaccctcacaagtaag

SEQ ID NO: 189 - DNA, 23 bp, synthetic construct
  misc_feature 1..23: note = source = /note="Description of Artificial Sequence: Synthetic oligonucleotide"
  source 1..23: mol_type = other DNA
tggtctcctcccccacgagtggg

SEQ ID NO: 190 - DNA, 23 bp, synthetic construct
  misc_feature 1..23: note = source = /note="Description of Artificial Sequence: Synthetic oligonucleotide"
  source 1..23: mol_type = other DNA
agggctcccaccccacgagtgag

SEQ ID NO: 191 - DNA, 23 bp, synthetic construct
  misc_feature 1..23: note = source = /note="Description of Artificial Sequence: Synthetic oligonucleotide"
  source 1..23: mol_type = other DNA
gaggctccatactcaccagtgag

SEQ ID NO: 192 - DNA, 23 bp, synthetic construct
  misc_feature 1..23: note = source = /note="Description of Artificial Sequence: Synthetic oligonucleotide"
  source 1..23: mol_type = other DNA
ggagctgccccttcacgagtggg

SEQ ID NO: 193 - DNA, 23 bp, synthetic construct
  misc_feature 1..23: note = source = /note="Description of Artificial Sequence: Synthetic oligonucleotide"
  source 1..23: mol_type = other DNA
atgactccaccctcaagagtaag

SEQ ID NO: 194 - DNA, 23 bp, synthetic construct
  misc_feature 1..23: note = source = /note="Description of Artificial Sequence: Synthetic oligonucleotide"
  source 1..23: mol_type = other DNA
gccttctttatcccctatcgagg

SEQ ID NO: 195 - DNA, 23 bp, synthetic construct
  misc_feature 1..23: note = source = /note="Description of Artificial Sequence: Synthetic oligonucleotide"
  source 1..23: mol_type = other DNA
gtctgctgtgtcccctatcgggg

SEQ ID NO: 196 - DNA, 23 bp, synthetic construct
  misc_feature 1..23: note = source = /note="Description of Artificial Sequence: Synthetic oligonucleotide"
  source 1..23: mol_type = other DNA
cccttctctatcccctgtcgtgg

SEQ ID NO: 197 - DNA, 23 bp, synthetic construct
  misc_feature 1..23: note = source = /note="Description of Artificial Sequence: Synthetic oligonucleotide"
  source 1..23: mol_type = other DNA
gccttctttatcccctctcttgg

SEQ ID NO: 198 - DNA, 23 bp, synthetic construct
  misc_feature 1..23: note = source = /note="Description of Artificial Sequence: Synthetic oligonucleotide"
  source 1..23: mol_type = other DNA
gcgctctttttcccctatcttag

SEQ ID NO: 199 - DNA, 23 bp, synthetic construct
  misc_feature 1..23: note = source = /note="Description of Artificial Sequence: Synthetic oligonucleotide"
  source 1..23: mol_type = other DNA
gccctctgtctcccctgtcgcag

SEQ ID NO: 200 - DNA, 23 bp, synthetic construct
  misc_feature 1..23: note = source = /note="Description of Artificial Sequence: Synthetic oligonucleotide"
  source 1..23: mol_type = other DNA
tccatctttgtcccctattgagg

SEQ ID NO: 201 - DNA, 23 bp, synthetic construct
  misc_feature 1..23: note = source = /note="Description of Artificial Sequence: Synthetic oligonucleotide"
  source 1..23: mol_type = other DNA
accttctctctcccctatagagg

SEQ ID NO: 202 - DNA, 23 bp, synthetic construct
  misc_feature 1..23: note = source = /note="Description of Artificial Sequence: Synthetic oligonucleotide"
  source 1..23: mol_type = other DNA
gttttctttttcccctatgggag

SEQ ID NO: 203 - DNA, 23 bp, synthetic construct
  misc_feature 1..23: note = source = /note="Description of Artificial Sequence: Synthetic oligonucleotide"
  source 1..23: mol_type = other DNA
tgcttcttaatcccctatcaaag

SEQ ID NO: 204 - DNA, 23 bp, synthetic construct
  misc_feature 1..23: note = source = /note="Description of Artificial Sequence: Synthetic oligonucleotide"
  source 1..23: mol_type = other DNA
accttcttactcccctatccggg

SEQ ID NO: 205 - DNA, 22 bp, synthetic construct
  misc_feature 1..22: note = source = /note="Description of Artificial Sequence: Synthetic primer"
  source 1..22: mol_type = other DNA
gagaggttatgtggctttacca

SEQ ID NO: 206 - DNA, 20 bp, synthetic construct
  misc_feature 1..20: note = source = /note="Description of Artificial Sequence: Synthetic primer"
  source 1..20: mol_type = other DNA
aaaaatgcttcccactttgc

SEQ ID NO: 207 - DNA, 20 bp, synthetic construct
  misc_feature 1..20: note = source = /note="Description of Artificial Sequence: Synthetic primer"
  source 1..20: mol_type = other DNA
ctcattctcatgcctggaca

SEQ ID NO: 208 - DNA, 25 bp, synthetic construct
  misc_feature 1..25: note = source = /note="Description of Artificial Sequence: Synthetic primer"
  source 1..25: mol_type = other DNA
gagtttggctcaaattgttactctt

SEQ ID NO: 209 - DNA, 25 bp, synthetic construct
  misc_feature 1..25: note = source = /note="Description of Artificial Sequence: Synthetic primer"
  source 1..25: mol_type = other DNA
gggaaatggtctaggagagtaaagt

SEQ ID NO: 210 - DNA, 25 bp, synthetic construct
  misc_feature 1..25: note = source = /note="Description of Artificial Sequence: Synthetic primer"
  source 1..25: mol_type = other DNA
gtttggctcaaattgttactcttca

SEQ ID NO: 211 - DNA, 25 bp, synthetic construct
  misc_feature 1..25: note = source = /note="Description of Artificial Sequence: Synthetic primer"
  source 1..25: mol_type = other DNA
gtgagagtaatgtgtttgctgagag

SEQ ID NO: 212 - DNA, 20 bp, synthetic construct
  misc_feature 1..20: note = source = /note="Description of Artificial Sequence: Synthetic primer"
  source 1..20: mol_type = other DNA
cgggcttggacagaacttac

SEQ ID NO: 213 - DNA, 20 bp, synthetic construct
  misc_feature 1..20: note = source = /note="Description of Artificial Sequence: Synthetic primer"
  source 1..20: mol_type = other DNA
ctgcgtagtgccaaaacaaa

SEQ ID NO: 214 - DNA, 24 bp, synthetic construct
  misc_feature 1..24: note = source = /note="Description of Artificial Sequence: Synthetic primer"
  source 1..24: mol_type = other DNA
taatttcattgaagagtggctgaa

SEQ ID NO: 215 - DNA, 24 bp, synthetic construct
  misc_feature 1..24: note = source = /note="Description of Artificial Sequence: Synthetic primer"
  source 1..24: mol_type = other DNA
aagccctgtgtggtagtagtcagt

SEQ ID NO: 216 - DNA, 24 bp, synthetic construct
  misc_feature 1..24: note = source = /note="Description of Artificial Sequence: Synthetic primer"
  source 1..24: mol_type = other DNA
tgagtcatgttggataaccagtct

SEQ ID NO: 217 - DNA, 24 bp, synthetic construct
  misc_feature 1..24: note = source = /note="Description of Artificial Sequence: Synthetic primer"
  source 1..24: mol_type = other DNA
gaaggtcaggaacatacaattcaa

SEQ ID NO: 218 - DNA, 24 bp, synthetic construct
  misc_feature 1..24: note = source = /note="Description of Artificial Sequence: Synthetic primer"
  source 1..24: mol_type = other DNA
gatatgggcatgtcagtttcatag

SEQ ID NO: 219 - DNA, 24 bp, synthetic construct
  misc_feature 1..24: note = source = /note="Description of Artificial Sequence: Synthetic primer"
  source 1..24: mol_type = other DNA
tgctgttgattaatggttgatagg

SEQ ID NO: 220 - DNA, 23 bp, synthetic construct
  misc_feature 1..23: note = source = /note="Description of Artificial Sequence: Synthetic primer"
  source 1..23: mol_type = other DNA
ttttaaattgccatgtttgtgtc

SEQ ID NO: 221 - DNA, 24 bp, synthetic construct
  misc_feature 1..24: note = source = /note="Description of Artificial Sequence: Synthetic primer"
  source 1..24: mol_type = other DNA
atgaataacctaatgggcagaaaa

SEQ ID NO: 222 - DNA, 24 bp, synthetic construct
  misc_feature 1..24: note = source = /note="Description of Artificial Sequence: Synthetic primer"
  source 1..24: mol_type = other DNA
tcaagtcgcttcattttgatagac

SEQ ID NO: 223 - DNA, 24 bp, synthetic construct
  misc_feature 1..24: note = source = /note="Description of Artificial Sequence: Synthetic primer"
  source 1..24: mol_type = other DNA
cacaacaaaacatatagccaaagc

SEQ ID NO: 224 - DNA, 25 bp, synthetic construct
  misc_feature 1..25: note = source = /note="Description of Artificial Sequence: Synthetic primer"
  source 1..25: mol_type = other DNA
tgctgctaaaataacacaaatcagt

SEQ ID NO: 225 - DNA, 23 bp, synthetic construct
  misc_feature 1..23: note = source = /note="Description of Artificial Sequence: Synthetic primer"
  source 1..23: mol_type = other DNA
ctgtgcctattgtggttatcctg

SEQ ID NO: 226 - DNA, 24 bp, synthetic construct
  misc_feature 1..24: note = source = /note="Description of Artificial Sequence: Synthetic primer"
  source 1..24: mol_type = other DNA
attgatctgcaatacatgtggagt

SEQ ID NO: 227 - DNA, 24 bp, synthetic construct
  misc_feature 1..24: note = source = /note="Description of Artificial Sequence: Synthetic primer"
  source 1..24: mol_type = other DNA
tttgcctctgctattacagtatgg

SEQ ID NO: 228 - DNA, 24 bp, synthetic construct
  misc_feature 1..24: note = source = /note="Description of Artificial Sequence: Synthetic primer"
  source 1..24: mol_type = other DNA
tgtagggtggttggctaaaataat

SEQ ID NO: 229 - DNA, 24 bp, synthetic construct
  misc_feature 1..24: note = source = /note="Description of Artificial Sequence: Synthetic primer"
  source 1..24: mol_type = other DNA
tttttgcacagtcaataacacaaa

SEQ ID NO: 230 - DNA, 24 bp, synthetic construct
  misc_feature 1..24: note = source = /note="Description of Artificial Sequence: Synthetic primer"
  source 1..24: mol_type = other DNA
ggctggtctcacaattgtacttta

SEQ ID NO: 231 - DNA, 24 bp, synthetic construct
  misc_feature 1..24: note = source = /note="Description of Artificial Sequence: Synthetic primer"
  source 1..24: mol_type = other DNA
cattatggactgaaaatctcagca

SEQ ID NO: 232 - DNA, 24 bp, synthetic construct
  misc_feature 1..24: note = source = /note="Description of Artificial Sequence: Synthetic primer"
  source 1..24: mol_type = other DNA
atcatcctagccataacacaatga

SEQ ID NO: 233 - DNA, 24 bp, synthetic construct
  misc_feature 1..24: note = source = /note="Description of Artificial Sequence: Synthetic primer"
  source 1..24: mol_type = other DNA
ttcagctttaacgtgattttctgt

SEQ ID NO: 234 - DNA, 24 bp, synthetic construct
  misc_feature 1..24: note = source = /note="Description of Artificial Sequence: Synthetic primer"
  source 1..24: mol_type = other DNA
ggattcagaagctgtttacgaagt

SEQ ID NO: 235 - DNA, 24 bp, synthetic construct
  misc_feature 1..24: note = source = /note="Description of Artificial Sequence: Synthetic primer"
  source 1..24: mol_type = other DNA
tttagctggattggaaaaacaaat

SEQ ID NO: 236 - DNA, 24 bp, synthetic construct
  misc_feature 1..24: note = source = /note="Description of Artificial Sequence: Synthetic primer"
  source 1..24: mol_type = other DNA
aactcaccccattgttggtatatt

SEQ ID NO: 237 - DNA, 24 bp, synthetic construct
  misc_feature 1..24: note = source = /note="Description of Artificial Sequence: Synthetic primer"
  source 1..24: mol_type = other DNA
ccttgtccaaataccgaaatacat

SEQ ID NO: 238 - DNA, 24 bp, synthetic construct
  misc_feature 1..24: note = source = /note="Description of Artificial Sequence: Synthetic primer"
  source 1..24: mol_type = other DNA
cacataattcatgaacttggcttc

SEQ ID NO: 239 - DNA, 24 bp, synthetic construct
  misc_feature 1..24: note = source = /note="Description of Artificial Sequence: Synthetic primer"
  source 1..24: mol_type = other DNA
tagtagctggggaggaagatacag

SEQ ID NO: 240 - DNA, 24 bp, synthetic construct
  misc_feature 1..24: note = source = /note="Description of Artificial Sequence: Synthetic primer"
  source 1..24: mol_type = other DNA
tttttgttttaattgcgactgtgt

SEQ ID NO: 241 - DNA, 24 bp, synthetic construct
  misc_feature 1..24: note = source = /note="Description of Artificial Sequence: Synthetic primer"
  source 1..24: mol_type = other DNA
agaaaaggggttttcttttgactt

SEQ ID NO: 242 - DNA, 24 bp, synthetic construct
  misc_feature 1..24: note = source = /note="Description of Artificial Sequence: Synthetic primer"
  source 1..24: mol_type = other DNA
cattgtgactggatgagaagaaac

SEQ ID NO: 243 - DNA, 24 bp, synthetic construct
  misc_feature 1..24: note = source = /note="Description of Artificial Sequence: Synthetic primer"
  source 1..24: mol_type = other DNA
aacggctgttattaaagtcctcag

SEQ ID NO: 244 - DNA, 24 bp, synthetic construct
  misc_feature 1..24: note = source = /note="Description of Artificial Sequence: Synthetic primer"
  source 1..24: mol_type = other DNA
caagtcagaagtcacttgctttgt

SEQ ID NO: 245 - DNA, 24 bp, synthetic construct
  misc_feature 1..24: note = source = /note="Description of Artificial Sequence: Synthetic primer"
  source 1..24: mol_type = other DNA
ttttatgtgcaggaatcagtctgt

SEQ ID NO: 246 - DNA, 18 bp, synthetic construct
  misc_feature 1..18: note = source = /note="Description of Artificial Sequence: Synthetic primer"
  source 1..18: mol_type = other DNA
tggcggcgttttcattat

SEQ ID NO: 247 - DNA, 26 bp, synthetic construct
  misc_feature 1..26: note = source = /note="Description of Artificial Sequence: Synthetic primer"
  source 1..26: mol_type = other DNA
ttcgatccgtaatgattgttctagcc

SEQ ID NO: 248 - DNA, 20 bp, synthetic construct
  misc_feature 1..20: note = source = /note="Description of Artificial Sequence: Synthetic primer"
  source 1..20: mol_type = other DNA
ggtcttccagagtgctgagg

SEQ ID NO: 249 - DNA, 24 bp, synthetic construct
  misc_feature 1..24: note = source = /note="Description of Artificial Sequence: Synthetic primer"
  source 1..24: mol_type = other DNA
tgtgtgcttctgtacacatcatct

SEQ ID NO: 250 - DNA, 24 bp, synthetic construct
  misc_feature 1..24: note = source = /note="Description of Artificial Sequence: Synthetic primer"
  source 1..24: mol_type = other DNA
agatttcaaccctcaaaaactgag

SEQ ID NO: 251 - DNA, 24 bp, synthetic construct
  misc_feature 1..24: note = source = /note="Description of Artificial Sequence: Synthetic primer"
  source 1..24: mol_type = other DNA
taaactctttcttttccgcaattc

SEQ ID NO: 252 - DNA, 24 bp, synthetic construct
  misc_feature 1..24: note = source = /note="Description of Artificial Sequence: Synthetic primer"
  source 1..24: mol_type = other DNA
caaggtgacctgctacctaaaaat

SEQ ID NO: 253 - DNA, 24 bp, synthetic construct
  misc_feature 1..24: note = source = /note="Description of Artificial Sequence: Synthetic primer"
  source 1..24: mol_type = other DNA
tatgaccaaggctatgtgttcact

SEQ ID NO: 254 - DNA, 24 bp, synthetic construct
  misc_feature 1..24: note = source = /note="Description of Artificial Sequence: Synthetic primer"
  source 1..24: mol_type = other DNA
acagcctctctccagtaacattct

SEQ ID NO: 255 - DNA, 24 bp, synthetic construct
  misc_feature 1..24: note = source = /note="Description of Artificial Sequence: Synthetic primer"
  source 1..24: mol_type = other DNA
tattcttgcagtggtttcacattt

SEQ ID NO: 256 - DNA, 24 bp, synthetic construct
  misc_feature 1..24: note = source = /note="Description of Artificial Sequence: Synthetic primer"
  source 1..24: mol_type = other DNA
atattttaagccaagacccaacaa

SEQ ID NO: 257 - DNA, 24 bp, synthetic construct
  misc_feature 1..24: note = source = /note="Description of Artificial Sequence: Synthetic primer"
  source 1..24: mol_type = other DNA
ctttcaactgtctgtctgattgct

SEQ ID NO: 258 - DNA, 24 bp, synthetic construct
  misc_feature 1..24: note = source = /note="Description of Artificial Sequence: Synthetic primer"
  source 1..24: mol_type = other DNA
aacagcctctcttcattgttctct

SEQ ID NO: 259 - DNA, 24 bp, synthetic construct
  misc_feature 1..24: note = source = /note="Description of Artificial Sequence: Synthetic primer"
  source 1..24: mol_type = other DNA
ctctggaacttgtctctgtcttga

SEQ ID NO: 260 - DNA, 24 bp, synthetic construct
  misc_feature 1..24: note = source = /note="Description of Artificial Sequence: Synthetic primer"
  source 1..24: mol_type = other DNA
ctttcctgcgttctcatgttacta

SEQ ID NO: 261 - DNA, 24 bp, synthetic construct
  misc_feature 1..24: note = source = /note="Description of Artificial Sequence: Synthetic primer"
  source 1..24: mol_type = other DNA
ccttatatccgtatcgctcactct

SEQ ID NO: 262 - DNA, 24 bp, synthetic construct
  misc_feature 1..24: note = source = /note="Description of Artificial Sequence: Synthetic primer"
  source 1..24: mol_type = other DNA
catatctgtctaacttccgcacac

SEQ ID NO: 263 - DNA, 24 bp, synthetic construct
  misc_feature 1..24: note = source = /note="Description of Artificial Sequence: Synthetic primer"
  source 1..24: mol_type = other DNA
acaggtgttatgttgtctgcatct

SEQ ID NO: 264 - DNA, 24 bp, synthetic construct
  misc_feature 1..24: note = source = /note="Description of Artificial Sequence: Synthetic primer"
  source 1..24: mol_type = other DNA
actccattcccagattagttatgc

SEQ ID NO: 265 - DNA, 24 bp, synthetic construct
  misc_feature 1..24: note = source = /note="Description of Artificial Sequence: Synthetic primer"
  source 1..24: mol_type = other DNA
ctgttttctttgtgagagtggaga

SEQ ID NO: 266 - DNA, 24 bp, synthetic construct
  misc_feature 1..24: note = source = /note="Description of Artificial Sequence: Synthetic primer"
  source 1..24: mol_type = other DNA
tgtaaggtggtcaaacttgctcta

SEQ ID NO: 267 - DNA, 25 bp, synthetic construct
  misc_feature 1..25: note = source = /note="Description of Artificial Sequence: Synthetic primer"
  source 1..25: mol_type = other DNA
tttttcctagtacccacagattttt

SEQ ID NO: 268 - DNA, 24 bp, synthetic construct
  misc_feature 1..24: note = source = /note="Description of Artificial Sequence: Synthetic primer"
  source 1..24: mol_type = other DNA
tccctgattctctcatttgtgtta

SEQ ID NO: 269 - DNA, 24 bp, synthetic construct
  misc_feature 1..24: note = source = /note="Description of Artificial Sequence: Synthetic primer"
  source 1..24: mol_type = other DNA
ttgggaacatcagagaaagtatga

SEQ ID NO: 270 - DNA, 24 bp, synthetic construct
  misc_feature 1..24: note = source = /note="Description of Artificial Sequence: Synthetic primer"
  source 1..24: mol_type = other DNA
acaaattacagtctcctgggaaag

SEQ ID NO: 271 - DNA, 24 bp, synthetic construct
  misc_feature 1..24: note = source = /note="Description of Artificial Sequence: Synthetic primer"
  source 1..24: mol_type = other DNA
agtagcttaccttggcagagaaaa

SEQ ID NO: 272 - DNA, 24 bp, synthetic construct
  misc_feature 1..24: note = source = /note="Description of Artificial Sequence: Synthetic primer"
  source 1..24: mol_type = other DNA
tgacatactgttaccctttgcagt

SEQ ID NO: 273 - DNA, 23 bp, synthetic construct
  misc_feature 1..23: note = source = /note="Description of Artificial Sequence: Synthetic primer"
  source 1..23: mol_type = other DNA
gaaaggctcagtgaatgtttgtt

SEQ ID NO: 274 - DNA, 24 bp, synthetic construct
  misc_feature 1..24: note = source = /note="Description of Artificial Sequence: Synthetic primer"
  source 1..24: mol_type = other DNA
cactgcatcatctcattaaatcaa

SEQ ID NO: 275 - DNA, 24 bp, synthetic construct
  misc_feature 1..24: note = source = /note="Description of Artificial Sequence: Synthetic primer"
  source 1..24: mol_type = other DNA
cccatatattcatgattacccaca

SEQ ID NO: 276 - DNA, 24 bp, synthetic construct
  misc_feature 1..24: note = source = /note="Description of Artificial Sequence: Synthetic primer"
  source 1..24: mol_type = other DNA
tatcagaacgagcactaaaagcac

SEQ ID NO: 277 - DNA, 20 bp, synthetic construct
  misc_feature 1..20: note = source = /note="Description of Artificial Sequence: Synthetic primer"
  source 1..20: mol_type = other DNA
ttgggaggctgaggtacaag

SEQ ID NO: 278 - DNA, 24 bp, synthetic construct
  misc_feature 1..24: note = source = /note="Description of Artificial Sequence: Synthetic primer"
  source 1..24: mol_type = other DNA
gaatgaaaaacaaacagaaggtga

SEQ ID NO: 279 - DNA, 24 bp, synthetic construct
  misc_feature 1..24: note = source = /note="Description of Artificial Sequence: Synthetic primer"
  source 1..24: mol_type = other DNA
ctcctcatctgtacccttcaatct

SEQ ID NO: 280 - DNA, 24 bp, synthetic construct
  misc_feature 1..24: note = source = /note="Description of Artificial Sequence: Synthetic primer"
  source 1..24: mol_type = other DNA
agagtggcatctagtgtcagtgag

SEQ ID NO: 281 - DNA, 24 bp, synthetic construct
  misc_feature 1..24: note = source = /note="Description of Artificial Sequence: Synthetic primer"
  source 1..24: mol_type = other DNA
taccaaaagcttctcctgtttacc

SEQ ID NO: 282 - DNA, 24 bp, synthetic construct
  misc_feature 1..24: note = source = /note="Description of Artificial Sequence: Synthetic primer"
  source 1..24: mol_type = other DNA
gtaagttggatggcctattctttg

SEQ ID NO: 283 - DNA, 24 bp, synthetic construct
  misc_feature 1..24: note = source = /note="Description of Artificial Sequence: Synthetic primer"
  source 1..24: mol_type = other DNA
gaaggaaatgcaaggatacaagat

SEQ ID NO: 284 - DNA, 24 bp, synthetic construct
  misc_feature 1..24: note = source = /note="Description of Artificial Sequence: Synthetic primer"
  source 1..24: mol_type = other DNA
tgattgaaagaatcattccagaaa

SEQ ID NO: 285 - DNA, 24 bp, synthetic construct
  misc_feature 1..24: note = source = /note="Description of Artificial Sequence: Synthetic primer"
  source 1..24: mol_type = other DNA
tcagaaggaaaattgaaattggtt

SEQ ID NO: 286 - DNA, 24 bp, synthetic construct
  misc_feature 1..24: note = source = /note="Description of Artificial Sequence: Synthetic primer"
  source 1..24: mol_type = other DNA
cagatgtgttcttcatcattcctc

SEQ ID NO: 287 - DNA, 24 bp, synthetic construct
  misc_feature 1..24: note = source = /note="Description of Artificial Sequence: Synthetic primer"
  source 1..24: mol_type = other DNA
ttctctttagggaaagctctcaaa

SEQ ID NO: 288 - DNA, 24 bp, synthetic construct
  misc_feature 1..24: note = source = /note="Description of Artificial Sequence: Synthetic primer"
  source 1..24: mol_type = other DNA
gggtatagatcatatggagggaag

SEQ ID NO: 289 - DNA, 20 bp, synthetic construct
  misc_feature 1..20: note = source = /note="Description of Artificial Sequence: Synthetic primer"
  source 1..20: mol_type = other DNA
agatgatctgcccacctcag

SEQ ID NO: 290 - DNA, 24 bp, synthetic construct
  misc_feature 1..24: note = source = /note="Description of Artificial Sequence: Synthetic primer"
  source 1..24: mol_type = other DNA
ctttcttcctcatttagtggcaat

SEQ ID NO: 291 - DNA, 24 bp, synthetic construct
  misc_feature 1..24: note = source = /note="Description of Artificial Sequence: Synthetic primer"
  source 1..24: mol_type = other DNA
atgaattgcagattgatggtactg

SEQ ID NO: 292 - DNA, 24 bp, synthetic construct
  misc_feature 1..24: note = source = /note="Description of Artificial Sequence: Synthetic primer"
  source 1..24: mol_type = other DNA
tctcaccaagaaccaaattgtcta

SEQ ID NO: 293 - DNA, 24 bp, synthetic construct
  misc_feature 1..24: note = source = /note="Description of Artificial Sequence: Synthetic primer"
  source 1..24: mol_type = other DNA
gtaggataccttggcaacagtctt

SEQ ID NO: 294 - DNA, 24 bp, synthetic construct
  misc_feature 1..24: note = source = /note="Description of Artificial Sequence: Synthetic primer"
  source 1..24: mol_type = other DNA
ttaacgaattgtgagatttgctgt

SEQ ID NO: 295 - DNA, 24 bp, synthetic construct
  misc_feature 1..24: note = source = /note="Description of Artificial Sequence: Synthetic primer"
  source 1..24: mol_type = other DNA
tcagaaagtcaagtagcacacaca

SEQ ID NO: 296 - DNA, 23 bp, synthetic construct
  misc_feature 1..23: note = source = /note="Description of Artificial Sequence: Synthetic primer"
  source 1..23: mol_type = other DNA
agaagcacacactcaggtaaagc

SEQ ID NO: 297 - DNA, 24 bp, synthetic construct
  misc_feature 1..24: note = source = /note="Description of Artificial Sequence: Synthetic primer"
  source 1..24: mol_type = other DNA
tctttgggggaataatgactaaaa

SEQ ID NO: 298 - DNA, 24 bp, synthetic construct
  misc_feature 1..24: note = source = /note="Description of Artificial Sequence: Synthetic primer"
  source 1..24: mol_type = other DNA
tttggcatttatgggaataaaact

SEQ ID NO: 299 - DNA, 23 bp, synthetic construct
  misc_feature 1..23: note = source = /note="Description of Artificial Sequence: Synthetic primer"
  source 1..23: mol_type = other DNA
actaattctggtcaagcccatca

SEQ ID NO: 300 - DNA, 24 bp, synthetic construct
  misc_feature 1..24: note = source = /note="Description of Artificial Sequence: Synthetic primer"
  source 1..24: mol_type = other DNA
ttaagacatcggatgaacagaaag

SEQ ID NO: 301 - DNA, 23 bp, synthetic construct
  misc_feature 1..23: note = source = /note="Description of Artificial Sequence: Synthetic primer"
  source 1..23: mol_type = other DNA
agaagctttctgacatgatctgc

SEQ ID NO: 302 - DNA, 24 bp, synthetic construct
  misc_feature 1..24: note = source = /note="Description of Artificial Sequence: Synthetic primer"
  source 1..24: mol_type = other DNA
tcaattgcattaggacttagacca

SEQ ID NO: 303 - DNA, 24 bp, synthetic construct
  misc_feature 1..24: note = source = /note="Description of Artificial Sequence: Synthetic primer"
  source 1..24: mol_type = other DNA
gttaaattacctgtgaagcccttg

SEQ ID NO: 304 - DNA, 24 bp, synthetic construct
  misc_feature 1..24: note = source = /note="Description of Artificial Sequence: Synthetic primer"
  source 1..24: mol_type = other DNA
cggaaaacagatccactttatgat

SEQ ID NO: 305 - DNA, 24 bp, synthetic construct
  misc_feature 1..24: note = source = /note="Description of Artificial Sequence: Synthetic primer"
  source 1..24: mol_type = other DNA
aaatccactggaaacatcttgagt

SEQ ID NO: 306 - DNA, 24 bp, synthetic construct
  misc_feature 1..24: note = source = /note="Description of Artificial Sequence: Synthetic primer"
  source 1..24: mol_type = other DNA
agtctcttcagaatcatgccctat

SEQ ID NO: 307 - DNA, 22 bp, synthetic construct
  misc_feature 1..22: note = source = /note="Description of Artificial Sequence: Synthetic primer"
  source 1..22: mol_type = other DNA
gcttggtggcacatacctgtag

SEQ ID NO: 308 - DNA, 24 bp, synthetic construct
  misc_feature 1..24: note = source = /note="Description of Artificial Sequence: Synthetic primer"
  source 1..24: mol_type = other DNA
ggtaggtagatttgcttgcttgtt

SEQ ID NO: 309 - DNA, 24 bp, synthetic construct
  misc_feature 1..24: note = source = /note="Description of Artificial Sequence: Synthetic primer"
  source 1..24: mol_type = other DNA
agctctcagcagagtagggattta

SEQ ID NO: 310 - DNA, 21 bp, synthetic construct
  misc_feature 1..21: note = source = /note="Description of Artificial Sequence: Synthetic primer"
  source 1..21: mol_type = other DNA
gtgagtctactgcaccccatc

SEQ ID NO: 311 - DNA, 24 bp, synthetic construct
  misc_feature 1..24: note = source = /note="Description of Artificial Sequence: Synthetic primer"
  source 1..24: mol_type = other DNA
tgacactgtgaagtcaattctgtc

SEQ ID NO: 312 - DNA, 24 bp, synthetic construct
  misc_feature 1..24: note = source = /note="Description of Artificial Sequence: Synthetic primer"
  source 1..24: mol_type = other DNA
tcaagaacttgacaatgagcaaat

SEQ ID NO: 313 - DNA, 22 bp, synthetic construct
  misc_feature 1..22: note = source = /note="Description of Artificial Sequence: Synthetic primer"
  source 1..22: mol_type = other DNA
tatccgatccactgttgtgtgt

SEQ ID NO: 314 - DNA, 23 bp, synthetic construct
  misc_feature 1..23: note = source = /note="Description of Artificial Sequence: Synthetic primer"
  source 1..23: mol_type = other DNA
caggagacccaaaaccactctac

SEQ ID NO: 315 - DNA, 24 bp, synthetic construct
  misc_feature 1..24: note = source = /note="Description of Artificial Sequence: Synthetic primer"
  source 1..24: mol_type = other DNA
ttgttctacaaatagggcttcctt

SEQ ID NO: 316 - DNA, 24 bp, synthetic construct
  misc_feature 1..24: note = source = /note="Description of Artificial Sequence: Synthetic primer"
  source 1..24: mol_type = other DNA
tgttaagtttgggcttatgttcct

SEQ ID NO: 317 - DNA, 23 bp, synthetic construct
  misc_feature 1..23: note = source = /note="Description of Artificial Sequence: Synthetic primer"
  source 1..23: mol_type = other DNA
cacaagtctcactgcacaaacat

SEQ ID NO: 318 - DNA, 24 bp, synthetic construct
  misc_feature 1..24: note = source = /note="Description of Artificial Sequence: Synthetic primer"
  source 1..24: mol_type = other DNA
tgacccatgattatctctctttga

SEQ ID NO: 319 - DNA, 24 bp, synthetic construct
  misc_feature 1..24: note = source = /note="Description of Artificial Sequence: Synthetic primer"
  source 1..24: mol_type = other DNA
ttcagcttctgattggttttaatg

SEQ ID NO: 320 - DNA, 24 bp, synthetic construct
  misc_feature 1..24: note = source = /note="Description of Artificial Sequence: Synthetic primer"
  source 1..24: mol_type = other DNA
ccaattccttaattttccctacag

SEQ ID NO: 321 - DNA, 21 bp, synthetic construct
  misc_feature 1..21: note = source = /note="Description of Artificial Sequence: Synthetic primer"
  source 1..21: mol_type = other DNA
atctcagaccaggagggagac

SEQ ID NO: 322 - DNA, 24 bp, synthetic construct
  misc_feature 1..24: note = source = /note="Description of Artificial Sequence: Synthetic primer"
  source 1..24: mol_type = other DNA
cctcagggtcagtacatttttcag

SEQ ID NO: 323 - DNA, 24 bp, synthetic construct
  misc_feature 1..24: note = source = /note="Description of Artificial Sequence: Synthetic primer"
  source 1..24: mol_type = other DNA
ttcttaggacattgctccacatac

SEQ ID NO: 324 - DNA, 24 bp, synthetic construct
  misc_feature 1..24: note = source = /note="Description of Artificial Sequence: Synthetic primer"
  source 1..24: mol_type = other DNA
gcaaacataatgcaactcgtaatc

SEQ ID NO: 325 - DNA, 21 bp, synthetic construct
  misc_feature 1..21: note = source = /note="Description of Artificial Sequence: Synthetic primer"
  source 1..21: mol_type = other DNA
gcaagggagtctgtgtctttg

SEQ ID NO: 326 - DNA, 24 bp, synthetic construct
  misc_feature 1..24: note = source = /note="Description of Artificial Sequence: Synthetic primer"
  source 1..24: mol_type = other DNA
tcatttaagtggctgttctgtgtt

SEQ ID NO: 327 - DNA, 24 bp, synthetic construct
  misc_feature 1..24: note = source = /note="Description of Artificial Sequence: Synthetic primer"
  source 1..24: mol_type = other DNA
acaaaacagagagaaaaggcagag

SEQ ID NO: 328 - DNA, 23 bp, synthetic construct
  misc_feature 1..23: note = source = /note="Description of Artificial Sequence: Synthetic primer"
  source 1..23: mol_type = other DNA
gttttgatttctggtgcctacag

SEQ ID NO: 329 - DNA, 20 bp, synthetic construct
  misc_feature 1..20: note = source = /note="Description of Artificial Sequence: Synthetic primer"
  source 1..20: mol_type = other DNA
actgaagctgaagcccagtc

SEQ ID NO: 330 - DNA, 23 bp, synthetic construct
  misc_feature 1..23: note = source = /note="Description of Artificial Sequence: Synthetic primer"
  source 1..23: mol_type = other DNA
acatgagctctcaggtttctgac

SEQ ID NO: 331 - DNA, 25 bp, synthetic construct
  misc_feature 1..25: note = source = /note="Description of Artificial Sequence: Synthetic primer"
  source 1..25: mol_type = other DNA
tcaaacttagatggttccctatgtt

SEQ ID NO: 332 - DNA, 24 bp, synthetic construct
  misc_feature 1..24: note = source = /note="Description of Artificial Sequence: Synthetic primer"
  source 1..24: mol_type = other DNA
gtaccctgaaaatgtagggtgact

SEQ ID NO: 333 - DNA, 20 bp, synthetic construct
  misc_feature 1..20: note = source = /note="Description of Artificial Sequence: Synthetic primer"
  source 1..20: mol_type = other DNA
cacttcccaagtgaggcaat

SEQ ID NO: 334 - DNA, 24 bp, synthetic construct
  misc_feature 1..24: note = source = /note="Description of Artificial Sequence: Synthetic primer"
  source 1..24: mol_type = other DNA
ctatacttggggctgacttgctac

SEQ ID NO: 335 - DNA, 24 bp, synthetic construct
  misc_feature 1..24: note = source = /note="Description of Artificial Sequence: Synthetic primer"
  source 1..24: mol_type = other DNA
tcgtataggttactttggctcaca

SEQ ID NO: 336 - DNA, 24 bp, synthetic construct
  misc_feature 1..24: note = source = /note="Description of Artificial Sequence: Synthetic primer"
  source 1..24: mol_type = other DNA
agggatctttactcctcagtgtgt

SEQ ID NO: 337 - DNA, 24 bp, synthetic construct
  misc_feature 1..24: note = source = /note="Description of Artificial Sequence: Synthetic primer"
  source 1..24: mol_type = other DNA
tgtagaagttggaatatcctgctg

SEQ ID NO: 338 - DNA, 24 bp, synthetic construct
  misc_feature 1..24: note = source = /note="Description of Artificial Sequence: Synthetic primer"
  source 1..24: mol_type = other DNA
gtcaacaatttgatctcaggcttc

SEQ ID NO: 339 - DNA, 24 bp, synthetic construct
  misc_feature 1..24: note = source = /note="Description of Artificial Sequence: Synthetic primer"
  source 1..24: mol_type = other DNA
ctcagtactaaagatggacgcttg

SEQ ID NO: 340 - DNA, 24 bp, synthetic construct
  misc_feature 1..24: note = source = /note="Description of Artificial Sequence: Synthetic primer"
  source 1..24: mol_type = other DNA
aatcatttcagtcttcccaacaat

SEQ ID NO: 341 - DNA, 24 bp, synthetic construct
  misc_feature 1..24: note = source = /note="Description of Artificial Sequence: Synthetic primer"
  source 1..24: mol_type = other DNA
gggaatcacagtagatgtttgtca

SEQ ID NO: 342 - DNA, 24 bp, synthetic construct
  misc_feature 1..24: note = source = /note="Description of Artificial Sequence: Synthetic primer"
  source 1..24: mol_type = other DNA
agaccaggaggtaagaacattttg

SEQ ID NO: 343 - DNA, 24 bp, synthetic construct
  misc_feature 1..24: note = source = /note="Description of Artificial Sequence: Synthetic primer"
  source 1..24: mol_type = other DNA
ccacatagaaagagacttgcagaa

SEQ ID NO: 344 - DNA, 24 bp, synthetic construct
  misc_feature 1..24: note = source = /note="Description of Artificial Sequence: Synthetic primer"
  source 1..24: mol_type = other DNA
agagatgccaaaagaacagtcaat

SEQ ID NO: 345 - DNA, 24 bp, synthetic construct
  misc_feature 1..24: note = source = /note="Description of Artificial Sequence: Synthetic primer"
  source 1..24: mol_type = other DNA
tgtgccttaggctatgtaaactgt

SEQ ID NO: 346 - DNA, 24 bp, synthetic construct
  misc_feature 1..24: note = source = /note="Description of Artificial Sequence: Synthetic primer"
  source 1..24: mol_type = other DNA
aaacccttgtaaccaaaattacca

SEQ ID NO: 347 - DNA, 24 bp, synthetic construct
  misc_feature 1..24: note = source = /note="Description of Artificial Sequence: Synthetic primer"
  source 1..24: mol_type = other DNA
taactgcatcagaagtccttgcta

SEQ ID NO: 348 - DNA, 22 bp, synthetic construct
  misc_feature 1..22: note = source = /note="Description of Artificial Sequence: Synthetic primer"
  source 1..22: mol_type = other DNA
ggagaccaagctgctaaagtca

SEQ ID NO: 349 - DNA, 37 bp, synthetic construct
  misc_feature 1..37: note = source = /note="Description of Artificial Sequence: Synthetic primer"
  source 1..37: mol_type = other DNA
gtggtgccgcgggagtttggctcaaattgttactctt

SEQ ID NO: 350 - DNA, 37 bp, synthetic construct
  misc_feature 1..37: note = source = /note="Description of Artificial Sequence: Synthetic primer"
  source 1..37: mol_type = other DNA
gtggtgccgcgggggaaatggtctaggagagtaaagt

SEQ ID NO: 351 - DNA, 34 bp, synthetic construct
  misc_feature 1..34: note = source = /note="Description of Artificial Sequence: Synthetic primer"
  source 1..34: mol_type = other DNA
gtggtgccgcgggagaggttatgtggctttacca

SEQ ID NO: 352 - DNA, 32 bp, synthetic construct
  misc_feature 1..32: note = source = /note="Description of Artificial Sequence: Synthetic primer"
  source 1..32: mol_type = other DNA
gtggtgccgcggctcattctcatgcctggaca

SEQ ID NO: 353 - DNA, 32 bp, synthetic construct
  misc_feature 1..32: note = source = /note="Description of Artificial Sequence: Synthetic primer"
  source 1..32: mol_type = other DNA
gtggtgccgcggcgggcttggacagaacttac

SEQ ID NO: 354 - DNA, 32 bp, synthetic construct
  misc_feature 1..32: note = source = /note="Description of Artificial Sequence: Synthetic primer"
  source 1..32: mol_type = other DNA
gtggtgccgcggctgcgtagtgccaaaacaaa

SEQ ID NO: 355 - DNA, 36 bp, synthetic construct
  misc_feature 1..36: note = source = /note="Description of Artificial Sequence: Synthetic primer"
  source 1..36: mol_type = other DNA
gtggtgccgcggtaatttcattgaagagtggctgaa

SEQ ID NO: 356 - DNA, 36 bp, synthetic construct
  misc_feature 1..36: note = source = /note="Description of Artificial Sequence: Synthetic primer"
  source 1..36: mol_type = other DNA
gtggtgccgcggaagccctgtgtggtagtagtcagt

SEQ ID NO: 357 - DNA, 36 bp, synthetic construct
  misc_feature 1..36: note = source = /note="Description of Artificial Sequence: Synthetic primer"
  source 1..36: mol_type = other DNA
gtggtgccgcggcaagtcagaagtcacttgctttgt

SEQ ID NO: 358 - DNA, 36 bp, synthetic construct
  misc_feature 1..36: note = source = /note="Description of Artificial Sequence: Synthetic primer"
  source 1..36: mol_type = other DNA
gtggtgccgcggttttatgtgcaggaatcagtctgt

SEQ ID NO: 359 - DNA, 36 bp, synthetic construct
  misc_feature 1..36: note = source = /note="Description of Artificial Sequence: Synthetic primer"
  source 1..36: mol_type = other DNA
gtggtgccgcggtgtgtgcttctgtacacatcatct

SEQ ID NO: 360 - DNA, 36 bp, synthetic construct
  misc_feature 1..36: note = source = /note="Description of Artificial Sequence: Synthetic primer"
  source 1..36: mol_type = other DNA
gtggtgccgcggagatttcaaccctcaaaaactgag

SEQ ID NO: 361 - DNA, 36 bp, synthetic construct
  misc_feature 1..36: note = source = /note="Description of Artificial Sequence: Synthetic primer"
  source 1..36: mol_type = other DNA
gtggtgccgcggttgggaacatcagagaaagtatga

SEQ ID NO: 362 - DNA, 36 bp, synthetic construct
  misc_feature 1..36: note = source = /note="Description of Artificial Sequence: Synthetic primer"
  source 1..36: mol_type = other DNA
gtggtgccgcggacaaattacagtctcctgggaaag

SEQ ID NO: 363 - DNA, 32 bp, synthetic construct
  misc_feature 1..32: note = source = /note="Description of Artificial Sequence: Synthetic primer"
  source 1..32: mol_type = other DNA
gtggtgccgcggcacttcccaagtgaggcaat

SEQ ID NO: 364 - DNA, 36 bp, synthetic construct
  misc_feature 1..36: note = source = /note="Description of Artificial Sequence: Synthetic primer"
  source 1..36: mol_type = other DNA
gtggtgccgcggctatacttggggctgacttgctac

SEQ ID NO: 365 - DNA, 34 bp, synthetic construct
  misc_feature 1..34: note = source = /note="Description of Artificial Sequence: Synthetic primer"
  source 1..34: mol_type = other DNA
gtggtgccgcggttggctctttagcttgtgtttc

SEQ ID NO: 366 - DNA, 32 bp, synthetic construct
  misc_feature 1..32: note = source = /note="Description of Artificial Sequence: Synthetic primer"
  source 1..32: mol_type = other DNA
gtggtgccgcggtgagactcccaaaggcaatc

SEQ ID NO: 367 - DNA, 34 bp, synthetic construct; identical to SEQ ID NO: 365
  misc_feature 1..34: note = source = /note="Description of Artificial Sequence: Synthetic primer"
  source 1..34: mol_type = other DNA

SEQ ID NO: 368 - DNA, 32 bp, synthetic construct
  misc_feature 1..32: note = source = /note="Description of Artificial Sequence: Synthetic primer"
  source 1..32: mol_type = other DNA
gtggtgccgcggactgaggggtgatcttggtg

SEQ ID NO: 369 - DNA, 32 bp, synthetic construct
  misc_feature 1..32: note = source = /note="Description of Artificial Sequence: Synthetic primer"
  source 1..32: mol_type = other DNA
gtggtgccgcgggcagagaaagccagtcggta

SEQ ID NO: 370 - DNA, 32 bp, synthetic construct; identical to SEQ ID NO: 366
  misc_feature 1..32: note = source = /note="Description of Artificial Sequence: Synthetic primer"
  source 1..32: mol_type = other DNA

SEQ ID NO: 371 - DNA, 32 bp, synthetic construct; identical to SEQ ID NO: 369
  misc_feature 1..32: note = source = /note="Description of Artificial Sequence: Synthetic primer"
  source 1..32: mol_type = other DNA

SEQ ID NO: 372 - DNA, 32 bp, synthetic construct; identical to SEQ ID NO: 368
  misc_feature 1..32: note = source = /note="Description of Artificial Sequence: Synthetic primer"
  source 1..32: mol_type = other DNA

SEQ ID NO: 373 - DNA, 32 bp, synthetic construct
  misc_feature 1..32: note = source = /note="Description of Artificial Sequence: Synthetic primer"
  source 1..32: mol_type = other DNA
gtggtgccgcggccagagttcctagggcagag

SEQ ID NO: 374 - DNA, 32 bp, synthetic construct
  misc_feature 1..32: note = source = /note="Description of Artificial Sequence: Synthetic primer"
  source 1..32: mol_type = other DNA
gtggtgccgcggagctagtccccacattccac

SEQ ID NO: 375 - DNA, 32 bp, synthetic construct; identical to SEQ ID NO: 373
  misc_feature 1..32: note = source = /note="Description of Artificial Sequence: Synthetic primer"
  source 1..32: mol_type = other DNA

SEQ ID NO: 376 - DNA, 32 bp, synthetic construct
  misc_feature 1..32: note = source = /note="Description of Artificial Sequence: Synthetic primer"
  source 1..32: mol_type = other DNA
gtggtgccgcggggtggagggaaactttaggc

SEQ ID NO: 377 - DNA, 32 bp, synthetic construct; identical to SEQ ID NO: 352
  misc_feature 1..32: note = source = /note="Description of Artificial Sequence: Synthetic primer"
  source 1..32: mol_type = other DNA

SEQ ID NO: 378 - DNA, 32 bp, synthetic construct; identical to SEQ ID NO: 374
  misc_feature 1..32: note = source = /note="Description of Artificial Sequence: Synthetic primer"
  source 1..32: mol_type = other DNA

SEQ ID NO: 379 - DNA, 34 bp, synthetic construct
  misc_feature 1..34: note = source = /note="Description of Artificial Sequence: Synthetic primer"
  source 1..34: mol_type = other DNA
gtggtgccgcggtctcatgcctggacaagtaact

SEQ ID NO: 380 - DNA, 32 bp, synthetic construct; identical to SEQ ID NO: 376
  misc_feature 1..32: note = source = /note="Description of Artificial Sequence: Synthetic primer"
  source 1..32: mol_type = other DNA

SEQ ID NO: 381 - DNA, 32 bp, synthetic construct
  misc_feature 1..32: note = source = /note="Description of Artificial Sequence: Synthetic primer"
  source 1..32: mol_type = other DNA
gtggtgccgcggggcttggacagaacttaccg

SEQ ID NO: 382 - DNA, 32 bp, synthetic construct
  misc_feature 1..32: note = source = /note="Description of Artificial Sequence: Synthetic primer"
  source 1..32: mol_type = other DNA
gtggtgccgcggcaccactgtctgcctaagga

SEQ ID NO: 383 - DNA, 32 bp, synthetic construct; identical to SEQ ID NO: 381
  misc_feature 1..32: note = source = /note="Description of Artificial Sequence: Synthetic primer"
  source 1..32: mol_type = other DNA

SEQ ID NO: 384 - DNA, 32 bp, synthetic construct; identical to SEQ ID NO: 376
  misc_feature 1..32: note = source = /note="Description of Artificial Sequence: Synthetic primer"
  source 1..32: mol_type = other DNA

SEQ ID NO: 385 - DNA, 33 bp, synthetic construct
  misc_feature 1..33: note = source = /note="Description of Artificial Sequence: Synthetic primer"
  source 1..33: mol_type = other DNA
gtggtgccgcggcgtagtgccaaaacaaacagt

SEQ ID NO: 386 - DNA, 32 bp, synthetic construct; identical to SEQ ID NO: 382
  misc_feature 1..32: note = source = /note="Description of Artificial Sequence: Synthetic primer"
  source 1..32: mol_type = other DNA

SEQ ID NO: 387 - DNA, 33 bp, synthetic construct; identical to SEQ ID NO: 385
  misc_feature 1..33: note = source = /note="Description of Artificial Sequence: Synthetic primer"
  source 1..33: mol_type = other DNA

SEQ ID NO: 388 - DNA, 32 bp, synthetic construct; identical to SEQ ID NO: 376
  misc_feature 1..32: note = source = /note="Description of Artificial Sequence: Synthetic primer"
  source 1..32: mol_type = other DNA

SEQ ID NO: 389 - DNA, 32 bp, synthetic construct
  misc_feature 1..32: note = source = /note="Description of Artificial Sequence: Synthetic primer"
  source 1..32: mol_type = other DNA
gtggtgccgcgggcgagggcctacttgatatg

SEQ ID NO: 390 - DNA, 32 bp, synthetic construct
  misc_feature 1..32: note = source = /note="Description of Artificial Sequence: Synthetic primer"
  source 1..32: mol_type = other DNA
gtggtgccgcggcttcccaagtgaggcaatgc

SEQ ID NO: 391 - DNA, 33 bp, synthetic construct
  misc_feature 1..33: note = source = /note="Description of Artificial Sequence: Synthetic primer"
  source 1..33: mol_type = other DNA
gtggtgccgcggacgttttgtgctgctgtaaca

SEQ ID NO: 392 - DNA, 32 bp, synthetic construct
  misc_feature 1..32: note = source = /note="Description of Artificial Sequence: Synthetic primer"
  source 1..32: mol_type = other DNA
gtggtgccgcggctgcaggcacattctcttcc

SEQ ID NO: 393 - DNA, 32 bp, synthetic construct
  misc_feature 1..32: note = source = /note="Description of Artificial Sequence: Synthetic primer"
  source 1..32: mol_type = other DNA
gtggtgccgcgggccctgtgtggtagtagtca

SEQ ID NO: 394 - DNA, 32 bp, synthetic construct; identical to SEQ ID NO: 390
  misc_feature 1..32: note = source = /note="Description of Artificial Sequence: Synthetic primer"
  source 1..32: mol_type = other DNA

SEQ ID NO: 395 - DNA, 33 bp, synthetic construct
  misc_feature 1..33: note = source = /note="Description of Artificial Sequence: Synthetic primer"
  source 1..33: mol_type = other DNA
gtggtgccgcggcagtattaaggggtgggagct

SEQ ID NO: 396 - DNA, 32 bp, synthetic construct
  misc_feature 1..32: note = source = /note="Description of Artificial Sequence: Synthetic primer"
  source 1..32: mol_type = other DNA
gtggtgccgcggtctcttcctcacacagctga

SEQ ID NO: 397 - DNA, 32 bp, synthetic construct
  misc_feature 1..32: note = source = /note="Description of Artificial Sequence: Synthetic primer"
  source 1..32: mol_type = other DNA
gtggtgccgcggggagcttggagggaagagaa

SEQ ID NO: 398 - DNA, 32 bp, synthetic construct; identical to SEQ ID NO: 390
  misc_feature 1..32: note = source = /note="Description of Artificial Sequence: Synthetic primer"
  source 1..32: mol_type = other DNA

SEQ ID NO: 399 - DNA, 32 bp, synthetic construct
  misc_feature 1..32: note = source = /note="Description of Artificial Sequence: Synthetic primer"
  source 1..32: mol_type = other DNA
gtggtgccgcggatggatggggaagacactgg

SEQ ID NO: 400 - DNA, 32 bp, synthetic construct; identical to SEQ ID NO: 392
  misc_feature 1..32: note = source = /note="Description of Artificial Sequence: Synthetic primer"
  source 1..32: mol_type = other DNA

SEQ ID NO: 401 - DNA, 32 bp, synthetic construct
  misc_feature 1..32: note = source = /note="Description of Artificial Sequence: Synthetic primer"
  source 1..32: mol_type = other DNA
gtggtgccgcggggatgaaacagggcaggaac

SEQ ID NO: 402 - DNA, 31 bp, synthetic construct
  misc_feature 1..31: note = source = /note="Description of Artificial Sequence: Synthetic primer"
  source 1..31: mol_type = other DNA
gtggtgccgcggttcccaagtgaggcaatgc

SEQ ID NO: 403 - DNA, 32 bp, synthetic construct
  misc_feature 1..32: note = source = /note="Description of Artificial Sequence: Synthetic primer"
  source 1..32: mol_type = other DNA
gtggtgccgcggtttgcagagccatgatgagg

SEQ ID NO: 404 - DNA, 30 bp, synthetic construct
  misc_feature 1..30: note = source = /note="Description of Artificial Sequence: Synthetic primer"
  source 1..30: mol_type = other DNA
gtggtgccgcggcgacagccaaaacagccg

SEQ ID NO: 405 - DNA, 44 bp, synthetic construct
  misc_feature 1..44: note = source = /note="Description of Artificial Sequence: Synthetic oligonucleotide"
  source 1..44: mol_type = other DNA
aaaatattttagctcctactcagactgttactctggtgacacaa

SEQ ID NO: 406 - DNA, 44 bp, synthetic construct
  misc_feature 1..44: note = source = /note="Description of Artificial Sequence: Synthetic oligonucleotide"
  source 1..44: mol_type = other DNA
ttgtgtcaccagagtaacagtctgagtaggagctaaaatatttt

SEQ ID NO: 407 - DNA, 36 bp, synthetic construct
  misc_feature 1..36: note = source = /note="Description of Artificial Sequence: Synthetic oligonucleotide"
  source 1..36: mol_type = other DNA
tagctcctactcagactgttactctggtgacacaac

SEQ ID NO: 408 - DNA, 28 bp, synthetic construct
  misc_feature 1..28: note = source = /note="Description of Artificial Sequence: Synthetic oligonucleotide"
  source 1..28: mol_type = other DNA
tagctcctactcagactggtgacccaac

SEQ ID NO: 409 - DNA, 24 bp, synthetic construct
  misc_feature 1..24: note = source = /note="Description of Artificial Sequence: Synthetic oligonucleotide"
  source 1..24: mol_type = other DNA
tagctcctactctggtgacacaac

SEQ ID NO: 410 - DNA, 28 bp, synthetic construct
  misc_feature 1..28: note = source = /note="Description of Artificial Sequence: Synthetic oligonucleotide"
  source 1..28: mol_type = other DNA
tagctcctactcagactggtgacacaac

SEQ ID NO: 411 - DNA, 16 bp, synthetic construct
  misc_feature 1..16: note = source = /note="Description of Artificial Sequence: Synthetic oligonucleotide"
  source 1..16: mol_type = other DNA
tagctcctactcagac

SEQ ID NO: 412 - DNA, 27 bp, synthetic construct
  misc_feature 1..27: note = source = /note="Description of Artificial Sequence: Synthetic oligonucleotide"
  source 1..27: mol_type = other DNA
tagctcctactcagactgttacacaac

SEQ ID NO: 413 - DNA, 30 bp, synthetic construct
  misc_feature 1..30: note = source = /note="Description of Artificial Sequence: Synthetic oligonucleotide"
  source 1..30: mol_type = other DNA
tagctcctactcagactgtggtgaggtgac

SEQ ID NO: 414 - DNA, 32 bp, synthetic construct
  misc_feature 1..32: note = source = /note="Description of Artificial Sequence: Synthetic oligonucleotide"
  source 1..32: mol_type = other DNA
tagctcctactcagactctctggtgacacaac

SEQ ID NO: 415 - DNA, 31 bp, synthetic construct
  misc_feature 1..31: note = source = /note="Description of Artificial Sequence: Synthetic oligonucleotide"
  source 1..31: mol_type = other DNA
tagctcctactcagacctctggtgacacaac

SEQ ID NO: 416 - DNA, 32 bp, synthetic construct
  misc_feature 1..32: note = source = /note="Description of Artificial Sequence: Synthetic oligonucleotide"
  source 1..32: mol_type = other DNA
tagctcctactcaggctgtctggtgacacaac

SEQ ID NO: 417 - DNA, 33 bp, synthetic construct
  misc_feature 1..33: note = source = /note="Description of Artificial Sequence: Synthetic oligonucleotide"
  source 1..33: mol_type = other DNA
tagctcctactcagactactctggtgacacaac

SEQ ID NO: 418 - DNA, 28 bp, synthetic construct
  misc_feature 1..28: note = source = /note="Description of Artificial Sequence: Synthetic oligonucleotide"
  source 1..28: mol_type = other DNA
tagctcctactcagactgttgacacaac

SEQ ID NO: 419 - DNA, 13 bp, synthetic construct
  misc_feature 1..13: note = source = /note="Description of Artificial Sequence: Synthetic oligonucleotide"
  source 1..13: mol_type = other DNA
ctggtgacacaac

SEQ ID NO: 420 - DNA, 29 bp, synthetic construct
  misc_feature 1..29: note = source = /note="Description of Artificial Sequence: Synthetic oligonucleotide"
  source 1..29: mol_type = other DNA
tagctcctactcagactgttagacacaac

SEQ ID NO: 421 - DNA, 33 bp, synthetic construct
  misc_feature 1..33: note = source = /note="Description of Artificial Sequence: Synthetic oligonucleotide"
  source 1..33: mol_type = other DNA
tagctcctactcagactgctctggtgacacaac

SEQ ID NO: 422 - DNA, 20 bp, synthetic construct
  misc_feature 1..20: note = source = /note="Description of Artificial Sequence: Synthetic oligonucleotide"
  source 1..20: mol_type = other DNA
cagactgttactctggtgac

SEQ ID NO: 423 - DNA, 29 bp, synthetic construct
  misc_feature 1..29: note = source = /note="Description of Artificial Sequence: Synthetic oligonucleotide"
  source 1..29: mol_type = other DNA
cagaccacctgtggtctcctactggtgac

SEQ ID NO: 424 - DNA, 18 bp, synthetic construct
  misc_feature 1..18: note = source = /note="Description of Artificial Sequence: Synthetic oligonucleotide"
  source 1..18: mol_type = other DNA
gctttgatttccctaggg

SEQ ID NO: 425 - DNA, 25 bp, synthetic construct
  misc_feature 1..25: note = source = /note="Description of Artificial Sequence: Synthetic oligonucleotide"
  source 1..25: mol_type = other DNA
gctttgatttccagttcttaggcaa

SEQ ID NO: 426 - DNA, 18 bp, synthetic construct
  misc_feature 1..18: note = source = /note="Description of Artificial Sequence: Synthetic oligonucleotide"
  source 1..18: mol_type = other DNA
gctttgattcttaggcaa

SEQ ID NO: 427 - DNA, 62 bp, synthetic construct
  variation 13..53: note = a, c, t, g, unknown or other
  misc_feature 1..62: note = source = /note="Description of Artificial Sequence: Synthetic oligonucleotide"
  source 1..62: mol_type = other DNA
gctttgatttccnnnnnnnnnnnnnnnnnnnnnnnnnnnnnnnnnnnnnnnnncttaggcaa

SEQ ID NO: 428 - DNA, 18 bp, synthetic construct
  misc_feature 1..18: note = source = /note="Description of Artificial Sequence: Synthetic oligonucleotide"
  source 1..18: mol_type = other DNA
tcttaaccattaccatag

SEQ ID NO: 429 - DNA, 32 bp, synthetic construct
  misc_feature 1..32: note = source = /note="Description of Artificial Sequence: Synthetic oligonucleotide"
  source 1..32: mol_type = other DNA
tcttaaccattaccatagagttcttaggcaac

SEQ ID NO: 430 - DNA, 30 bp, synthetic construct
  misc_feature 1..30: note = source = /note="Description of Artificial Sequence: Synthetic oligonucleotide"
  source 1..30: mol_type = other DNA
tcttaaccattaccaaagttcttaggcaac

SEQ ID NO: 431 - DNA, 31 bp, synthetic construct
  misc_feature 1..31: note = source = /note="Description of Artificial Sequence: Synthetic oligonucleotide"
  source 1..31: mol_type = other DNA
tcttaaccattaccataggttcttaggcaac

SEQ ID NO: 432 - DNA, 14 bp, synthetic construct
  misc_feature 1..14: note = source = /note="Description of Artificial Sequence: Synthetic oligonucleotide"
  source 1..14: mol_type = other DNA
gaaccaaacccact

SEQ ID NO: 433 - DNA, 24 bp, synthetic construct
  misc_feature 1..24: note = source = /note="Description of Artificial Sequence: Synthetic oligonucleotide"
  source 1..24: mol_type = other DNA
gaaccaaacccacttaggggataa

SEQ ID NO: 434 - DNA, 2328 bp, synthetic construct
  misc_feature 1..2328: note = source = /note="Description of Artificial Sequence: Synthetic polynucleotide"
  source 1..2328: mol_type = other DNA
atgaggtctgactacaaagaccatgacggtgattataaagatcatgacatcgattacaaggatgacgatgacaagatggcccccaagaagaagaggaaggtgggcctcgagcccggagaaaaaccgtacaagtgccctgagtgcgggaaatcattctccgaccctggggcgctcgtccggcaccaaaggacgcatacaggggaaaagccgtataagtgccccgagtgtggaaagagcttctcgcagagagcccaccttgaacgacaccaaagaacacacactggtgagaaaccctataagtgtccagagtgcggcaaatcgtttagcagatccgatgacttggtgcgccaccagcggacacacacgggtgaaaagccctacaaatgcccggagtgtgggaagtcgttttcaaggtcggatcatctgactacccatcagcgcacccatacgggagcggccgcccgcgccctggtgaagagcgagctggaggagaagaagtccgagctgcggcacaagctgaagtacgtgccccacgagtacatcgagctgatcgagatcgccaggaaccccacccaggaccgcatcctggagatgaaggtgatggagttcttcatgaaggtgtacggctacaggggagagcacctgggcggaagcagaaagcctgacggcgccatctatacagtgggcagccccatcgattacggcgtgatcgtggacacaaaggcctacagcggcggctacaatctgcctatcggccaggccgacgagatgcagagatacgtgaaggagaaccagacccggaataagcacatcaaccccaacgagtggtggaaggtgtaccctagcagcgtgaccgagttcaagttcctgttcgtgagcggccacttcaagggcaactacaaggcccagctgaccaggctgaaccgcaaaaccaactgcaatggcgccgtgctgagcgtggaggagctgctgatcggcggcgagatgatcaaagccggcaccctgacactggaggaggtgcggcgcaagttcaacaacggcgagatcaacttcgagggcagaggaagtcttctaacatgcggtgacgtggaggagaatcccggccctagatctgactacaaagaccatgacggtgattataaagatcatgacatcgattacaaggatgacgatgacaagatggcccccaagaagaagaggaaggtgggcctcgagccgggagagaagccgtacaagtgtcccgaatgtggaaagagcttctcacagtcgggggaccttcggcgccaccagcgcacacatactggtgaaaagccgtataagtgtccagaatgtggcaaatcattctccacatcagggagcctggtcaggcaccagcgaacccacacgggtgagaagccctataagtgccccgaatgcgggaagtccttttcgcagagagcccacttggagaggcaccagaggacccatacgggggagaaaccttacaagtgccctgaatgcggaaagtcgttctcgacccatctggatctcatcagacatcagagaacgcacactggagagaaaccctacaaatgtcccgagtgtgggaagtcgtttagccgaaaggacaatctcaaaaaccatcaacggacacacacgggtgaaaaaccatacaaatgcccggagtgcggcaaatcgttttcccaacttgcgcacttgcgggcacaccaacgcacgcatactggagcggccgcccgcgccctggtgaagagcgagctggaggagaagaagtccgagctgcggcacaagctgaagtacgtgccccacgagtacatcgagctgatcgagatcgccaggaaccccacccaggaccgcatcctggagatgaaggtgatggagttcttcatgaaggtgtacggctacaggggagagcacctgggcggaagcagaaagcctgacggcgccatctatacagtgggcagccccatcgattacggcgtgatcgtggacacaaaggcctacagcggcggctacaatctgcctatcggccaggccgacgagatggagagatacgtggaggagaaccagacacgggataagcacctcaaccccaacgagtggtggaaggtgtaccctagcagcgtgaccgagttcaagttcctgttcgtgagcggccacttcaagggcaactacaaggcccagctgaccaggctgaaccacatcaccaactgcaatggcgccgtgctgagcgtggaggagctgctgatcggcggcgagatgatcaaagccggcaccctgacactggaggaggtgcggcgcaagttcaacaacggcgagatcaacttctga

SEQ ID NO: 435 - protein, 775 aa, synthetic construct
  REGION 1..775: note = source = /note="Description of Artificial Sequence: Synthetic polypeptide"
MRSDYKDHDGDYKDHDIDYKDDDDKMAPKKKRKVGLEPGEKPYKCPECGKSFSDPGALVRHQRTHTGEKPYKCPECGKSFSQRAHLERHQRTHTGEKPYKCPECGKSFSRSDDLVRHQRTHTGEKPYKCPECGKSFSRSDHLTTHQRTHTGAAARALVKSELEEKKSELRHKLKYVPHEYIELIEIARNPTQDRILEMKVMEFFMKVYGYRGEHLGGSRKPDGAIYTVGSPIDYGVIVDTKAYSGGYNLPIGQADEMQRYVKENQTRNKHINPNEWWKVYPSSVTEFKFLFVSGHFKGNYKAQLTRLNRKTNCNGAVLSVEELLIGGEMIKAGTLTLEEVRRKFNNGEINFEGRGSLLTCGDVEENPGPRSDYKDHDGDYKDHDIDYKDDDDKMAPKKKRKVGLEPGEKPYKCPECGKSFSQSGDLRRHQRTHTGEKPYKCPECGKSFSTSGSLVRHQRTHTGEKPYKCPECGKSFSQRAHLERHQRTHTGEKPYKCPECGKSFSTHLDLIRHQRTHTGEKPYKCPECGKSFSRKDNLKNHQRTHTGEKPYKCPECGKSFSQLAHLRAHQRTHTGAAARALVKSELEEKKSELRHKLKYVPHEYIELIEIARNPTQDRILEMKVMEFFMKVYGYRGEHLGGSRKPDGAIYTVGSPIDYGVIVDTKAYSGGYNLPIGQADEMERYVEENQTRDKHLNPNEWWKVYPSSVTEFKFLFVSGHFKGNYKAQLTRLNHITNCNGAVLSVEELLIGGEMIKAGTLTLEEVRRKFNNGEINF

SEQ ID NO: 436 - DNA, 4725 bp, synthetic construct
  misc_feature 1..4725: note = source = /note="Description of Artificial Sequence: Synthetic polynucleotide"
  source 1..4725: mol_type = other DNA
tggccactccctctatgcgcactcgctcgctcggtggggcctggcgaccaaaggtcgccagacggacgtgctttgcacgtccggccccaccgagcgagcgagtgcgcatagagggagtggccaactccatcactagaggtatggcagtgacgtaacgcgaagcgcgcgaagcgagaccacgcctaccagctgcgtcagcagtcaggtgacccttttgcgacagtttgcgacaccacgtggccgctgagggtatatattctcgagtgagcgaaccaggagctccattttgaccgcgaaatttgaacgagcagcagccatgccggggttctacgagattgtcctgaaggtcccgagtgacctggacgagcacctgccgggcatttctaactcgtttgttaactgggtggccgagaaggaatgggagctgccgccggattctgacatggatccgaatctgattgagcaggcacccctgaccgtggccgaaaagcttcagcgcgagttcctggtggagtggcgccgcgtgagtaaggccccggaggccctcttttttgtccagttcgaaaagggggagacctacttccacctgcacgtgctgattgagaccatcggggtcaaatccatggtggtcggccgctacgtgagccagattaaagagaagctggtgacccgcatctaccgcggggtcgagccgcagcttccgaactggttcgcggtgaccaaaacgcgaaatggcgccgggggcgggaacaaggtggtggacgactgctacatccccaactacctgctccccaagacccagcccgagctccagtgggcgtggactaacatggaccagtatttaagcgcctgtttgaatctcgcggagcgtaaacggctggtggcgcagcatctgacgcacgtgtcgcagacgcaggagcagaacaaagagaatcagaaccccaattctgacgcgccggtcatcaggtcaaaaacctcagccaggtacatggagctggtcgggtggctggtggaccgcgggatcacgtcagaaaagcaatggattcaggaggaccaggcctcgtacatctccttcaacgccgcctccaactcgcggtcccagatcaaggccgcgctggacaatgcctccaagatcatgagcctgacaaagacggctccggactacctggtgggcagcaacccgccggaggacattaccaaaaatcggatctaccaaatcctggagctgaacgggtacgatccgcagtacgcggcctccgtcttcctgggctgggcgcaaaagaagttcgggaagaggaacaccatctggctctttgggccggccacgacgggtaaaaccaacatcgcggaagccatcgcccacgccgtgcccttctacggctgcgtaaactggaccaatgagaactttcccttcaacgattgcgtcgacaagatggtgatctggtgggaggagggcaagatgacggccaaggtcgtggagagcgccaaggccattctgggcggaagcaaggtgcgcgtggaccaaaagtgcaagtcatcggcccagatcgaacccactcccgtgatcgtcacctccaacaccaacatgtgcgccgtgattgacgggaacagcaccaccttcgagcatcagcagccgctgcaggaccggatgtttaaatttgaacttacccgccgtttggaccatgactttgggaaggtcaccaaacaggaagtaaaggactttttccggtgggcttccgatcacgtgactgacgtggctcatgagttctacgtcagaaagggtggagctaagaaacgccccgcctccaatgacgcggatgtaagcgagccaaaacggcagtgcacgtcacttgcgcagccgacaacgtcagacgcggaagcaccggcggactacgcggacaggtaccaaaacaaatgttctcgtcacgtgggcatgaatctgatgctttttccctgtaaaacatgcgagagaatgaatcaaatttccaatgtctgttttacgcatggtcaaagagactgtggggaatgcttccctggaatgtcagaatctcaacccgtttctgtcgtcaaaaagaagacttatcagaaactgtgtccaattcatcatatcctgggaagggcacccgagattgcctgttcggcctgcgatttggccaatgtggacttggatgactgtgtttctgagcaataaatgacttaaaccaggtatggctgctgacggttatcttccagattggctcgaggacaacctttctgaaggcattcgtgagtggtgggctctgaaacctggagtccctcaacccaaagcgaaccaacaacaccaggacaaccgtcggggtcttgtgcttccgggttacaaatacctcggacccggtaacggactcgacaaaggagagccggtcaacgaggcggacgcggcagccctcgaacacgacaaagcttacgaccagcagctcaaggccggtgacaacccgtacctcaagtacaaccacgccgacgccgagtttcaggagcgtcttcaagaagatacgtcttttgggggcaaccttggcagagcagtcttccaggccaaaaagaggatccttgagcctcttggtctggttgaggaagcagctaaaacggctcctggaaagaagaggcctgtagatcagtctcctcaggaaccggactcatcatctggtgttggcaaatcgggcaaacagcctgccagaaaaagactaaatttcggtcagactggcgactcagagtcagtcccagaccctcaacctctcggagaaccaccagcagcccccacaagtttgggatctaatacaatggcttcaggcggtggcgcaccaatggcagacaataacgagggtgccgatggagtgggtaattcctcaggaaattggcattgcgattcccaatggctgggcgacagagtcatcaccaccagcaccagaacctgggccctgcccacttacaacaaccatctctacaagcaaatctccagcgcttcaacgggagcttcaaacgacaaccactactttggctacagcaccccttgggggtattttgactttaacagattccactgccacttctcaccacgtgactggcagcgactcattaacaacaactggggattccggcccaagaaactcagcttcaagctcttcaacatccaagttaaagaggtcacgcagaacgatggcacgacgactattgccaataaccttaccagcacggttcaagtgtttacggactcggagtatcagctcccgtacgtgctcgggtcggcgcaccaaggctgtctcccgccgtttccagcggacgtcttcatggtccctcagtatggatacctcaccctgaacaacggaagtcaagcggtgggacgctcatccttttactgcctggagtacttcccttcgcagatgctaaggactggaaataacttccaattcagctataccttcgaggatgtaccttttcacagcagctacgctcacagccagagtttggatcgcttgatgaatcctcttattgatcagtatctgtactacctgaacagaacgcaaggaacaacctctggaacaaccaaccaatcacggctgctttttagccaggctgggcctcagtctatgtctttgcaggccagaaattggctacctgggccctgctaccggcaacagagactttcaaagactgctaacgacaacaacaacagtaactttccttggacagcggccagcaaatatcatctcaatggccgcgactcgctggtgaatccaggaccagctatggccagtcacaaggacgatgaagaaaaatttttccctatgcacggcaatctaatatttggcaaagaagggacaacggcaagtaacgcagaattagataatgtaatgattacggatgaagaagagattcgtaccaccaatcctgtggcaacagagcagtatggaactgtggcaaataacttgcagagctcaaatacagctcccacgactagaactgtcaatgatcagggggccttacctggcatggtgtggcaagatcgtgacgtgtaccttcaaggacctatctgggcaaagattcctcacacggatggacactttcatccttctcctctgatgggaggctttggactgaaacatccgcctcctcaaatcatgatcaaaaatactccggtaccggcaaatcctccgacgactttcagcccggccaagtttgcttcatttatcactcagtactccactggacaggtcagcgtggaaattgagtgggagctacagaaagaaaacagcaaacgttggaatccagagattcagtacacttccaactacaacaagtctgttaatgtggactttactgtagacactaatggtgtttatagtgaacctcgccctattggaacccggtatctcacacgaaacttgtaatcctggttaatcaataaaccgtttaattcgtttcagttgaactttggctcttgtgcacttcttatcttatcttgtttccatggctactgcgtagataagcagcggcctgcggcgcttgcgcttcgcggtttacaactgctggttaatatttaactctcgccatacctctagtgatggagttggccactccctctatgcgcactcgctcgctcggtggggccggacgtgcaaagcacgtccgtctggcgacctttggtcgccaggccccaccgagcgagcgagtgcgcatagagggagtggccaa

SEQ ID NO: 437 - protein, 737 aa, synthetic construct
  REGION 1..737: note = source = /note="Description of Artificial Sequence: Synthetic polypeptide"
MAADGYLPDWLEDNLSEGIREWWALKPGVPQPKANQQHQDNRRGLVLPGYKYLGPGNGLDKGEPVNEADAAALEHDKAYDQQLKAGDNPYLKYNHADAEFQERLQEDTSFGGNLGRAVFQAKKRILEPLGLVEEAAKTAPGKKRPVDQSPQEPDSSSGVGKSGKQPARKRLNFGQTGDSESVPDPQPLGEPPAAPTSLGSNTMASGGGAPMADNNEGADGVGNSSGNWHCDSQWLGDRVITTSTRTWALPTYNNHLYKQISSASTGASNDNHYFGYSTPWGYFDFNRFHCHFSPRDWQRLINNNWGFRPKKLSFKLFNIQVKEVTQNDGTTTIANNLTSTVQVFTDSEYQLPYVLGSAHQGCLPPFPADVFMVPQYGYLTLNNGSQAVGRSSFYCLEYFPSQMLRTGNNFQFSYTFEDVPFHSSYAHSQSLDRLMNPLIDQYLYYLNRTQGTTSGTTNQSRLLFSQAGPQSMSLQARNWLPGPCYRQQRLSKTANDNNNSNFPWTAASKYHLNGRDSLVNPGPAMASHKDDEEKFFPMHGNLIFGKEGTTASNAELDNVMITDEEEIRTTNPVATEQYGTVANNLQSSNTAPTTRTVNDQGALPGMVWQDRDVYLQGPIWAKIPHTDGHFHPSPLMGGFGLKHPPPQIMIKNTPVPANPPTTFSPAKFASFITQYSTGQVSVEIEWELQKENSKRWNPEIQYTSNYNKSVNVDFTVDTNGVYSEPRPIGTRYLTRNL

SEQ ID NO: 438 - protein, 406 aa, synthetic construct
  REGION 1..406: note = source = /note="Description of Artificial Sequence: Synthetic polypeptide"
MDYKDHDGDYKDHDIDYKDDDDKMAPKKKRKVGRLEPGEKPYKCPECGKSFSRKDALRGHQRTHTGEKPYKCPECGKSFSHRTTLTNHQRTHTGEKPYKCPECGKSFSQRNALAGHQRTHTGEKPYKCPECGKSFSHKNALQNHQRTHTGEKPYKCPECGKSFSDPGHLVRHQRTHTGEKPYKCPECGKSFSTSGNLVRHQRTHTGAAARALVKSELEEKKSELRHKLKYVPHEYIELIEIARNPTQDRILEMKVMEFFMKVYGYRGEHLGGSRKPDGAIYTVGSPIDYGVIVDTKAYSGGYNLPIGQADEMERYVEENQTRDKHLNPNEWWKVYPSSVTEFKFLFVSGHFKGNYKAQLTRLNHITNCNGAVLSVEELLIGGEMIKAGTLTLEEVRRKFNNGEINF

SEQ ID NO: 439 - protein, 406 aa, synthetic construct
  REGION 1..406: note = source = /note="Description of Artificial Sequence: Synthetic polypeptide"
MDYKDHDGDYKDHDIDYKDDDDKMAPKKKRKVGRLEPGEKPYKCPECGKSFSQQRSLVGHQRTHTGEKPYKCPECGKSFSDKKDLTRHQRTHTGEKPYKCPECGKSFSTSGHLVRHQRTHTGEKPYKCPECGKSFSQRAHLERHQRTHTGEKPYKCPECGKSFSTSGSLVRHQRTHTGEKPYKCPECGKSFSTSGNLVRHQRTHTGAAARALVKSELEEKKSELRHKLKYVPHEYIELIEIARNPTQDRILEMKVMEFFMKVYGYRGEHLGGSRKPDGAIYTVGSPIDYGVIVDTKAYSGGYNLPIGQADEMQRYVKENQTRNKHINPNEWWKVYPSSVTEFKFLFVSGHFKGNYKAQLTRLNRKTNCNGAVLSVEELLIGGEMIKAGTLTLEEVRRKFNNGEINF

SEQ ID NO: 440 - protein, 320 aa, synthetic construct
  REGION 1..320: note = source = /note="Description of Artificial Sequence: Synthetic polypeptide"
MDYKDHDGDYKDHDIDYKDDDDKMAPKKKRKVGRLEPGERPFQCRICMRNFSSKQALAVHTRTHTGEKPFQCRICMRNFSQSTTLKRHLRTHTGEKPFQCRICMRNFSRSDHLSLHLKTHLRGSQLVKSELEEKKSELRHKLKYVPHEYIELIEIARNPTQDRILEMKVMEFFMKVYGYRGEHLGGSRKPDGAIYTVGSPIDYGVIVDTKAYSGGYNLPIGQADEMQRYVKENQTRNKHINPNEWWKVYPSSVTEFKFLFVSGHFKGNYKAQLTRLNRKTNCNGAVLSVEELLIGGEMIKAGTLTLEEVRRKFNNGEINF

SEQ ID NO: 441 - protein, 320 aa, synthetic construct
  REGION 1..320: note = source = /note="Description of Artificial Sequence: Synthetic polypeptide"
MDYKDHDGDYKDHDIDYKDDDDKMAPKKKRKVGRLEPGERPFQCRICMRNFSRRAHLQNHTRTHTGEKPFQCRICMRNFSQSTTLKRHLRTHTGEKPFQCRICMRNFSDGGHLTRHLKTHLRGSQLVKSELEEKKSELRHKLKYVPHEYIELIEIARNPTQDRILEMKVMEFFMKVYGYRGEHLGGSRKPDGAIYTVGSPIDYGVIVDTKAYSGGYNLPIGQADEMERYVEENQTRDKHLNPNEWWKVYPSSVTEFKFLFVSGHFKGNYKAQLTRLNHITNCNGAVLSVEELLIGGEMIKAGTLTLEEVRRKFNNGEINF

SEQ ID NO: 442 - DNA, 42 bp, synthetic construct
  misc_feature 1..42: note = source = /note="Description of Artificial Sequence: Synthetic oligonucleotide"
  source 1..42: mol_type = other DNA
caaactagaaatgccatcttccttgatgttggaggtacctgc

SEQ ID NO: 443 - protein, 406 aa, synthetic construct; identical to SEQ ID NO: 438
  REGION 1..406: note = source = /note="Description of Artificial Sequence: Synthetic polypeptide"

SEQ ID NO: 444 - protein, 406 aa, synthetic construct; identical to SEQ ID NO: 439
  REGION 1..406: note = source = /note="Description of Artificial Sequence: Synthetic polypeptide"

SEQ ID NO: 445 - DNA, 25 bp, synthetic construct
  misc_feature 1: note = Variation - /replace=" "
  misc_feature 25: note = Variation - /replace=" "
  misc_feature 1..25: note = /note="Variations given in the sequence have no preference with respect to those in the annotations"
  misc_feature 1..25: note = source = /note="Description of Artificial Sequence: Synthetic oligonucleotide"
  source 1..25: mol_type = other DNA
tatctgcccatgactggcgcaggga

SEQ ID NO: 446 - protein, 320 aa, synthetic construct; identical to SEQ ID NO: 440
  REGION 1..320: note = source = /note="Description of Artificial Sequence: Synthetic polypeptide"

SEQ ID NO: 447 - protein, 320 aa, synthetic construct; identical to SEQ ID NO: 441
  REGION 1..320: note = source = /note="Description of Artificial Sequence: Synthetic polypeptide"

SEQ ID NO: 448 - DNA, 42 bp, synthetic construct
  misc_feature 1..42: note = source = /note="Description of Artificial Sequence: Synthetic oligonucleotide"
  source 1..42: mol_type = other DNA
actagaaatgccatcttccttgatgttggaggtacctgctct

SEQ ID NO: 449 - protein, 406 aa, synthetic construct
  REGION 1..406: note = source = /note="Description of Artificial Sequence: Synthetic polypeptide"
MDYKDHDGDYKDHDIDYKDDDDKMAPKKKRKVGRLEPGEKPYKCPECGKSFSHRTTLTNHQRTHTGEKPYKCPECGKSFSQRNALAGHQRTHTGEKPYKCPECGKSFSHKNALQNHQRTHTGEKPYKCPECGKSFSDPGHLVRHQRTHTGEKPYKCPECGKSFSTSGNLVRHQRTHTGEKPYKCPECGKSFSQSSNLVRHQRTHTGAAARALVKSELEEKKSELRHKLKYVPHEYIELIEIARNPTQDRILEMKVMEFFMKVYGYRGEHLGGSRKPDGAIYTVGSPIDYGVIVDTKAYSGGYNLPIGQADEMERYVEENQTRDKHLNPNEWWKVYPSSVTEFKFLFVSGHFKGNYKAQLTRLNHITNCNGAVLSVEELLIGGEMIKAGTLTLEEVRRKFNNGEINF

SEQ ID NO: 450 - protein, 406 aa, synthetic construct
  REGION 1..406: note = source = /note="Description of Artificial Sequence: Synthetic polypeptide"
MDYKDHDGDYKDHDIDYKDDDDKMAPKKKRKVGRLEPGEKPYKCPECGKSFSQRNALAGHQRTHTGEKPYKCPECGKSFSQQRSLVGHQRTHTGEKPYKCPECGKSFSDKKDLTRHQRTHTGEKPYKCPECGKSFSTSGHLVRHQRTHTGEKPYKCPECGKSFSQRAHLERHQRTHTGEKPYKCPECGKSFSTSGSLVRHQRTHTGAAARALVKSELEEKKSELRHKLKYVPHEYIELIEIARNPTQDRILEMKVMEFFMKVYGYRGEHLGGSRKPDGAIYTVGSPIDYGVIVDTKAYSGGYNLPIGQADEMQRYVKENQTRNKHINPNEWWKVYPSSVTEFKFLFVSGHFKGNYKAQLTRLNRKTNCNGAVLSVEELLIGGEMIKAGTLTLEEVRRKFNNGEINF

SEQ ID NO: 451 - protein, 378 aa, synthetic construct
  REGION 1..378: note = source = /note="Description of Artificial Sequence: Synthetic polypeptide"
MDYKDHDGDYKDHDIDYKDDDDKMAPKKKRKVGRLEPGEKPYKCPECGKSFSQRNALAGHQRTHTGEKPYKCPECGKSFSHKNALQNHQRTHTGEKPYKCPECGKSFSDPGHLVRHQRTHTGEKPYKCPECGKSFSTSGNLVRHQRTHTGEKPYKCPECGKSFSQSSNLVRHQRTHTGAAARALVKSELEEKKSELRHKLKYVPHEYIELIEIARNPTQDRILEMKVMEFFMKVYGYRGEHLGGSRKPDGAIYTVGSPIDYGVIVDTKAYSGGYNLPIGQADEMERYVEENQTRDKHLNPNEWWKVYPSSVTEFKFLFVSGHFKGNYKAQLTRLNHITNCNGAVLSVEELLIGGEMIKAGTLTLEEVRRKFNNGEINF

SEQ ID NO: 452 - protein, 378 aa, synthetic construct
  REGION 1..378: note = source = /note="Description of Artificial Sequence: Synthetic polypeptide"
MDYKDHDGDYKDHDIDYKDDDDKMAPKKKRKVGRLEPGEKPYKCPECGKSFSQQRSLVGHQRTHTGEKPYKCPECGKSFSDKKDLTRHQRTHTGEKPYKCPECGKSFSTSGHLVRHQRTHTGEKPYKCPECGKSFSQRAHLERHQRTHTGEKPYKCPECGKSFSTSGSLVRHQRTHTGAAARALVKSELEEKKSELRHKLKYVPHEYIELIEIARNPTQDRILEMKVMEFFMKVYGYRGEHLGGSRKPDGAIYTVGSPIDYGVIVDTKAYSGGYNLPIGQADEMQRYVKENQTRNKHINPNEWWKVYPSSVTEFKFLFVSGHFKGNYKAQLTRLNRKTNCNGAVLSVEELLIGGEMIKAGTLTLEEVRRKFNNGEINF

SEQ ID NO: 453 - DNA, 26 bp, synthetic construct
  misc_feature 1: note = Variation - /replace=" "
  misc_feature 26: note = Variation - /replace=" "
  misc_feature 1..26: note = /note="Variations given in the sequence have no preference with respect to those in the annotations"
  misc_feature 1..26: note = source = /note="Description of Artificial Sequence: Synthetic oligonucleotide"
  source 1..26: mol_type = other DNA
tgccatcttccttgatgttggaggta

SEQ ID NO: 454 - protein, 322 aa, synthetic construct
  REGION 1..322: note = source = /note="Description of Artificial Sequence: Synthetic polypeptide"
MDYKDHDGDYKDHDIDYKDDDDKMAPKKKRKVGRLEPGERPFQCRICMRNFSSPSKLARHTRTHTGEKPFQCRICMRNFSVRHNLTRHLRTHTGEKPFQCRICMRNFSQRNNLGRHLKTHTGAAARALVKSELEEKKSELRHKLKYVPHEYIELIEIARNPTQDRILEMKVMEFFMKVYGYRGEHLGGSRKPDGAIYTVGSPIDYGVIVDTKAYSGGYNLPIGQADEMQRYVKENQTRNKHINPNEWWKVYPSSVTEFKFLFVSGHFKGNYKAQLTRLNRKTNCNGAVLSVEELLIGGEMIKAGTLTLEEVRRKFNNGEINF

SEQ ID NO: 455 - protein, 322 aa, synthetic construct
  REGION 1..322: note = source = /note="Description of Artificial Sequence: Synthetic polypeptide"
MDYKDHDGDYKDHDIDYKDDDDKMAPKKKRKVGRLEPGERPFQCRICMRNFSIPNHLARHTRTHTGEKPFQCRICMRNFSQSAHLKRHLRTHTGEKPFQCRICMRNFSHHNSLTRHLKTHTGAAARALVKSELEEKKSELRHKLKYVPHEYIELIEIARNPTQDRILEMKVMEFFMKVYGYRGEHLGGSRKPDGAIYTVGSPIDYGVIVDTKAYSGGYNLPIGQADEMERYVEENQTRDKHLNPNEWWKVYPSSVTEFKFLFVSGHFKGNYKAQLTRLNHITNCNGAVLSVEELLIGGEMIKAGTLTLEEVRRKFNNGEINF

SEQ ID NO: 456 - DNA, 6626 bp, synthetic construct
  misc_feature 1..6626: note = source = /note="Description of Artificial Sequence: Synthetic polynucleotide"
  source 1..6626: mol_type = other DNA
ggggggggggggggggggttggccactccctctctgcgcgctcgctcgctcactgaggccgggcgaccaaaggtcgcccgacgcccgggctttgcccgggcggcctcagtgagcgagcgagcgcgcagagagggagtggccaactccatcactaggggttcctagatctgaattcggtacccgttacataacttacggtaaatggcccgcctggctgaccgcccaacgacccccgcccattgacgtcaataatgacgtatgttcccatagtaacgccaatagggactttccattgacgtcaatgggtggagtatttacggtaaactgcccacttggcagtacatcaagtgtatcatatgccaagtacgccccctattgacgtcaatgacggtaaatggcccgcctggcattatgcccagtacatgaccttatgggactttcctacttggcagtacatctacgtattagtcatcgctattaccatggtgatgcggttttggcagtacatcaatgggcgtggatagcggtttgactcacggggatttccaagtctccaccccattgacgtcaatgggagtttgttttggcaccaaaatcaacgggactttccaaaatgtcgtaacaactccgccccattgacgcaaatgggcggtaggcgtgtacggtgggaggtctatataagcagagctcgtttagtgaaccgtcagatcgcctggagacgccatccacgctgttttgacctccatagaagacaccgggaccgatccagcctccggactctagaggatccggtactcgaggaactgaaaaaccagaaagttaactggtaagtttagtctttttgtcttttatttcaggtcccggatccggtggtggtgcaaatcaaagaactgctcctcagtggatgttgcctttacttctaggcctgtacggaagtgttacttctgctctaaaagctgcggaattgtacccgcggcccgggatccaccggtggctagcgtctataggcccacccccttggtggaattcgccatgaggtctgactacaaagaccatgacggtgattataaagatcatgacatcgattacaaggatgacgatgacaagatggcccccaagaagaagaggaaggtgggcctcgagcccggagaaaaaccgtacaagtgccctgagtgcgggaaatcattctccgaccctggggcgctcgtccggcaccaaaggacgcatacaggggaaaagccgtataagtgccccgagtgtggaaagagcttctcgcagagagcccaccttgaacgacaccaaagaacacacactggtgagaaaccctataagtgtccagagtgcggcaaatcgtttagcagatccgatgacttggtgcgccaccagcggacacacacgggtgaaaagccctacaaatgcccggagtgtgggaagtcgttttcaaggtcggatcatctgactacccatcagcgcacccatacgggagcggccgcccgcgccctggtgaagagcgagctggaggagaagaagtccgagctgcggcacaagctgaagtacgtgccccacgagtacatcgagctgatcgagatcgccaggaaccccacccaggaccgcatcctggagatgaaggtgatggagttcttcatgaaggtgtacggctacaggggagagcacctgggcggaagcagaaagcctgacggcgccatctatacagtgggcagccccatcgattacggcgtgatcgtggacacaaaggcctacagcggcggctacaatctgcctatcggccaggccgacgagatgcagagatacgtgaaggagaaccagacccggaataagcacatcaaccccaacgagtggtggaaggtgtaccctagcagcgtgaccgagttcaagttcctgttcgtgagcggccacttcaagggcaactacaaggcccagctgaccaggctgaaccgcaaaaccaactgcaatggcgccgtgctgagcgtggaggagctgctgatcggcggcgagatgatcaaagccggcaccctgacactggaggaggtgcggcgcaagttcaacaacggcgagatcaacttcgagggcagaggaagtcttctaacatgcggtgacgtggaggagaatcccggccctagatctgactacaaagaccatgacggtgattataaagatcatgacatcgattacaaggatgacgatgacaagatggcccccaagaagaagaggaaggtgggcctcgagccgggagagaagccgtacaagtgtcccgaatgtggaaagagcttctcacagtcgggggaccttcggcgccaccagcgcacacatactggtgaaaagccgtataagtgtccagaatgtggcaaatcattctccacatcagggagcctggtcaggcaccagcgaacccacacgggtgagaagccctataagtgccccgaatgcgggaagtccttttcgcagagagcccacttggagaggcaccagaggacccatacgggggagaaaccttacaagtgccctgaatgcggaaagtcgttctcgacccatctggatctcatcagacatcagagaacgcacactggagagaaaccctacaaatgtcccgagtgtgggaagtcgtttagccgaaaggacaatctcaaaaaccatcaacggacacacacgggtgaaaaaccatacaaatgcccggagtgcggcaaatcgttttcccaacttgcgcacttgcgggcacaccaacgcacgcatactggagcggccgcccgcgccctggtgaagagcgagctggaggagaagaagtccgagctgcggcacaagctgaagtacgtgccccacgagtacatcgagctgatcgagatcgccaggaaccccacccaggaccgcatcctggagatgaaggtgatggagttcttcatgaaggtgtacggctacaggggagagcacctgggcggaagcagaaagcctgacggcgccatctatacagtgggcagccccatcgattacggcgtgatcgtggacacaaaggcctacagcggcggctacaatctgcctatcggccaggccgacgagatggagagatacgtggaggagaaccagacacgggataagcacctcaaccccaacgagtggtggaaggtgtaccctagcagcgtgaccgagttcaagttcctgttcgtgagcggccacttcaagggcaactacaaggcccagctgaccaggctgaaccacatcaccaactgcaatggcgccgtgctgagcgtggaggagctgctgatcggcggcgagatgatcaaagccggcaccctgacactggaggaggtgcggcgcaagttcaacaacggcgagatcaacttctgattaattaactaatctagagtcgactagagctcgctgatcagcctcgactgtgccttctagttgccagccatctgttgtttgcccctcccccgtgccttccttgaccctggaaggtgccactcccactgtcctttcctaataaaatgaggaaattgcatcgcattgtctgagtaggtgtcattctattctggggggtggggtggggcaggacagcaagggggaggattgggaagacaatagcaggcatgctggggagagatctaggaacccctagtgatggagttggccactccctctctgcgcgctcgctcgctcactgaggccgcccgggcaaagcccgggcgtcgggcgacctttggtcgcccggcctcagtgagcgagcgagcgcgcagagagggagtggccaacccccccccccccccccctgcagcccagctgcattaatgaatcggccaacgcgcggggagaggcggtttgcgtattgggcgctcttccgcttcctcgctcactgactcgctgcgctcggtcgttcggctgcggcgagcggtatcagctcactcaaaggcggtaatacggttatccacagaatcaggggataacgcaggaaagaacatgtgagcaaaaggccagcaaaaggccaggaaccgtaaaaaggccgcgttgctggcgtttttccataggctccgcccccctgacgagcatcacaaaaatcgacgctcaagtcagaggtggcgaaacccgacaggactataaagataccaggcgtttccccctggaagctccctcgtgcgctctcctgttccgaccctgccgcttaccggatacctgtccgcctttctcccttcgggaagcgtggcgctttctcaatgctcacgctgtaggtatctcagttcggtgtaggtcgttcgctccaagctgggctgtgtgcacgaaccccccgttcagcccgaccgctgcgccttatccggtaactatcgtcttgagtccaacccggtaagacacgacttatcgccactggcagcagccactggtaacaggattagcagagcgaggtatgtaggcggtgctacagagttcttgaagtggtggcctaactacggctacactagaaggacagtatttggtatctgcgctctgctgaagccagttaccttcggaaaaagagttggtagctcttgatccggcaaacaaaccaccgctggtagcggtggtttttttgtttgcaagcagcagattacgcgcagaaaaaaaggatctcaagaagatcctttgatcttttctacggggtctgacgctcagtggaacgaaaactcacgttaagggattttggtcatgagattatcaaaaaggatcttcacctagatccttttaaattaaaaatgaagttttaaatcaatctaaagtatatatgagtaaacttggtctgacagttaccaatgcttaatcagtgaggcacctatctcagcgatctgtctatttcgttcatccatagttgcctgactccccgtcgtgtagataactacgatacgggagggcttaccatctggccccagtgctgcaatgataccgcgagacccacgctcaccggctccagatttatcagcaataaaccagccagccggaagggccgagcgcagaagtggtcctgcaactttatccgcctccatccagtctattaattgttgccgggaagctagagtaagtagttcgccagttaatagtttgcgcaacgttgttgccattgctacaggcatcgtggtgtcacgctcgtcgtttggtatggcttcattcagctccggttcccaacgatcaaggcgagttacatgatcccccatgttgtgcaaaaaagcggttagctccttcggtcctccgatcgttgtcagaagtaagttggccgcagtgttatcactcatggttatggcagcactgcataattctcttactgtcatgccatccgtaagatgcttttctgtgactggtgagtactcaaccaagtcattctgagaatagtgtatgcggcgaccgagttgctcttgcccggcgtcaatacgggataataccgcgccacatagcagaactttaaaagtgctcatcattggaaaacgttcttcggggcgaaaactctcaaggatcttaccgctgttgagatccagttcgatgtaacccactcgtgcacccaactgatcttcagcatcttttactttcaccagcgtttctgggtgagcaaaaacaggaaggcaaaatgccgcaaaaaagggaataagggcgacacggaaatgttgaatactcatactcttcctttttcaatattattgaagcatttatcagggttattgtctcatgagcggatacatatttgaatgtatttagaaaaataaacaaataggggttccgcgcacatttccccgaaaagtgccacctgacgtctaagaaaccattattatcatgacattaacctataaaaataggcgtatcacgaggccctttcgtctcgcgcgtttcggtgatgacggtgaaaacctctgacacatgcagctcccggagacggtcacagcttgtctgtaagcggatgccgggagcagacaagcccgtcagggcgcgtcagcgggtgttggcgggtgtcggggctggcttaactatgcggcatcagagcagattgtactgagagtgcaccatatgcggtgtgaaataccgcacagatgcgtaaggagaaaataccgcatcaggaaattgtaaacgttaatattttgttaaaattcgcgttaaatttttgttaaatcagctcattttttaaccaataggccgaaatcggcaaaatcccttataaatcaaaagaatagaccgagatagggttgagtgttgttccagtttggaacaagagtccactattaaagaacgtggactccaacgtcaaagggcgaaaaaccgtctatcagggcgatggcccactacgtgaaccatcaccctaatcaagttttttggggtcgaggtgccgtaaagcactaaatcggaaccctaaagggagcccccgatttagagcttgacggggaaagccggcgaacgtggcgagaaaggaagggaagaaagcgaaaggagcgggcgctagggcgctggcaagtgtagcggtcacgctgcgcgtaaccaccacacccgccgcgcttaatgcgccgctacagggcgcgtcgcgccattcgccattcaggctacgcaactgttgggaagggcgatcggtgcgggcctcttcgctattacgccagctggctgca

SEQ ID NO: 457 - DNA, 22 bp, synthetic construct
  misc_feature 1..22: note = source = /note="Description of Artificial Sequence: Synthetic primer"
  source 1..22: mol_type = other DNA
gagaggttatgtggctttacca

SEQ ID NO: 458 - DNA, 20 bp, synthetic construct
  misc_feature 1..20: note = source = /note="Description of Artificial Sequence: Synthetic primer"
  source 1..20: mol_type = other DNA
ctgcgtagtgccaaaacaaa

SEQ ID NO: 459 - DNA, 3252 bp, synthetic construct
  misc_feature 1..3252: note = source = /note="Description of Artificial Sequence: Synthetic polynucleotide"
  source 1..3252: mol_type = other DNA
atgaaaaggaactacattctggggctggacatcgggattacaagcgtggggtatgggattattgactatgaaacaagggacgtgatcgacgcaggcgtcagactgttcaaggaggccaacgtggaaaacaatgagggacggagaagcaagaggggagccaggcgcctgaaacgacggagaaggcacagaatccagagggtgaagaaactgctgttcgattacaacctgctgaccgaccattctgagctgagtggaattaatccttatgaagccagggtgaaaggcctgagtcagaagctgtcagaggaagagttttccgcagctctgctgcacctggctaagcgccgaggagtgcataacgtcaatgaggtggaagaggacaccggcaacgagctgtctacaaaggaacagatctcacgcaatagcaaagctctggaagagaagtatgtcgcagagctgcagctggaacggctgaagaaagatggcgaggtgagagggtcaattaataggttcaagacaagcgactacgtcaaagaagccaagcagctgctgaaagtgcagaaggcttaccaccagctggatcagagcttcatcgatacttatatcgacctgctggagactcggagaacctactatgagggaccaggagaagggagccccttcggatggaaagacatcaaggaatggtacgagatgctgatgggacattgcacctattttccagaagagctgagaagcgtcaagtacgcttataacgcagatctgtacaacgccctgaatgacctgaacaacctggtcatcaccagggatgaaaacgagaaactggaatactatgagaagttccagatcatcgaaaacgtgtttaagcagaagaaaaagcctacactgaaacagattgctaaggagatcctggtcaacgaagaggacatcaagggctaccgggtgacaagcactggaaaaccagagttcaccaatctgaaagtgtatcacgatattaaggacatcacagcacggaaagaaatcattgagaacgccgaactgctggatcagattgctaagatcctgactatctaccagagctccgaggacatccaggaagagctgactaacctgaacagcgagctgacccaggaagagatcgaacagattagtaatctgaaggggtacaccggaacacacaacctgtccctgaaagctatcaatctgattctggatgagctgtggcatacaaacgacaatcagattgcaatctttaaccggctgaagctggtcccaaaaaaggtggacctgagtcagcagaaagagatcccaaccacactggtggacgatttcattctgtcacccgtggtcaagcggagcttcatccagagcatcaaagtgatcaacgccatcatcaagaagtacggcctgcccaatgatatcattatcgagctggctagggagaagaacagcaaggacgcacagaagatgatcaatgagatgcagaaacgaaaccggcagaccaatgaacgcattgaagagattatccgaactaccgggaaagagaacgcaaagtacctgattgaaaaaatcaagctgcacgatatgcaggagggaaagtgtctgtattctctggaggccatccccctggaggacctgctgaacaatccattcaactacgaggtcgatcatattatccccagaagcgtgtccttcgacaattcctttaacaacaaggtgctggtcaagcaggaagagaactctaaaaagggcaataggactcctttccagtacctgtctagttcagattccaagatctcttacgaaacctttaaaaagcacattctgaatctggccaaaggaaagggccgcatcagcaagaccaaaaaggagtacctgctggaagagcgggacatcaacagattctccgtccagaaggattttattaaccggaatctggtggacacaagatacgctactcgcggcctgatgaatctgctgcgatcctatttccgggtgaacaatctggatgtgaaagtcaagtccatcaacggcgggttcacatcttttctgaggcgcaaatggaagtttaaaaaggagcgcaacaaagggtacaagcaccatgccgaagatgctctgattatcgcaaatgccgacttcatctttaaggagtggaaaaagctggacaaagccaagaaagtgatggagaaccagatgttcgaagagaagcaggccgaatctatgcccgaaatcgagacagaacaggagtacaaggagattttcatcactcctcaccagatcaagcatatcaaggatttcaaggactacaagtactctcaccgggtggataaaaagcccaacagagagctgatcaatgacaccctgtatagtacaagaaaagacgataaggggaataccctgattgtgaacaatctgaacggactgtacgacaaagataatgacaagctgaaaaagctgatcaacaaaagtcccgagaagctgctgatgtaccaccatgatcctcagacatatcagaaactgaagctgattatggagcagtacggcgacgagaagaacccactgtataagtactatgaagagactgggaactacctgaccaagtatagcaaaaaggataatggccccgtgatcaagaagatcaagtactatgggaacaagctgaatgcccatctggacatcacagacgattaccctaacagtcgcaacaaggtggtcaagctgtcactgaagccatacagattcgatgtctatctggacaacggcgtgtataaatttgtgactgtcaagaatctggatgtcatcaaaaaggagaactactatgaagtgaatagcaagtgctacgaagaggctaaaaagctgaaaaagattagcaaccaggcagagttcatcgcctccttttacaacaacgacctgattaagatcaatggcgaactgtatagggtcatcggggtgaacaatgatctgctgaaccgcattgaagtgaatatgattgacatcacttaccgagagtatctggaaaacatgaatgataagcgcccccctcgaattatcaaaacaattgcctctaagactcagagtatcaaaaagtactcaaccgacattctgggaaacctgtatgaggtgaagagcaaaaagcaccctcagattatcaaaaagggcagcggaggcaagcgtcctgctgctactaagaaagctggtcaagctaagaaaaagaaaggatcctacccatacgatgttccagattacgcttaa

SEQ ID NO: 460 - DNA, 83 bp, synthetic construct
  misc_feature 1..83: note = source = /note="Description of Artificial Sequence: Synthetic oligonucleotide"
  source 1..83: mol_type = other DNA
gttttagtactctggaaacagaatctactaaaacaaggcaaaatgccgtgtttatctcgtcaacttgttggcgagattttttt

SEQ ID NO: 461 - DNA, 3333 bp, synthetic construct
  misc_feature 1..3333: note = source = /note="Description of Artificial Sequence: Synthetic polynucleotide"
  source 1..3333: mol_type = other DNA
atggtgcctaagaagaagagaaaggtggctgccttcaaacctaattcaatcaactacatcctcggcctcgatatcggcatcgcatccgtcggctgggcgatggtagaaattgacgaagaagaaaaccccatccgcctgattgatttgggcgtgcgcgtatttgagcgtgccgaagtaccgaaaacaggcgactcccttgccatggcaaggcgtttggcgcgcagtgttcgccgcctgacccgccgtcgcgcccaccgcctgcttcggacccgccgcctattgaaacgcgaaggcgtattacaagccgccaattttgacgaaaacggcttgattaaatccttaccgaatacaccatggcaacttcgcgcagccgcattagaccgcaaactgacgcctttagagtggtcggcagtcttgttgcatttaatcaaacatcgcggctatttatcgcaacggaaaaacgagggcgaaactgccgataaggagcttggcgctttgcttaaaggcgtagccggcaatgcccatgccttacagacaggcgatttccgcacaccggccgaattggctttaaataaatttgagaaagaaagcggccatatccgcaatcagcgcagcgattattcgcatacgttcagccgcaaagatttacaggcggagctgattttgctgtttgaaaaacaaaaagaatttggcaatccgcatgtttcaggcggccttaaagaaggtattgaaaccctactgatgacgcaacgccctgccctgtccggcgatgccgttcaaaaaatgttggggcattgcaccttcgaaccggcagagccgaaagccgctaaaaacacctacacagccgaacgtttcatctggctgaccaagctgaacaacctgcgtattttagagcaaggcagcgagcggccattgaccgataccgaacgcgccacgcttatggacgagccatacagaaaatccaaactgacttacgcacaagcccgtaagctgctgggtttagaagataccgcctttttcaaaggcttgcgctatggtaaagacaatgccgaagcctcaacattgatggaaatgaaggcctaccatgccatcagccgtgcactggaaaaagaaggattgaaagacaaaaaatccccattaaacctttctcccgaattacaagacgaaatcggcacggcattctccctgttcaaaaccgatgaagacattacaggccgtctgaaagaccgtatacagcccgaaatcttagaagcgctgttgaaacacatcagcttcgataagttcgtccaaatttccttgaaagcattgcgccgaattgtgcctctaatggaacaaggcaaacgttacgatgaagcctgcgccgaaatctacggagaccattacggcaagaagaatacggaagaaaagatttatctgccgccgattcccgccgacgaaatccgcaaccccgtcgtcttgcgcgccttatctcaagcacgtaaggtcattaacggcgtggtacgccgttacggctccccagctcgtatccatattgaaactgcaagggaagtaggtaaatcgtttaaagaccgcaaagaaattgagaaacgccaagaagaaaaccgcaaagaccgggaaaaagccgccgccaaattccgagagtatttccccaattttgtcggagaacccaaatccaaagatattctgaaactgcgcctgtacgagcaacaacacggcaaatgcctgtattcgggcaaagaaatcaacttaggccgtctgaacgaaaaaggctatgtcgaaatcgaccatgccctgccgttctcgcgcacatgggacgacagtttcaacaataaagtactggtattgggcagcgaaaaccaaaacaaaggcaatcaaaccccttacgaatacttcaacggcaaagacaacagccgcgaatggcaggaatttaaagcgcgtgtcgaaaccagccgtttcccgcgcagtaaaaaacaacggattctgctgcaaaaattcgatgaagacggctttaaagaacgcaatctgaacgacacgcgctacgtcaaccgtttcctgtgtcaatttgttgccgaccgtatgcggctgacaggtaaaggcaagaaacgtgtctttgcatccaacggacaaattaccaatctgttgcgcggcttttggggattgcgcaaagtgcgtgcggaaaacgaccgccatcacgccttggacgccgtcgtcgttgcctgctcgaccgttgccatgcagcagaaaattacccgttttgtacgctataaagagatgaacgcgtttgacggtaaaaccatagacaaagaaacaggagaagtgctgcatcaaaaaacacacttcccacaaccttgggaatttttcgcacaagaagtcatgattcgcgtcttcggcaaaccggacggcaaacccgaattcgaagaagccgataccctagaaaaactgcgcacgttgcttgccgaaaaattatcatctcgccccgaagccgtacacgaatacgttacgccactgtttgtttcacgcgcgcccaatcggaagatgagcgggcaagggcatatggagaccgtcaaatccgccaaacgactggacgaaggcgtcagcgtgttgcgcgtaccgctgacacagttaaaactgaaagacttggaaaaaatggtcaatcgggagcgcgaacctaagctatacgaagcactgaaagcacggctggaagcacataaagacgatcctgccaaagcctttgccgagccgttttacaaatacgataaagcaggcaaccgcacccaacaggtaaaagccgtacgcgtagagcaagtacagaaaaccggcgtatgggtgcgcaaccataacggtattgccgacaacgcaaccatggtgcgcgtagatgtgtttgagaaaggcgacaagtattatctggtaccgatttacagttggcaggtagcgaaagggattttgccggatagggctgttgtacaaggaaaagatgaagaagattggcaacttattgatgatagtttcaactttaaattctcattacaccctaatgatttagtcgaggttataacaaaaaaagctagaatgtttggttactttgccagctgccatcgaggcacaggtaatatcaatatacgcattcatgatcttgatcataaaattggcaaaaatggaatactggaaggtatcggcgtcaaaaccgccctttcattccaaaaataccaaattgacgaactgggcaaagaaatcagaccatgccgtctgaaaaaacgcccgcctgtccgttacccatacgatgttccagattacgctgcagctccagcagcgaagaaaaagaagctggattaa

SEQ ID NO: 462 - DNA, 120 bp, synthetic construct
  misc_feature 1..120: note = source = /note="Description of Artificial Sequence: Synthetic polynucleotide"
  source 1..120: mol_type = other DNA
gttgtagctccctttctcatttcggaaacgaaatgagaaccgttgctacaataaggccgtctgaaaagatgtgccgcaacgctctgccccttaaagcttctgctttaaggggcttttttt

SEQ ID NO: 463 - DNA, 144 bp, synthetic construct
  misc_feature 1..144: note = source = /note="Description of Artificial Sequence: Synthetic polynucleotide"
  source 1..144: mol_type = other DNA
gttgtagctccctttctcatttcgcagtgctacaatgaaaattgtcgcactgcgaaatgagaaccgttgctacaataaggccgtctgaaaagatgtgccgcaacgctctgccccttaaagcttctgctttaaggggcttttttt

SEQ ID NO: 464 - DNA, 24 bp, synthetic construct
  misc_feature 1..24: note = source = /note="Description of Artificial Sequence: Synthetic primer"
  source 1..24: mol_type = other DNA
tcgggtttattacagggacagcag

SEQ ID NO: 465 - DNA, 24 bp, synthetic construct
  misc_feature 1..24: note = source = /note="Description of Artificial Sequence: Synthetic primer"
  source 1..24: mol_type = other DNA
tctaaggccgagtcttatgagcag

SEQ ID NO: 466 - DNA, 4564 bp, synthetic construct
  misc_feature 1..4564: note = source = /note="Description of Artificial Sequence: Synthetic polynucleotide"
  source 1..4564: mol_type = other DNA
atggactacaaagaccatgacggtgattataaagatcatgacatcgattacaaggatgacgatgacaagatggcccccaagaagaagaggaaggtgggccgcggaatggacaagaagtactccattgggctcgccatcggcacaaacagcgtcggctgggccgtcattacggacgagtacaaggtgccgagcaaaaaattcaaagttctgggcaataccgatcgccacagcataaagaagaacctcattggcgccctcctgttcgactccggggaaaccgccgaagccacgcggctcaaaagaacagcacggcgcagatatacccgcagaaagaatcggatctgctacctgcaggagatctttagtaatgagatggctaaggtggatgactctttcttccataggctggaggagtcctttttggtggaggaggataaaaagcacgagcgccacccaatctttggcaatatcgtggacgaggtggcgtaccatgaaaagtacccaaccatatatcatctgaggaagaagcttgtagacagtactgataaggctgacttgcggttgatctatctcgcgctggcgcatatgatcaaatttcggggacacttcctcatcgagggggacctgaacccagacaacagcgatgtcgacaaactctttatccaactggttcagacttacaatcagcttttcgaagagaacccgatcaacgcatccggagttgacgccaaagcaatcctgagcgctaggctgtccaaatcccggcggctcgaaaacctcatcgcacagctccctggggagaagaagaacggcctgtttggtaatcttatcgccctgtcactcgggctgacccccaactttaaatctaacttcgacctggccgaagatgccaagcttcaactgagcaaagacacctacgatgatgatctcgacaatctgctggcccagatcggcgaccagtacgcagacctttttttggcggcaaagaacctgtcagacgccattctgctgagtgatattctgcgagtgaacacggagatcaccaaagctccgctgagcgctagtatgatcaagcgctatgatgagcaccaccaagacttgactttgctgaaggcccttgtcagacagcaactgcctgagaagtacaaggaaattttcttcgatcagtctaaaaatggctacgccggatacattgacggcggagcaagccaggaggaattttacaaatttattaagcccatcttggaaaaaatggacggcaccgaggagctgctggtaaagcttaacagagaagatctgttgcgcaaacagcgcactttcgacaatggaagcatcccccaccagattcacctgggcgaactgcacgctatcctcaggcggcaagaggatttctacccctttttgaaagataacagggaaaagattgagaaaatcctcacatttcggataccctactatgtaggccccctcgcccggggaaattccagattcgcgtggatgactcgcaaatcagaagagaccatcactccctggaacttcgaggaagtcgtggataagggggcctctgcccagtccttcatcgaaaggatgactaactttgataaaaatctgcctaacgaaaaggtgcttcctaaacactctctgctgtacgagtacttcacagtttataacgagctcaccaaggtcaaatacgtcacagaagggatgagaaagccagcattcctgtctggagagcagaagaaagctatcgtggacctcctcttcaagacgaaccggaaagttaccgtgaaacagctcaaagaagactatttcaaaaagattgaatgtttcgactctgttgaaatcagcggagtggaggatcgcttcaacgcatccctgggaacgtatcacgatctcctgaaaatcattaaagacaaggacttcctggacaatgaggagaacgaggacattcttgaggacattgtcctcacccttacgttgtttgaagatagggagatgattgaagaacgcttgaaaacttacgctcatctcttcgacgacaaagtcatgaaacagctcaagaggcgccgatatacaggatgggggcggctgtcaagaaaactgatcaatgggatccgagacaagcagagtggaaagacaatcctggattttcttaagtccgatggatttgccaaccggaacttcatgcagttgatccatgatgactctctcacctttaaggaggacatccagaaagcacaagtttctggccagggggacagtcttcacgagcacatcgctaatcttgcaggtagcccagctatcaaaaagggaatactgcagaccgttaaggtcgtggatgaactcgtcaaagtaatgggaaggcataagcccgagaatatcgttatcgagatggcccgagagaaccaaactacccagaagggacagaagaacagtagggaaaggatgaagaggattgaagagggtataaaagaactggggtcccaaatccttaaggaacacccagttgaaaacacccagcttcagaatgagaagctctacctgtactacctgcagaacggcagggacatgtacgtggatcaggaactggacatcaatcggctctccgactacgacgtggatgccatcgtgccccagtcttttctcaaagatgattctattgataataaagtgttgacaagatccgataaaaatagagggaagagtgataacgtcccctcagaagaagttgtcaagaaaatgaaaaattattggcggcagctgctgaacgccaaactgatcacacaacggaagttcgataatctgactaaggctgaacgaggtggcctgtctgagttggataaagccggcttcatcaaaaggcagcttgttgagacacgccagatcaccaagcacgtggcccaaattctcgattcacgcatgaacaccaagtacgatgaaaatgacaaactgattcgagaggtgaaagttattactctgaagtctaagctggtctcagatttcagaaaggactttcagttttataaggtgagagagatcaacaattaccaccatgcgcatgatgcctacctgaatgcagtggtaggcactgcacttatcaaaaaatatcccaagcttgaatctgaatttgtttacggagactataaagtgtacgatgttaggaaaatgatcgcaaagtctgagcaggaaataggcaaggccaccgctaagtacttcttttacagcaatattatgaattttttcaagaccgagattacactggccaatggagagattcggaagcgaccacttatcgaaacaaacggagaaacaggagaaatcgtgtgggacaagggtagggatttcgcgacagtccggaaggtcctgtccatgccgcaggtgaacatcgttaaaaagaccgaagtacagaccggaggcttctccaaggaaagtatcctcccgaaaaggaacagcgacaagctgatcgcacgcaaaaaagattgggaccccaagaaatacggcggattcgattctcctacagtcgcttacagtgtactggttgtggccaaagtggagaaagggaagtctaaaaaactcaaaagcgtcaaggaactgctgggcatcacaatcatggagcgatcaagcttcgaaaaaaaccccatcgactttctcgaggcgaaaggatataaagaggtcaaaaaagacctcatcattaagcttcccaagtactctctctttgagcttgaaaacggccggaaacgaatgctcgctagtgcgggcgagctgcagaaaggtaacgagctggcactgccctctaaatacgttaatttcttgtatctggccagccactatgaaaagctcaaagggtctcccgaagataatgagcagaagcagctgttcgtggaacaacacaaacactaccttgatgagatcatcgagcaaataagcgaattctccaaaagagtgatcctcgccgacgctaacctcgataaggtgctttctgcttacaataagcacagggataagcccatcagggagcaggcagaaaacattatccacttgtttactctgaccaacttgggcgcgcctgcagccttcaagtacttcgacaccaccatagacagaaagcggtacacctctacaaaggaggtcctggacgccacactgattcatcagtcaattacggggctctatgaaacaagaatcgacctctctcagctcggtggagacagcagggctgaccccaagaagaagaggaaggtggctagcgatgctaagtcactgactgcctggtcccggacactggtgaccttcaaggatgtgtttgtggacttcaccagggaggagtggaagctgctggacactgctcagcagatcctgtacagaaatgtgatgctggagaactataagaacctggtttccttgggttatcagcttactaagccagatgtgatcctccggttggagaagggagaagagccctggctggtggagagagaaattcaccaagagacccatcctgattcagagactgcatttgaaatcaaatcatcagttccgaaaaagaaacgcaaagttgctagcg

SEQ ID NO: 467 - DNA, 388 bp, synthetic construct
  misc_feature 1..388: note = source = /note="Description of Artificial Sequence: Synthetic polynucleotide"
  source 1..388: mol_type = other DNA
taagcttcagtttttccttagttcctgttacatttctgtgtgtctccattagtgacctcccatagtccaagcatgagcagttctggccaggcccctgtcggggtcagtgccccacccccgccttctggttctgtgtaaccttctaagcaaaccttctggctcaagcacagcaatgctgagtcatgatgagtcatgctgaggcttagggtgtgtgcccagatgttctcagcctagagtgatgactcctatctgggtccccagcaggatgcttacagggcagatggcaaaaaaaaggagaagctgaccacctgactaaaactccacctcaaacggcatcataaagaaaatggatgcctgagacagaatgtgacatattctagaatatatt

SEQ ID NO: 468 - DNA, 19 bp, synthetic construct
  misc_feature 1..19: note = source = /note="Description of Artificial Sequence: Synthetic oligonucleotide"
  source 1..19: mol_type = other DNA
cagccgctcgctgcagcag

SEQ ID NO: 469 - DNA, 19 bp, synthetic construct
  misc_feature 1..19: note = source = /note="Description of Artificial Sequence: Synthetic oligonucleotide"
  source 1..19: mol_type = other DNA
ctgctgcagcgagcggctg

SEQ ID NO: 470 - DNA, 19 bp, synthetic construct
  misc_feature 1..19: note = source = /note="Description of Artificial Sequence: Synthetic oligonucleotide"
  source 1..19: mol_type = other DNA
gctgggtgtcccattgaaa

SEQ ID NO: 471 - DNA, 19 bp, synthetic construct
  misc_feature 1..19: note = source = /note="Description of Artificial Sequence: Synthetic oligonucleotide"
  source 1..19: mol_type = other DNA
tttcaatgggacacccagc

SEQ ID NO: 472 - DNA, 19 bp, synthetic construct
  misc_feature 1..19: note = source = /note="Description of Artificial Sequence: Synthetic oligonucleotide"
  source 1..19: mol_type = other DNA
gtttattcagccgggagtc

SEQ ID NO: 473 - DNA, 19 bp, synthetic construct
  misc_feature 1..19: note = source = /note="Description of Artificial Sequence: Synthetic oligonucleotide"
  source 1..19: mol_type = other DNA
gactcccggctgaataaac

SEQ ID NO: 474 - DNA, 19 bp, synthetic construct
  misc_feature 1..19: note = source = /note="Description of Artificial Sequence: Synthetic oligonucleotide"
  source 1..19: mol_type = other DNA
tggagagtttgcaaggagc

SEQ ID NO: 475 - DNA, 19 bp, synthetic construct
  misc_feature 1..19: note = source = /note="Description of Artificial Sequence: Synthetic oligonucleotide"
  source 1..19: mol_type = other DNA
gctccttgcaaactctcca

SEQ ID NO: 476 - DNA, 19 bp, synthetic construct
  misc_feature 1..19: note = source = /note="Description of Artificial Sequence: Synthetic oligonucleotide"
  source 1..19: mol_type = other DNA
ccctccagactttccacct

SEQ ID NO: 477 - DNA, 19 bp, synthetic construct
  misc_feature 1..19: note = source = /note="Description of Artificial Sequence: Synthetic oligonucleotide"
  source 1..19: mol_type = other DNA
aggtggaaagtctggaggg

SEQ ID NO: 478 - DNA, 19 bp, synthetic construct
  misc_feature 1..19: note = source = /note="Description of Artificial Sequence: Synthetic oligonucleotide"
  source 1..19: mol_type = other DNA
aattttcttccaagttctc

SEQ ID NO: 479 - DNA, 19 bp, synthetic construct
  misc_feature 1..19: note = source = /note="Description of Artificial Sequence: Synthetic oligonucleotide"
  source 1..19: mol_type = other DNA
gagaacttggaagaaaatt

SEQ ID NO: 480 - DNA, 19 bp, synthetic construct
  misc_feature 1..19: note = source = /note="Description of Artificial Sequence: Synthetic oligonucleotide"
  source 1..19: mol_type = other DNA
ctgcggagagaagaaaggg

SEQ ID NO: 481 - DNA, 19 bp, synthetic construct
  misc_feature 1..19: note = source = /note="Description of Artificial Sequence: Synthetic oligonucleotide"
  source 1..19: mol_type = other DNA
ccctttcttctctccgcag

SEQ ID NO: 482 - DNA, 19 bp, synthetic construct
  misc_feature 1..19: note = source = /note="Description of Artificial Sequence: Synthetic oligonucleotide"
  source 1..19: mol_type = other DNA
agagccaccccctggctcc

SEQ ID NO: 483 - DNA, 19 bp, synthetic construct
  misc_feature 1..19: note = source = /note="Description of Artificial Sequence: Synthetic oligonucleotide"
  source 1..19: mol_type = other DNA
ggagccagggggtggctct

SEQ ID NO: 484 - DNA, 19 bp, synthetic construct
  misc_feature 1..19: note = source = /note="Description of Artificial Sequence: Synthetic oligonucleotide"
  source 1..19: mol_type = other DNA
cgaagccaaccgcggcggg

SEQ ID NO: 485 - DNA, 19 bp, synthetic construct
  misc_feature 1..19: note = source = /note="Description of Artificial Sequence: Synthetic oligonucleotide"
  source 1..19: mol_type = other DNA
cccgccgcggttggcttcg

SEQ ID NO: 486 - DNA, 19 bp, synthetic construct
  misc_feature 1..19: note = source = /note="Description of Artificial Sequence: Synthetic oligonucleotide"
  source 1..19: mol_type = other DNA
agagggaagacgatcgccc

SEQ ID NO: 487 - DNA, 19 bp, synthetic construct
  misc_feature 1..19: note = source = /note="Description of Artificial Sequence: Synthetic oligonucleotide"
  source 1..19: mol_type = other DNA
gggcgatcgtcttccctct

SEQ ID NO: 488 - DNA, 19 bp, synthetic construct
  misc_feature 1..19: note = source = /note="Description of Artificial Sequence: Synthetic oligonucleotide"
  source 1..19: mol_type = other DNA
cccctttaactttcctccg

SEQ ID NO: 489 - DNA, 19 bp, synthetic construct
  misc_feature 1..19: note = source = /note="Description of Artificial Sequence: Synthetic oligonucleotide"
  source 1..19: mol_type = other DNA
cggaggaaagttaaagggg

SEQ ID NO: 490 - DNA, 19 bp, synthetic construct
  misc_feature 1..19: note = source = /note="Description of Artificial Sequence: Synthetic oligonucleotide"
  source 1..19: mol_type = other DNA
gcagccccgcttccttcaa

SEQ ID NO: 491 - DNA, 19 bp, synthetic construct
  misc_feature 1..19: note = source = /note="Description of Artificial Sequence: Synthetic oligonucleotide"
  source 1..19: mol_type = other DNA
ttgaaggaagcggggctgc

SEQ ID NO: 492 - DNA, 24 bp, synthetic construct
  misc_feature 1..24: note = source = /note="Description of Artificial Sequence: Synthetic oligonucleotide"
  source 1..24: mol_type = other DNA
caccgcagccgctcgctgcagcag

SEQ ID NO: 493 - DNA, 24 bp, synthetic construct
  misc_feature 1..24: note = source = /note="Description of Artificial Sequence: Synthetic oligonucleotide"
  source 1..24: mol_type = other DNA
aaacctgctgcagcgagcggctgc

SEQ ID NO: 494 - DNA, 24 bp, synthetic construct
  misc_feature 1..24: note = source = /note="Description of Artificial Sequence: Synthetic oligonucleotide"
  source 1..24: mol_type = other DNA
caccggctgggtgtcccattgaaa

SEQ ID NO: 495 - DNA, 24 bp, synthetic construct
  misc_feature 1..24: note = source = /note="Description of Artificial Sequence: Synthetic oligonucleotide"
  source 1..24: mol_type = other DNA
aaactttcaatgggacacccagcc

SEQ ID NO: 496 - DNA, 24 bp, synthetic construct
  misc_feature 1..24: note = source = /note="Description of Artificial Sequence: Synthetic oligonucleotide"
  source 1..24: mol_type = other DNA
caccggtttattcagccgggagtc

SEQ ID NO: 497 - DNA, 24 bp, synthetic construct
  misc_feature 1..24: note = source = /note="Description of Artificial Sequence: Synthetic oligonucleotide"
  source 1..24: mol_type = other DNA
aaacgactcccggctgaataaacc

SEQ ID NO: 498 - DNA, 24 bp, synthetic construct
  misc_feature 1..24: note = source = /note="Description of Artificial Sequence: Synthetic oligonucleotide"
  source 1..24: mol_type = other DNA
caccgtggagagtttgcaaggagc

SEQ ID NO: 499 - DNA, 24 bp, synthetic construct
  misc_feature 1..24: note = source = /note="Description of Artificial Sequence: Synthetic oligonucleotide"
  source 1..24: mol_type = other DNA
aaacgctccttgcaaactctccac

SEQ ID NO: 500 - DNA, 24 bp, synthetic construct
  misc_feature 1..24: note = source = /note="Description of Artificial Sequence: Synthetic oligonucleotide"
  source 1..24: mol_type = other DNA
caccgccctccagactttccacct

SEQ ID NO: 501 - DNA, 24 bp, synthetic construct
  misc_feature 1..24: note = source = /note="Description of Artificial Sequence: Synthetic oligonucleotide"
  source 1..24: mol_type = other DNA
aaacaggtggaaagtctggagggc

SEQ ID NO: 502 - DNA, 24 bp, synthetic construct
  misc_feature 1..24: note = source = /note="Description of Artificial Sequence: Synthetic oligonucleotide"
  source 1..24: mol_type = other DNA
caccgaattttcttccaagttctc

SEQ ID NO: 503 - DNA, 24 bp, synthetic construct
  misc_feature 1..24: note = source = /note="Description of Artificial Sequence: Synthetic oligonucleotide"
  source 1..24: mol_type = other DNA
aaacgagaacttggaagaaaattc

SEQ ID NO: 504 - DNA, 24 bp, synthetic construct
  misc_feature 1..24: note = source = /note="Description of Artificial Sequence: Synthetic oligonucleotide"
  source 1..24: mol_type = other DNA
caccgctgcggagagaagaaaggg

SEQ ID NO: 505 - DNA, 24 bp, synthetic construct
  misc_feature 1..24: note = source = /note="Description of Artificial Sequence: Synthetic oligonucleotide"
  source 1..24: mol_type = other DNA
aaacccctttcttctctccgcagc

SEQ ID NO: 506 - DNA, 24 bp, synthetic construct
  misc_feature 1..24: note = source = /note="Description of Artificial Sequence: Synthetic oligonucleotide"
  source 1..24: mol_type = other DNA
caccgagagccaccccctggctcc

SEQ ID NO: 507 - DNA, 24 bp, synthetic construct
  misc_feature 1..24: note = source = /note="Description of Artificial Sequence: Synthetic oligonucleotide"
  source 1..24: mol_type = other DNA
aaacggagccagggggtggctctc

SEQ ID NO: 508 - DNA, 24 bp, synthetic construct
  misc_feature 1..24: note = source = /note="Description of Artificial Sequence: Synthetic oligonucleotide"
  source 1..24: mol_type = other DNA
caccgcgaagccaaccgcggcggg

SEQ ID NO: 509 - DNA, 24 bp, synthetic construct
  misc_feature 1..24: note = source = /note="Description of Artificial Sequence: Synthetic oligonucleotide"
  source 1..24: mol_type = other DNA
aaaccccgccgcggttggcttcgc

SEQ ID NO: 510 - DNA, 24 bp, synthetic construct
  misc_feature 1..24: note = source = /note="Description of Artificial Sequence: Synthetic oligonucleotide"
  source 1..24: mol_type = other DNA
caccgagagggaagacgatcgccc

SEQ ID NO: 511 - DNA, 24 bp, synthetic construct
  misc_feature 1..24: note = source = /note="Description of Artificial Sequence: Synthetic oligonucleotide"
  source 1..24: mol_type = other DNA
aaacgggcgatcgtcttccctctc

SEQ ID NO: 512 - DNA, 24 bp, synthetic construct
  misc_feature 1..24: note = source = /note="Description of Artificial Sequence: Synthetic oligonucleotide"
  source 1..24: mol_type = other DNA
caccgcccctttaactttcctccg

SEQ ID NO: 513 - DNA, 24 bp, synthetic construct
  misc_feature 1..24: note = source = /note="Description of Artificial Sequence: Synthetic oligonucleotide"
  source 1..24: mol_type = other DNA
aaaccggaggaaagttaaaggggc

SEQ ID NO: 514 - DNA, 24 bp, synthetic construct
  misc_feature 1..24: note = source = /note="Description of Artificial Sequence: Synthetic oligonucleotide"
  source 1..24: mol_type = other DNA
caccggcagccccgcttccttcaa

SEQ ID NO: 515 - DNA, 24 bp, synthetic construct
  misc_feature 1..24: note = source = /note="Description of Artificial Sequence: Synthetic oligonucleotide"
  source 1..24: mol_type = other DNA
aaacttgaaggaagcggggctgcc

SEQ ID NO: 516 - DNA, 19 bp, synthetic construct
  misc_feature 1..19: note = source = /note="Description of Artificial Sequence: Synthetic oligonucleotide"
  source 1..19: mol_type = other DNA
cgagagcgagaggagggag

SEQ ID NO: 517 - DNA, 19 bp, synthetic construct
  misc_feature 1..19: note = source = /note="Description of Artificial Sequence: Synthetic oligonucleotide"
  source 1..19: mol_type = other DNA
ctccctcctctcgctctcg

SEQ ID NO: 518 - DNA, 19 bp, synthetic construct
  misc_feature 1..19: note = source = /note="Description of Artificial Sequence: Synthetic oligonucleotide"
  source 1..19: mol_type = other DNA
gagagagcttgagagcgcg

SEQ ID NO: 519 - DNA, 19 bp, synthetic construct
  misc_feature 1..19: note = source = /note="Description of Artificial Sequence: Synthetic oligonucleotide"
  source 1..19: mol_type = other DNA
cgcgctctcaagctctctc

SEQ ID NO: 520 - DNA, 19 bp, synthetic construct
  misc_feature 1..19: note = source = /note="Description of Artificial Sequence: Synthetic oligonucleotide"
  source 1..19: mol_type = other DNA
ggtggagggggcggggccc

SEQ ID NO: 521 - DNA, 19 bp, synthetic construct
  misc_feature 1..19: note = source = /note="Description of Artificial Sequence: Synthetic oligonucleotide"
  source 1..19: mol_type = other DNA
gggccccgccccctccacc

SEQ ID NO: 522 - DNA, 19 bp, synthetic construct
  misc_feature 1..19: note = source = /note="Description of Artificial Sequence: Synthetic oligonucleotide"
  source 1..19: mol_type = other DNA
ggtatccacgtaaatcaaa

SEQ ID NO: 523 - DNA, 19 bp, synthetic construct
  misc_feature 1..19: note = source = /note="Description of Artificial Sequence: Synthetic oligonucleotide"
  source 1..19: mol_type = other DNA
tttgatttacgtggatacc

SEQ ID NO: 524 - DNA, 19 bp, synthetic construct
  misc_feature 1..19: note = source = /note="Description of Artificial Sequence: Synthetic oligonucleotide"
  source 1..19: mol_type = other DNA
ccaatcactggctccggtc

SEQ ID NO: 525 - DNA, 19 bp, synthetic construct
  misc_feature 1..19: note = source = /note="Description of Artificial Sequence: Synthetic oligonucleotide"
  source 1..19: mol_type = other DNA
gaccggagccagtgattgg

SEQ ID NO: 526 - DNA, 19 bp, synthetic construct
  misc_feature 1..19: note = source = /note="Description of Artificial Sequence: Synthetic oligonucleotide"
  source 1..19: mol_type = other DNA
ggcgcccgagggaagaaga

SEQ ID NO: 527 - DNA, 19 bp, synthetic construct
  misc_feature 1..19: note = source = /note="Description of Artificial Sequence: Synthetic oligonucleotide"
  source 1..19: mol_type = other DNA
tcttcttccctcgggcgcc

SEQ ID NO: 528 - DNA, 19 bp, synthetic construct
  misc_feature 1..19: note = source = /note="Description of Artificial Sequence: Synthetic oligonucleotide"
  source 1..19: mol_type = other DNA
gggtgggggtaccagagga

SEQ ID NO: 529 - DNA, 19 bp, synthetic construct
  misc_feature 1..19: note = source = /note="Description of Artificial Sequence: Synthetic oligonucleotide"
  source 1..19: mol_type = other DNA
tcctctggtacccccaccc

SEQ ID NO: 530 - DNA, 19 bp, synthetic construct
  misc_feature 1..19: note = source = /note="Description of Artificial Sequence: Synthetic oligonucleotide"
  source 1..19: mol_type = other DNA
ccggggacagaagagaggg

SEQ ID NO: 531 - DNA, 19 bp, synthetic construct
  misc_feature 1..19: note = source = /note="Description of Artificial Sequence: Synthetic oligonucleotide"
  source 1..19: mol_type = other DNA
ccctctcttctgtccccgg

SEQ ID NO: 532 - DNA, 19 bp, synthetic construct
  misc_feature 1..19: note = source = /note="Description of Artificial Sequence: Synthetic oligonucleotide"
  source 1..19: mol_type = other DNA
gagagagagtgggagaagc

SEQ ID NO: 533 - DNA, 19 bp, synthetic construct
  misc_feature 1..19: note = source = /note="Description of Artificial Sequence: Synthetic oligonucleotide"
  source 1..19: mol_type = other DNA
gcttctcccactctctctc

SEQ ID NO: 534 - DNA, 19 bp, synthetic construct
  misc_feature 1..19: note = source = /note="Description of Artificial Sequence: Synthetic oligonucleotide"
  source 1..19: mol_type = other DNA
aaagtaactgtcaaatgcg

SEQ ID NO: 535 - DNA, 19 bp, synthetic construct
  misc_feature 1..19: note = source = /note="Description of Artificial Sequence: Synthetic oligonucleotide"
  source 1..19: mol_type = other DNA
cgcatttgacagttacttt

SEQ ID NO: 536 - DNA, 19 bp, synthetic construct
  misc_feature 1..19: note = source = /note="Description of Artificial Sequence: Synthetic oligonucleotide"
  source 1..19: mol_type = other DNA
ttaaccagagcgcccagtc

SEQ ID NO: 537 - DNA, 19 bp, synthetic construct
  misc_feature 1..19: note = source = /note="Description of Artificial Sequence: Synthetic oligonucleotide"
  source 1..19: mol_type = other DNA
gactgggcgctctggttaa

SEQ ID NO: 538 - DNA, 19 bp, synthetic construct
  misc_feature 1..19: note = source = /note="Description of Artificial Sequence: Synthetic oligonucleotide"
  source 1..19: mol_type = other DNA
cgtcggagctgcccgctag

SEQ ID NO: 539 - DNA, 19 bp, synthetic construct
  misc_feature 1..19: note = source = /note="Description of Artificial Sequence: Synthetic oligonucleotide"
  source 1..19: mol_type = other DNA
ctagcgggcagctccgacg

SEQ ID NO: 540 - DNA, 24 bp, synthetic construct
  misc_feature 1..24: note = source = /note="Description of Artificial Sequence: Synthetic oligonucleotide"
  source 1..24: mol_type = other DNA
caccgcgagagcgagaggagggag

SEQ ID NO: 541 - DNA, 24 bp, synthetic construct
  misc_feature 1..24: note = source = /note="Description of Artificial Sequence: Synthetic oligonucleotide"
  source 1..24: mol_type = other DNA
aaacctccctcctctcgctctcgc

SEQ ID NO: 542 - DNA, 24 bp, synthetic construct
  misc_feature 1..24: note = source = /note="Description of Artificial Sequence: Synthetic oligonucleotide"
  source 1..24: mol_type = other DNA
caccggagagagcttgagagcgcg

SEQ ID NO: 543 - DNA, 24 bp, synthetic construct
  misc_feature 1..24: note = source = /note="Description of Artificial Sequence: Synthetic oligonucleotide"
  source 1..24: mol_type = other DNA
aaaccgcgctctcaagctctctcc

SEQ ID NO: 544 - DNA, 24 bp, synthetic construct
  misc_feature 1..24: note = source = /note="Description of Artificial Sequence: Synthetic oligonucleotide"
  source 1..24: mol_type = other DNA
caccgggtggagggggcggggccc

SEQ ID NO: 545 - DNA, 24 bp, synthetic construct
  misc_feature 1..24: note = source = /note="Description of Artificial Sequence: Synthetic oligonucleotide"
  source 1..24: mol_type = other DNA
aaacgggccccgccccctccaccc

SEQ ID NO: 546 - DNA, 24 bp, synthetic construct
  misc_feature 1..24: note = source = /note="Description of Artificial Sequence: Synthetic oligonucleotide"
  source 1..24: mol_type = other DNA
caccgggtatccacgtaaatcaaa

SEQ ID NO: 547 - DNA, 24 bp, synthetic construct
  misc_feature 1..24: note = source = /note="Description of Artificial Sequence: Synthetic oligonucleotide"
  source 1..24: mol_type = other DNA
aaactttgatttacgtggataccc

SEQ ID NO: 548 - DNA, 24 bp, synthetic construct
  misc_feature 1..24: note = source = /note="Description of Artificial Sequence: Synthetic oligonucleotide"
  source 1..24: mol_type = other DNA
caccgccaatcactggctccggtc

SEQ ID NO: 549 - DNA, 24 bp, synthetic construct
  misc_feature 1..24: note = source = /note="Description of Artificial Sequence: Synthetic oligonucleotide"
  source 1..24: mol_type = other DNA
aaacgaccggagccagtgattggc

SEQ ID NO: 550 - DNA, 24 bp, synthetic construct
  misc_feature 1..24: note = source = /note="Description of Artificial Sequence: Synthetic oligonucleotide"
  source 1..24: mol_type = other DNA
caccgggcgcccgagggaagaaga

SEQ ID NO: 551 - DNA, 24 bp, synthetic construct
  misc_feature 1..24: note = source = /note="Description of Artificial Sequence: Synthetic oligonucleotide"
  source 1..24: mol_type = other DNA
aaactcttcttccctcgggcgccc

SEQ ID NO: 552 - DNA, 24 bp, synthetic construct
  misc_feature 1..24: note = source = /note="Description of Artificial Sequence: Synthetic oligonucleotide"
  source 1..24: mol_type = other DNA
caccggggtgggggtaccagagga

SEQ ID NO: 553 - DNA, 24 bp, synthetic construct
  misc_feature 1..24: note = source = /note="Description of Artificial Sequence: Synthetic oligonucleotide"
  source 1..24: mol_type = other DNA
aaactcctctggtacccccacccc

SEQ ID NO: 554 - DNA, 24 bp, synthetic construct
  misc_feature 1..24: note = source = /note="Description of Artificial Sequence: Synthetic oligonucleotide"
  source 1..24: mol_type = other DNA
caccgccggggacagaagagaggg

SEQ ID NO: 555 - DNA, 24 bp, synthetic construct
  misc_feature 1..24: note = source = /note="Description of Artificial Sequence: Synthetic oligonucleotide"
  source 1..24: mol_type = other DNA
aaacccctctcttctgtccccggc

SEQ ID NO: 556 - DNA, 24 bp, synthetic construct
  misc_feature 1..24: note = source = /note="Description of Artificial Sequence: Synthetic oligonucleotide"
  source 1..24: mol_type = other DNA
caccggagagagagtgggagaagc

SEQ ID NO: 557 - DNA, 24 bp, synthetic construct
  misc_feature 1..24: note = source = /note="Description of Artificial Sequence: Synthetic oligonucleotide"
  source 1..24: mol_type = other DNA
aaacgcttctcccactctctctcc

SEQ ID NO: 558 - DNA, 24 bp, synthetic construct
  misc_feature 1..24: note = source = /note="Description of Artificial Sequence: Synthetic oligonucleotide"
  source 1..24: mol_type = other DNA
caccgaaagtaactgtcaaatgcg

SEQ ID NO: 559 - DNA, 24 bp, synthetic construct
  misc_feature 1..24: note = source = /note="Description of Artificial Sequence: Synthetic oligonucleotide"
  source 1..24: mol_type = other DNA
aaaccgcatttgacagttactttc

SEQ ID NO: 560 - DNA, 24 bp, synthetic construct
  misc_feature 1..24: note = source = /note="Description of Artificial Sequence: Synthetic oligonucleotide"
  source 1..24: mol_type = other DNA
caccgttaaccagagcgcccagtc

SEQ ID NO: 561 - DNA, 24 bp, synthetic construct
  misc_feature 1..24: note = source = /note="Description of Artificial Sequence: Synthetic oligonucleotide"
  source 1..24: mol_type = other DNA
aaacgactgggcgctctggttaac

SEQ ID NO: 562 - DNA, 24 bp, synthetic construct
  misc_feature 1..24: note = source = /note="Description of Artificial Sequence: Synthetic oligonucleotide"
  source 1..24: mol_type = other DNA
caccgcgtcggagctgcccgctag

SEQ ID NO: 563 - DNA, 24 bp, synthetic construct
  misc_feature 1..24: note = source = /note="Description of Artificial Sequence: Synthetic oligonucleotide"
  source 1..24: mol_type = other DNA
aaacctagcgggcagctccgacgc

SEQ ID NO: 564 - DNA, 20 bp, synthetic construct
  misc_feature 1..20: note = source = /note="Description of Artificial Sequence: Synthetic oligonucleotide"
  source 1..20: mol_type = other DNA
gagacacacagaaatgtaac

SEQ ID NO: 565 - DNA, 20 bp, synthetic construct
  misc_feature 1..20: note = source = /note="Description of Artificial Sequence: Synthetic oligonucleotide"
  source 1..20: mol_type = other DNA
ggtggggcactgaccccgac

SEQ ID NO: 566 - DNA, 20 bp, synthetic construct
  misc_feature 1..20: note = source = /note="Description of Artificial Sequence: Synthetic oligonucleotide"
  source 1..20: mol_type = other DNA
ctagagtgatgactcctatc

SEQ ID NO: 567 - DNA, 20 bp, synthetic construct
  misc_feature 1..20: note = source = /note="Description of Artificial Sequence: Synthetic oligonucleotide"
  source 1..20: mol_type = other DNA
gactaaaactccacctcaaa

SEQ ID NO: 568 - DNA, 20 bp, synthetic construct
  misc_feature 1..20: note = source = /note="Description of Artificial Sequence: Synthetic oligonucleotide"
  source 1..20: mol_type = other DNA
aatatgtcacattctgtctc

SEQ ID NO: 569 - DNA, 20 bp, synthetic construct
  misc_feature 1..20: note = source = /note="Description of Artificial Sequence: Synthetic oligonucleotide"
  source 1..20: mol_type = other DNA
ggactatgggaggtcactaa

SEQ ID NO: 570 - DNA, 20 bp, synthetic construct
  misc_feature 1..20: note = source = /note="Description of Artificial Sequence: Synthetic oligonucleotide"
  source 1..20: mol_type = other DNA
gctcatgcttggactatggg

SEQ ID NO: 571 - DNA, 20 bp, synthetic construct
  misc_feature 1..20: note = source = /note="Description of Artificial Sequence: Synthetic oligonucleotide"
  source 1..20: mol_type = other DNA
gttctggccaggcccctgtc

SEQ ID NO: 572 - DNA, 20 bp, synthetic construct
  misc_feature 1..20: note = source = /note="Description of Artificial Sequence: Synthetic oligonucleotide"
  source 1..20: mol_type = other DNA
agtgccccacccccgccttc

SEQ ID NO: 573 - DNA, 20 bp, synthetic construct
  misc_feature 1..20: note = source = /note="Description of Artificial Sequence: Synthetic oligonucleotide"
  source 1..20: mol_type = other DNA
gtggggcactgaccccgaca

SEQ ID NO: 574 - DNA, 20 bp, synthetic construct
  misc_feature 1..20: note = source = /note="Description of Artificial Sequence: Synthetic oligonucleotide"
  source 1..20: mol_type = other DNA
aaccttctaagcaaaccttc

SEQ ID NO: 575 - DNA, 20 bp, synthetic construct
  misc_feature 1..20: note = source = /note="Description of Artificial Sequence: Synthetic oligonucleotide"
  source 1..20: mol_type = other DNA
gttacacagaaccagaaggc

SEQ ID NO: 576 - DNA, 20 bp, synthetic construct
  misc_feature 1..20: note = source = /note="Description of Artificial Sequence: Synthetic oligonucleotide"
  source 1..20: mol_type = other DNA
gaaggttacacagaaccaga

SEQ ID NO: 577 - DNA, 20 bp, synthetic construct
  misc_feature 1..20: note = source = /note="Description of Artificial Sequence: Synthetic oligonucleotide"
  source 1..20: mol_type = other DNA
agtcatgatgagtcatgctg

SEQ ID NO: 578 - DNA, 20 bp, synthetic construct
  misc_feature 1..20: note = source = /note="Description of Artificial Sequence: Synthetic oligonucleotide"
  source 1..20: mol_type = other DNA
gatgagtcatgctgaggctt

SEQ ID NO: 579 - DNA, 20 bp, synthetic construct
  misc_feature 1..20: note = source = /note="Description of Artificial Sequence: Synthetic oligonucleotide"
  source 1..20: mol_type = other DNA
actctaggctgagaacatct

SEQ ID NO: 580 - DNA, 20 bp, synthetic construct
  misc_feature 1..20: note = source = /note="Description of Artificial Sequence: Synthetic oligonucleotide"
  source 1..20: mol_type = other DNA
gtccccagcaggatgcttac

SEQ ID NO: 581 - DNA, 20 bp, synthetic construct
  misc_feature 1..20: note = source = /note="Description of Artificial Sequence: Synthetic oligonucleotide"
  source 1..20: mol_type = other DNA
gccctgtaagcatcctgctg

SEQ ID NO: 582 - DNA, 20 bp, synthetic construct
  misc_feature 1..20: note = source = /note="Description of Artificial Sequence: Synthetic oligonucleotide"
  source 1..20: mol_type = other DNA
cagggcagatggcaaaaaaa

SEQ ID NO: 583 - DNA, 20 bp, synthetic construct
  misc_feature 1..20: note = source = /note="Description of Artificial Sequence: Synthetic oligonucleotide"
  source 1..20: mol_type = other DNA
gaggtggagttttagtcagg

SEQ ID NO: 584 - DNA, 20 bp, synthetic construct
  misc_feature 1..20: note = source = /note="Description of Artificial Sequence: Synthetic oligonucleotide"
  source 1..20: mol_type = other DNA
aaacggcatcataaagaaaa

SEQ ID NO: 585 - DNA, 105 bp, synthetic construct
  misc_feature 1..105: note = source = /note="Description of Artificial Sequence: Synthetic polynucleotide"
  source 1..105: mol_type = other DNA
gagacacacagaaatgtaacgttttagagctagaaatagcaagttaaaataaggctagtccgttatcaacttgaaaaagtggcaccgagtcggtgctttttttcc

SEQ ID NO: 586 - DNA, 105 bp, synthetic construct
  misc_feature 1..105: note = source = /note="Description of Artificial Sequence: Synthetic polynucleotide"
  source 1..105: mol_type = other DNA
ggtggggcactgaccccgacgttttagagctagaaatagcaagttaaaataaggctagtccgttatcaacttgaaaaagtggcaccgagtcggtgctttttttcc

SEQ ID NO: 587 - DNA, 105 bp, synthetic construct
  misc_feature 1..105: note = source = /note="Description of Artificial Sequence: Synthetic polynucleotide"
  source 1..105: mol_type = other DNA
ctagagtgatgactcctatcgttttagagctagaaatagcaagttaaaataaggctagtccgttatcaacttgaaaaagtggcaccgagtcggtgctttttttcc

SEQ ID NO: 588 - DNA, 105 bp, synthetic construct
  misc_feature 1..105: note = source = /note="Description of Artificial Sequence: Synthetic polynucleotide"
  source 1..105: mol_type = other DNA
gactaaaactccacctcaaagttttagagctagaaatagcaagttaaaataaggctagtccgttatcaacttgaaaaagtggcaccgagtcggtgctttttttcc

SEQ ID NO: 589 - DNA, 105 bp, synthetic construct
  misc_feature 1..105: note = source = /note="Description of Artificial Sequence: Synthetic polynucleotide"
  source 1..105: mol_type = other DNA
aatatgtcacattctgtctcgttttagagctagaaatagcaagttaaaataaggctagtccgttatcaacttgaaaaagtggcaccgagtcggtgctttttttcc

SEQ ID NO: 590 - DNA, 105 bp, synthetic construct
  misc_feature 1..105: note = source = /note="Description of Artificial Sequence: Synthetic polynucleotide"
  source 1..105: mol_type = other DNA
ggactatgggaggtcactaagttttagagctagaaatagcaagttaaaataaggctagtccgttatcaacttgaaaaagtggcaccgagtcggtgctttttttcc

SEQ ID NO: 591 - DNA, 105 bp, synthetic construct
  misc_feature 1..105: note = source = /note="Description of Artificial Sequence: Synthetic polynucleotide"
  source 1..105: mol_type = other DNA
gctcatgcttggactatggggttttagagctagaaatagcaagttaaaataaggctagtccgttatcaacttgaaaaagtggcaccgagtcggtgctttttttcc

SEQ ID NO: 592 - DNA, 105 bp, synthetic construct
  misc_feature 1..105: note = source = /note="Description of Artificial Sequence: Synthetic polynucleotide"
  source 1..105: mol_type = other DNA
gttctggccaggcccctgtcgttttagagctagaaatagcaagttaaaataaggctagtccgttatcaacttgaaaaagtggcaccgagtcggtgctttttttcc

SEQ ID NO: 593 - DNA, 105 bp, synthetic construct
  misc_feature 1..105: note = source = /note="Description of Artificial Sequence: Synthetic polynucleotide"
  source 1..105: mol_type = other DNA
agtgccccacccccgccttcgttttagagctagaaatagcaagttaaaataaggctagtccgttatcaacttgaaaaagtggcaccgagtcggtgctttttttcc

SEQ ID NO: 594 - DNA, 105 bp, synthetic construct
  misc_feature 1..105: note = source = /note="Description of Artificial Sequence: Synthetic polynucleotide"
  source 1..105: mol_type = other DNA
gtggggcactgaccccgacagttttagagctagaaatagcaagttaaaataaggctagtccgttatcaacttgaaaaagtggcaccgagtcggtgctttttttcc

SEQ ID NO: 595 - DNA, 105 bp, synthetic construct
  misc_feature 1..105: note = source = /note="Description of Artificial Sequence: Synthetic polynucleotide"
  source 1..105: mol_type = other DNA
aaccttctaagcaaaccttcgttttagagctagaaatagcaagttaaaataaggctagtccgttatcaacttgaaaaagtggcaccgagtcggtgctttttttcc

SEQ ID NO: 596 - DNA, 105 bp, synthetic construct
  misc_feature 1..105: note = source = /note="Description of Artificial Sequence: Synthetic polynucleotide"
  source 1..105: mol_type = other DNA
gttacacagaaccagaaggcgttttagagctagaaatagcaagttaaaataaggctagtccgttatcaacttgaaaaagtggcaccgagtcggtgctttttttcc

SEQ ID NO: 597 - DNA, 105 bp, synthetic construct
  misc_feature 1..105: note = source = /note="Description of Artificial Sequence: Synthetic polynucleotide"
  source 1..105: mol_type = other DNA
gaaggttacacagaaccagagttttagagctagaaatagcaagttaaaataaggctagtccgttatcaacttgaaaaagtggcaccgagtcggtgctttttttcc

SEQ ID NO: 598 - DNA, 105 bp, synthetic construct
  misc_feature 1..105: note = source = /note="Description of Artificial Sequence: Synthetic polynucleotide"
  source 1..105: mol_type = other DNA
agtcatgatgagtcatgctggttttagagctagaaatagcaagttaaaataaggctagtccgttatcaacttgaaaaagtggcaccgagtcggtgctttttttcc

SEQ ID NO: 599 - DNA, 105 bp, synthetic construct
  misc_feature 1..105: note = source = /note="Description of Artificial Sequence: Synthetic polynucleotide"
  source 1..105: mol_type = other DNA
gatgagtcatgctgaggcttgttttagagctagaaatagcaagttaaaataaggctagtccgttatcaacttgaaaaagtggcaccgagtcggtgctttttttcc

SEQ ID NO: 600 - DNA, 105 bp, synthetic construct
  misc_feature 1..105: note = source = /note="Description of Artificial Sequence: Synthetic polynucleotide"
  source 1..105: mol_type = other DNA
actctaggctgagaacatctgttttagagctagaaatagcaagttaaaataaggctagtccgttatcaacttgaaaaagtggcaccgagtcggtgctttttttcc

SEQ ID NO: 601 - DNA, 105 bp, synthetic construct
  misc_feature 1..105: note = source = /note="Description of Artificial Sequence: Synthetic polynucleotide"
  source 1..105: mol_type = other DNA
gtccccagcaggatgcttacgttttagagctagaaatagcaagttaaaataaggctagtccgttatcaacttgaaaaagtggcaccgagtcggtgctttttttcc

SEQ ID NO: 602 - DNA, 105 bp, synthetic construct
  misc_feature 1..105: note = source = /note="Description of Artificial Sequence: Synthetic polynucleotide"
  source 1..105: mol_type = other DNA
gccctgtaagcatcctgctggttttagagctagaaatagcaagttaaaataaggctagtccgttatcaacttgaaaaagtggcaccgagtcggtgctttttttcc

SEQ ID NO: 603 - DNA, 105 bp, synthetic construct
  misc_feature 1..105: note = source = /note="Description of Artificial Sequence: Synthetic polynucleotide"
  source 1..105: mol_type = other DNA
cagggcagatggcaaaaaaagttttagagctagaaatagcaagttaaaataaggctagtccgttatcaacttgaaaaagtggcaccgagtcggtgctttttttcc

SEQ ID NO: 604 - DNA, 105 bp, synthetic construct
  misc_feature 1..105: note = source = /note="Description of Artificial Sequence: Synthetic polynucleotide"
  source 1..105: mol_type = other DNA
gaggtggagttttagtcagggttttagagctagaaatagcaagttaaaataaggctagtccgttatcaacttgaaaaagtggcaccgagtcggtgctttttttcc

SEQ ID NO: 605 - DNA, 105 bp, synthetic construct
  misc_feature 1..105: note = source = /note="Description of Artificial Sequence: Synthetic polynucleotide"
  source 1..105: mol_type = other DNA
aaacggcatcataaagaaaagttttagagctagaaatagcaagttaaaataaggctagtccgttatcaacttgaaaaagtggcaccgagtcggtgctttttttcc

SEQ ID NO: 606 - DNA, 19 bp, synthetic construct
  misc_feature 1..19: note = source = /note="Description of Artificial Sequence: Synthetic oligonucleotide"
  source 1..19: mol_type = other DNA
tgtactctctgaggtgctc

SEQ ID NO: 607 - DNA, 19 bp, synthetic construct
  misc_feature 1..19: note = source = /note="Description of Artificial Sequence: Synthetic oligonucleotide"
  source 1..19: mol_type = other DNA
acgcagataagaaccagtt

SEQ ID NO: 608 - DNA, 19 bp, synthetic construct
  misc_feature 1..19: note = source = /note="Description of Artificial Sequence: Synthetic oligonucleotide"
  source 1..19: mol_type = other DNA
catcaagtcagccatcagc

SEQ ID NO: 609 - DNA, 19 bp, synthetic construct
  misc_feature 1..19: note = source = /note="Description of Artificial Sequence: Synthetic oligonucleotide"
  source 1..19: mol_type = other DNA
gagtcaccctcctggaaac

SEQ ID NO: 610 - DNA, 19 bp, synthetic construct
  misc_feature 1..19: note = source = /note="Description of Artificial Sequence: Synthetic oligonucleotide"
  source 1..19: mol_type = other DNA
cctgggctccggggcgttt

SEQ ID NO: 611 - DNA, 19 bp, synthetic construct
  misc_feature 1..19: note = source = /note="Description of Artificial Sequence: Synthetic oligonucleotide"
  source 1..19: mol_type = other DNA
ggcccctgcggccaccccg

SEQ ID NO: 612 - DNA, 19 bp, synthetic construct
  misc_feature 1..19: note = source = /note="Description of Artificial Sequence: Synthetic oligonucleotide"
  source 1..19: mol_type = other DNA
ctccctccctgcccggtag

SEQ ID NO: 613 - DNA, 19 bp, synthetic construct
  misc_feature 1..19: note = source = /note="Description of Artificial Sequence: Synthetic oligonucleotide"
  source 1..19: mol_type = other DNA
aggtttggaaagggcgtgc

SEQ ID NO: 614 - DNA, 20 bp, synthetic construct
  misc_feature 1..20: note = source = /note="Description of Artificial Sequence: Synthetic oligonucleotide"
  source 1..20: mol_type = other DNA
actccactgcactccagtct

SEQ ID NO: 615 - DNA, 20 bp, synthetic construct
  misc_feature 1..20: note = source = /note="Description of Artificial Sequence: Synthetic oligonucleotide"
  source 1..20: mol_type = other DNA
tctgtgggggacctgcactg

SEQ ID NO: 616 - DNA, 20 bp, synthetic construct
  misc_feature 1..20: note = source = /note="Description of Artificial Sequence: Synthetic oligonucleotide"
  source 1..20: mol_type = other DNA
ggggcgccagttgtgtctcc

SEQ ID NO: 617 - DNA, 20 bp, synthetic construct
  misc_feature 1..20: note = source = /note="Description of Artificial Sequence: Synthetic oligonucleotide"
  source 1..20: mol_type = other DNA
acaccattgccaccaccatt

SEQ ID NO: 618 - DNA, 20 bp, synthetic construct
  misc_feature 1..20: note = source = /note="Description of Artificial Sequence: Synthetic primer"
  source 1..20: mol_type = other DNA
caatgaccccttcattgacc

SEQ ID NO: 619 - DNA, 20 bp, synthetic construct
  misc_feature 1..20: note = source = /note="Description of Artificial Sequence: Synthetic primer"
  source 1..20: mol_type = other DNA
ttgattttggagggatctcg

SEQ ID NO: 620 - DNA, 20 bp, synthetic construct
  misc_feature 1..20: note = source = /note="Description of Artificial Sequence: Synthetic primer"
  source 1..20: mol_type = other DNA
ggaatccatggagggaagat

SEQ ID NO: 621 - DNA, 20 bp, synthetic construct
  misc_feature 1..20: note = source = /note="Description of Artificial Sequence: Synthetic primer"
  source 1..20: mol_type = other DNA
tgttctcgctcaggtcagtg

SEQ ID NO: 622 - DNA, 20 bp, synthetic construct
  misc_feature 1..20: note = source = /note="Description of Artificial Sequence: Synthetic primer"
  source 1..20: mol_type = other DNA
ctctctgctcctttgccaca

SEQ ID NO: 623 - DNA, 20 bp, synthetic construct
  misc_feature 1..20: note = source = /note="Description of Artificial Sequence: Synthetic primer"
  source 1..20: mol_type = other DNA
gtgctcttcgggtttcagga

SEQ ID NO: 624 - DNA, 30 bp, synthetic construct
  misc_feature 1..30: note = source = /note="Description of Artificial Sequence: Synthetic primer"
  source 1..30: mol_type = other DNA
cgaaagagaaagcgaaccagtatcgagaac

SEQ ID NO: 625 - DNA, 27 bp, synthetic construct
  misc_feature 1..27: note = source = /note="Description of Artificial Sequence: Synthetic primer"
  source 1..27: mol_type = other DNA
cgttgtgcatagtcgctgcttgatcgc

SEQ ID NO: 626 - DNA, 25 bp, synthetic construct
  misc_feature 1..25: note = source = /note="Description of Artificial Sequence: Synthetic primer"
  source 1..25: mol_type = other DNA
gagtttggctcaaattgttactctt

SEQ ID NO: 627 - DNA, 25 bp, synthetic construct
  misc_feature 1..25: note = source = /note="Description of Artificial Sequence: Synthetic primer"
  source 1..25: mol_type = other DNA
gggaaatggtctaggagagtaaagt

SEQ ID NO: 628 - DNA, 23 bp, synthetic construct
  misc_feature 1..23: note = source = /note="Description of Artificial Sequence: Synthetic oligonucleotide"
  source 1..23: mol_type = other DNA
gattggctttgatttccctaggg

SEQ ID NO: 629 - DNA, 23 bp, synthetic construct
  misc_feature 1..23: note = source = /note="Description of Artificial Sequence: Synthetic oligonucleotide"
  source 1..23: mol_type = other DNA
gcctactcagactgttactctgg

SEQ ID NO: 630 - DNA, 23 bp, synthetic construct
  misc_feature 1..23: note = source = /note="Description of Artificial Sequence: Synthetic oligonucleotide"
  source 1..23: mol_type = other DNA
gcagttgcctaagaactggtggg

SEQ ID NO: 631 - DNA, 23 bp, synthetic construct
  misc_feature 1..23: note = source = /note="Description of Artificial Sequence: Synthetic oligonucleotide"
  source 1..23: mol_type = other DNA
ggggctccaccctcacgagtggg

SEQ ID NO: 632 - DNA, 23 bp, synthetic construct
  misc_feature 1..23: note = source = /note="Description of Artificial Sequence: Synthetic oligonucleotide"
  source 1..23: mol_type = other DNA
gccttctttatcccctatcgagg

SEQ ID NO: 633 - DNA, 48 bp, synthetic construct
  misc_feature 1..48: note = source = /note="Description of Artificial Sequence: Synthetic oligonucleotide"
  source 1..48: mol_type = other DNA
  CDS 1..45
gaaggaccatttgacgttcagctcctactcagactgttactctggtga

SEQ ID NO: 634 - protein, 15 aa, synthetic construct
  REGION 1..15: note = source = /note="Description of Artificial Sequence: Synthetic peptide"
EGPFDVQLLLRLLLW

SEQ ID NO: 635 - DNA, 46 bp, synthetic construct
  misc_feature 1..46: note = source = /note="Description of Artificial Sequence: Synthetic oligonucleotide"
  source 1..46: mol_type = other DNA
  CDS 1..42
gaaggaccatttgacgttcagctcctactcagactgtctctggtga

SEQ ID NO: 636 - protein, 14 aa, synthetic construct
  REGION 1..14: note = source = /note="Description of Artificial Sequence: Synthetic peptide"
EGPFDVQLLLRLSL

SEQ ID NO: 637 - RNA, 20 nt, synthetic construct
  misc_feature 1..20: note = source = /note="Description of Artificial Sequence: Synthetic oligonucleotide"
  source 1..20: mol_type = other RNA
gcctactcagactgttactc

SEQ ID NO: 638 - DNA, 19 bp, synthetic construct
  misc_feature 1..19: note = source = /note="Description of Artificial Sequence: Synthetic oligonucleotide"
  source 1..19: mol_type = other DNA
cccaccagttcttaggcaa

SEQ ID NO: 639 - DNA, 20 bp, synthetic construct
  misc_feature 1..20: note = source = /note="Description of Artificial Sequence: Synthetic oligonucleotide"
  source 1..20: mol_type = other DNA
cccaccagttcttaggcaac

SEQ ID NO: 640 - DNA, 20 bp, synthetic construct
  misc_feature 1..20: note = source = /note="Description of Artificial Sequence: Synthetic oligonucleotide"
  source 1..20: mol_type = other DNA
tttgatttccagttcttagg

SEQ ID NO: 641 - DNA, 19 bp, synthetic construct
  misc_feature 1..19: note = source = /note="Description of Artificial Sequence: Synthetic oligonucleotide"
  source 1..19: mol_type = other DNA
attaccatagagttcttag

SEQ ID NO: 642 - DNA, 19 bp, synthetic construct
  misc_feature 1..19: note = source = /note="Description of Artificial Sequence: Synthetic oligonucleotide"
  source 1..19: mol_type = other DNA
gtggataaaggcaacaatg

SEQ ID NO: 643 - DNA, 16 bp, synthetic construct
  misc_feature 1..16: note = source = /note="Description of Artificial Sequence: Synthetic oligonucleotide"
  source 1..16: mol_type = other DNA
cctcgataggggataa

SEQ ID NO: 644 - DNA, 23 bp, synthetic construct
  misc_feature 1..23: note = source = /note="Description of Artificial Sequence: Synthetic oligonucleotide"
  source 1..23: mol_type = other DNA
accaaacccacttaggggataaa

SEQ ID NO: 645 - DNA, 21 bp, synthetic construct
  misc_feature 1..21: note = source = /note="Description of Artificial Sequence: Synthetic oligonucleotide"
  source 1..21: mol_type = other DNA
ggtatcttaaggacctccaag

SEQ ID NO: 646 - DNA, 47 bp, synthetic construct
  misc_feature 1..47: note = source = /note="Description of Artificial Sequence: Synthetic oligonucleotide"
  source 1..47: mol_type = other DNA
taggaagtaaattaatttgaagcttgccaattaatccaaatcttacc

SEQ ID NO: 647 - DNA, 83 bp, synthetic construct
  misc_feature 1..83: note = source = /note="Description of Artificial Sequence: Synthetic primer"
  source 1..83: mol_type = other DNA
tttcctttttgcaaaacccaaaatattttagctcctactcagactgttagagtaggaggagaaggagggctgtggctcttgtg

SEQ ID NO: 648 - DNA, 83 bp, synthetic construct
  variation 20: note = a, c, t, g, unknown or other
  variation 31: note = a, c, t, g, unknown or other
  variation 69: note = a, c, t, g, unknown or other
  misc_feature 1..83: note = source = /note="Description of Artificial Sequence: Synthetic primer"
  source 1..83: mol_type = other DNA
aaaacccccaaaccctcccnctttttcctcntactctaacagtgtgagtaggaggccacacttagctgnggctctagtaagtc

SEQ ID NO: 649 - DNA, 94 bp, synthetic construct
  variation 50: note = a, c, t, g, unknown or other
  misc_feature 1..94: note = source = /note="Description of Artificial Sequence: Synthetic primer"
  source 1..94: mol_type = other DNA
cttcttttttcctttttgcaaaaacccaaaatattttagctcctactcanaccgttttcggggggtattttgtatttggatgaaacacttgatg

SEQ ID NO: 650 - DNA, 93 bp, synthetic construct
  misc_feature 1..93: note = source = /note="Description of Artificial Sequence: Synthetic primer"
  source 1..93: mol_type = other DNA
tcttcttttttccttcccgcaaaaacccaaaatattttcgctcctactcaggacctggtcgtggggtattttgtatttggatgaaacacttga

SEQ ID NO: 651 - DNA, 104 bp, synthetic construct
  stem_loop 21..22: note = a, c, t, g, unknown or other
  misc_feature 1..104: note = source = /note="Description of Artificial Sequence: Synthetic primer"
  source 1..104: mol_type = other DNA
tcaaggaagatggcatttctnntttggagatggcagtttccttagtaaccacaggttgtgtcaccatggccagtaagaaggatgccacacttgtgtgtgtcgct

SEQ ID NO: 652 - DNA, 86 bp, synthetic construct
  variation 35..36: note = a, c, t, g, unknown or other
  variation 42..44: note = a, c, t, g, unknown or other
  misc_feature 1..86: note = source = /note="Description of Artificial Sequence: Synthetic primer"
  source 1..86: mol_type = other DNA
ttggagatagcagtttccttggtaagtacaggttnntcaccnnnacagtgtgagtaggaggccacacttagctgtggctctagtaa

SEQ ID NO: 653 - DNA, 71 bp, synthetic construct
  variation 54: note = a, c, t, g, unknown or other
  variation 61..63: note = a, c, t, g, unknown or other
  variation 69: note = a, c, t, g, unknown or other
  misc_feature 1..71: note = source = /note="Description of Artificial Sequence: Synthetic primer"
  source 1..71: mol_type = other DNA
tttctagtttggagatggcagtttccttagtaaccacaggttgtgtcaccaggnctcgagnnntggttntg

SEQ ID NO: 654 - DNA, 87 bp, synthetic construct
  misc_feature 1..87: note = source = /note="Description of Artificial Sequence: Synthetic primer"
  source 1..87: mol_type = other DNA
cagttgccatagtcttcactaaccgcgtcaccagagctcaggacctggtcgtggggtattttgtatttggatgaaacacttgatggt

SEQ ID NO: 655 - DNA, 92 bp, synthetic construct
  variation 52: note = a, c, t, g, unknown or other
  variation 59: note = a, c, t, g, unknown or other
  variation 78: note = a, c, t, g, unknown or other
  misc_feature 1..92: note = source = /note="Description of Artificial Sequence: Synthetic primer"
  source 1..92: mol_type = other DNA
tattgtatcttggtttttcttcactgctggccagtttactaacaatctgaantaagccnattaatccaaatcttaccngacgaaaaatcaaa

SEQ ID NO: 656 - DNA, 89 bp, synthetic construct
  variation 6: note = a, c, t, g, unknown or other
  variation 10: note = a, c, t, g, unknown or other
  variation 19: note = a, c, t, g, unknown or other
  variation 30: note = a, c, t, g, unknown or other
  variation 57: note = a, c, t, g, unknown or other
  misc_feature 1..89: note = source = /note="Description of Artificial Sequence: Synthetic primer"
  source 1..89: mol_type = other DNA
atggtntttngtcattgcnggccagttttntaacaatgtgatcaatgccaattaatncaaatcttaccagaggaaaaatcaagccacag

SEQ ID NO: 657 - DNA, 94 bp, synthetic construct
  variation 93..94: note = a, c, t, g, unknown or other
  misc_feature 1..94: note = source = /note="Description of Artificial Sequence: Synthetic primer"
  source 1..94: mol_type = other DNA
aataaaaagaaaaaaatatgataaactgctcccagtataaaatacagagctaagacaagaacgtttcattggctgttaaaagtcggaaatcgnn

SEQ ID NO: 658 - DNA, 94 bp, synthetic construct
  misc_feature 1..94: note = source = /note="Description of Artificial Sequence: Synthetic primer"
  source 1..94: mol_type = other DNA
ttctgatttaaaattcccttgaataggaagtaaattaatttgaagcttgccaattaatccaaatcttaccagaggaaaaatcaagccacagata

SEQ ID NO: 659 - DNA, 90 bp, synthetic construct
  misc_feature 1..90: note = source = /note="Description of Artificial Sequence: Synthetic primer"
  source 1..90: mol_type = other DNA
caaaacaagatgggataaaatcttctttctgatttaaaattcccttgaataggaagtaaattactagagctgttcaaggcctgaactcta

SEQ ID NO: 660 - DNA, 96 bp, synthetic construct
  variation 49: note = a, c, t, g, unknown or other
  variation 51..52: note = a, c, t, g, unknown or other
  variation 54: note = a, c, t, g, unknown or other
  misc_feature 1..96: note = source = /note="Description of Artificial Sequence: Synthetic primer"
  source 1..96: mol_type = other DNA
ctgatttaaaattcccttgaataggaagtaaattactagagctgttcangnncngaactctaggctagcatttccagcccaaaacaaacacagttc

SEQ ID NO: 661-668 - skipped (8 entries)

SEQ ID NO: 669 - DNA, 26 bp, synthetic construct
  misc_feature 1..26: note = source = /note="Description of Artificial Sequence: Synthetic oligonucleotide"
  source 1..26: mol_type = other DNA
ttgtttgtcttcgagaagacctgttt

SEQ ID NO: 670 - DNA, 26 bp, synthetic construct
  misc_feature 1..26: note = source = /note="Description of Artificial Sequence: Synthetic oligonucleotide"
  source 1..26: mol_type = other DNA
caccgggtcttcgagaagacctgttt

SEQ ID NO: 671 - DNA, 26 bp, synthetic construct
  misc_feature 1..26: note = source = /note="Description of Artificial Sequence: Synthetic oligonucleotide"
  source 1..26: mol_type = other DNA
tcccaggtcttcgagaagacctgttt

SEQ ID NO: 672 - DNA, 26 bp, synthetic construct
  misc_feature 1..26: note = source = /note="Description of Artificial Sequence: Synthetic oligonucleotide"
  source 1..26: mol_type = other DNA
cctcgggtcttcgagaagacctgttt

SEQ ID NO: 673 - DNA, 25 bp, synthetic construct
  misc_feature 1..25: note = source = /note="Description of Artificial Sequence: Synthetic oligonucleotide"
  source 1..25: mol_type = other DNA
ggcctaccgctaaggctagcctagt

SEQ ID NO: 674 - protein, 1411 aa, synthetic construct
  REGION 1..1411: note = source = /note="Description of Artificial Sequence: Synthetic polypeptide"
MDYKDHDGDYKDHDIDYKDDDDKMAPKKKRKVGRGMDKKYSIGLAIGTNSVGWAVITDEYKVPSKKFKVLGNTDRHSIKKNLIGALLFDSGETAEATRLKRTARRRYTRRKNRICYLQEIFSNEMAKVDDSFFHRLEESFLVEEDKKHERHPIFGNIVDEVAYHEKYPTIYHLRKKLVDSTDKADLRLIYLALAHMIKFRGHFLIEGDLNPDNSDVDKLFIQLVQTYNQLFEENPINASGVDAKAILSARLSKSRRLENLIAQLPGEKKNGLFGNLIALSLGLTPNFKSNFDLAEDAKLQLSKDTYDDDLDNLLAQIGDQYADLFLAAKNLSDAILLSDILRVNTEITKAPLSASMIKRYDEHHQDLTLLKALVRQQLPEKYKEIFFDQSKNGYAGYIDGGASQEEFYKFIKPILEKMDGTEELLVKLNREDLLRKQRTFDNGSIPHQIHLGELHAILRRQEDFYPFLKDNREKIEKILTFRIPYYVGPLARGNSRFAWMTRKSEETITPWNFEEVVDKGASAQSFIERMTNFDKNLPNEKVLPKHSLLYEYFTVYNELTKVKYVTEGMRKPAFLSGEQKKAIVDLLFKTNRKVTVKQLKEDYFKKIECFDSVEISGVEDRFNASLGTYHDLLKIIKDKDFLDNEENEDILEDIVLTLTLFEDREMIEERLKTYAHLFDDKVMKQLKRRRYTGWGRLSRKLINGIRDKQSGKTILDFLKSDGFANRNFMQLIHDDSLTFKEDIQKAQVSGQGDSLHEHIANLAGSPAIKKGILQTVKVVDELVKVMGRHKPENIVIEMARENQTTQKGQKNSRERMKRIEEGIKELGSQILKEHPVENTQLQNEKLYLYYLQNGRDMYVDQELDINRLSDYDVDHIVPQSFLKDDSIDNKVLTRSDKNRGKSDNVPSEEVVKKMKNYWRQLLNAKLITQRKFDNLTKAERGGLSELDKAGFIKRQLVETRQITKHVAQILDSRMNTKYDENDKLIREVKVITLKSKLVSDFRKDFQFYKVREINNYHHAHDAYLNAVVGTALIKKYPKLESEFVYGDYKVYDVRKMIAKSEQEIGKATAKYFFYSNIMNFFKTEITLANGEIRKRPLIETNGETGEIVWDKGRDFATVRKVLSMPQVNIVKKTEVQTGGFSKESILPKRNSDKLIARKKDWDPKKYGGFDSPTVAYSVLVVAKVEKGKSKKLKSVKELLGITIMERSSFEKNPIDFLEAKGYKEVKKDLIIKLPKYSLFELENGRKRMLASAGELQKGNELALPSKYVNFLYLASHYEKLKGSPEDNEQKQLFVEQHKHYLDEIIEQISEFSKRVILADANLDKVLSAYNKHRDKPIREQAENIIHLFTLTNLGAPAAFKYFDTTIDRKRYTSTKEVLDATLIHQSITGLYETRIDLSQLGGDPKKKRKVG

SEQ ID NO: 675 - protein, 1483 aa, synthetic construct; identical to SEQ ID NO: 1
  REGION 1..1483: note = source = /note="Description of Artificial Sequence: Synthetic polypeptide"

SEQ ID NO: 676 - protein, 2048 aa, synthetic construct
  REGION 1..2048: note = source = /note="Description of Artificial Sequence: Synthetic polypeptide"
MDYKDHDGDYKDHDIDYKDDDDKMAPKKKRKVGRGMDKKYSIGLAIGTNSVGWAVITDEYKVPSKKFKVLGNTDRHSIKKNLIGALLFDSGETAEATRLKRTARRRYTRRKNRICYLQEIFSNEMAKVDDSFFHRLEESFLVEEDKKHERHPIFGNIVDEVAYHEKYPTIYHLRKKLVDSTDKADLRLIYLALAHMIKFRGHFLIEGDLNPDNSDVDKLFIQLVQTYNQLFEENPINASGVDAKAILSARLSKSRRLENLIAQLPGEKKNGLFGNLIALSLGLTPNFKSNFDLAEDAKLQLSKDTYDDDLDNLLAQIGDQYADLFLAAKNLSDAILLSDILRVNTEITKAPLSASMIKRYDEHHQDLTLLKALVRQQLPEKYKEIFFDQSKNGYAGYIDGGASQEEFYKFIKPILEKMDGTEELLVKLNREDLLRKQRTFDNGSIPHQIHLGELHAILRRQEDFYPFLKDNREKIEKILTFRIPYYVGPLARGNSRFAWMTRKSEETITPWNFEEVVDKGASAQSFIERMTNFDKNLPNEKVLPKHSLLYEYFTVYNELTKVKYVTEGMRKPAFLSGEQKKAIVDLLFKTNRKVTVKQLKEDYFKKIECFDSVEISGVEDRFNASLGTYHDLLKIIKDKDFLDNEENEDILEDIVLTLTLFEDREMIEERLKTYAHLFDDKVMKQLKRRRYTGWGRLSRKLINGIRDKQSGKTILDFLKSDGFANRNFMQLIHDDSLTFKEDIQKAQVSGQGDSLHEHIANLAGSPAIKKGILQTVKVVDELVKVMGRHKPENIVIEMARENQTTQKGQKNSRERMKRIEEGIKELGSQILKEHPVENTQLQNEKLYLYYLQNGRDMYVDQELDINRLSDYDVDAIVPQSFLKDDSIDNKVLTRSDKNRGKSDNVPSEEVVKKMKNYWRQLLNAKLITQRKFDNLTKAERGGLSELDKAGFIKRQLVETRQITKHVAQILDSRMNTKYDENDKLIREVKVITLKSKLVSDFRKDFQFYKVREINNYHHAHDAYLNAVVGTALIKKYPKLESEFVYGDYKVYDVRKMIAKSEQEIGKATAKYFFYSNIMNFFKTEITLANGEIRKRPLIETNGETGEIVWDKGRDFATVRKVLSMPQVNIVKKTEVQTGGFSKESILPKRNSDKLIARKKDWDPKKYGGFDSPTVAYSVLVVAKVEKGKSKKLKSVKELLGITIMERSSFEKNPIDFLEAKGYKEVKKDLIIKLPKYSLFELENGRKRMLASAGELQKGNELALPSKYVNFLYLASHYEKLKGSPEDNEQKQLFVEQHKHYLDEIIEQISEFSKRVILADANLDKVLSAYNKHRDKPIREQAENIIHLFTLTNLGAPAAFKYFDTTIDRKRYTSTKEVLDATLIHQSITGLYETRIDLSQLGGDPIAGSKASPKKKRKVGRAIFKPEELRQALMPTLEALYRQDPESLPFRQPVDPQLLGIPDYFDIVKSPMDLSTIKRKLDTGQYQEPWQYVDDIWLMFNNAWLYNRKTSRVYKYCSKLSEVFEQEIDPVMQSLGYCCGRKLEFSPQTLCCYGKQLCTIPRDATYYSYQNRYHFCEKCFNEIQGESVSLGDDPSQPQTTINKEQFSKRKNDTLDPELFVECTECGRKMHQICVLHHEIIWPAGFVCDGCLKKSARTRKENKFSAKRLPSTRLGTFLENRVNDFLRRQNHPESGEVTVRVVHASDKTVEVKPGMKARFVDSGEMAESFPYRTKALFAFEEIDGVDLCFFGMHVQEYGSDCPPPNQRRVYISYLDSVHFFRPKCLRTAVYHEILIGYLEYVKKLGYTTGHIWACPPSEGDDYIFHCHPPDQKIPKPKRLQEWYKKMLDKAVSERIVHDYKDIFKQATEDRLTSAKELPYFEGDFWPNVLEESIKELEQEEEERKREENTSNESTDVTKGDSKNAKKKNNKKTSKNKSSLSRGNKKKPGMPNVSNDLSQKLYATMEKHKEVFFVIRLIAGPAANSLPPIVDPDPLIPCDLMDGRDAFLTLARDKHLEFSSLRRAQWSTMCMLVELHTQSQDYPYDVPDYAS